European Patent Application EP 4 768 595 A1, published July 1, 2026. Title: Antigens and related assay to detect and measure auto-antibodies in a subject developing type 1 diabetes (T1D). Applicant: Ospedale S. Raffaele. The sequence listing filed with the application follows.

SEQUENCE LISTING (97 sequences)

SEQ ID NO: 1 - DNA, 864 bp, synthetic construct
  source 1..864: mol_type = other DNA; note = Insulin B NLuc
atggccctgtggatgcgcctcctgcccctgctggcgctgctggccctctggggacctgacccagccgcagcctttgtgaaccaacacctgtgcggctcacacctggtggaagctctctacctagtgtgcggggaacgaggcttcttctacacacccaagaccatggtcttcacactcgaagatttcgttggggactggcgacagacagccggctacaacctggaccaagtccttgaacagggaggtgtgtccagtttgtttcagaatctcggggtgtccgtaactccgatccaaaggattgtcctgagcggtgaaaatgggctgaagatcgacatccatgtcatcatcccgtatgaaggtctgagcggcgaccaaatgggccagatcgaaaaaatttttaaggtggtgtaccctgtggatgatcatcactttaaggtgatcctgcactatggcacactggtaatcgacggggttacgccgaacatgatcgactatttcggacggccgtatgaaggcatcgccgtgttcgacggcaaaaagatcactgtaacagggaccctgtggaacggcaacaaaattatcgacgagcgcctgatcaaccccgacggctccctgctgttccgagtaaccatcaacggagtgaccggctggcggctgtgcgaacgcattctggcggctgctgctgcgcgccggaagcgggaggacctgcaggtggggcaggtggagctgggcgggggcccaggccctggtgcaggcagcctgcagcccttggccctggaggggtcccgacgcaagcgtggcattgtggaacaatgctgtaccagcatctgctccctctaccagctggagaactactgcaactag

SEQ ID NO: 2 - DNA, 1689 bp, synthetic construct
  source 1..1689: mol_type = other DNA; note = NLuc IA-2ic
atggtcttcacactcgaagatttcgttggggactggcgacagacagccggctacaacctggaccaagtccttgaacagggaggtgtgtccagtttgtttcagaatctcggggtgtccgtaactccgatccaaaggattgtcctgagcggtgaaaatgggctgaagatcgacatccatgtcatcatcccgtatgaaggtctgagcggcgaccaaatgggccagatcgaaaaaatttttaaggtggtgtaccctgtggatgatcatcactttaaggtgatcctgcactatggcacactggtaatcgacggggttacgccgaacatgatcgactatttcggacggccgtatgaaggcatcgccgtgttcgacggcaaaaagatcactgtaacagggaccctgtggaacggcaacaaaattatcgacgagcgcctgatcaaccccgacggctccctgctgttccgagtaaccatcaacggagtgaccggctggcggctgtgcgaacgcattctggcgggtggaggctctagagaattcacgcgtggtaccgccgccaccatggagcggcagcaagacaaggagcgcctggcagccctggggcctgagggggcccatggtgacactacctttgagtaccaggacctgtgccgccagcacatggccacgaagtccttgttcaaccgggcagagggtccaccggagccttcacgggtgagcagtgtgtcctcccagttcagcgacgcagcccaggccagccccagctcccacagcagcaccccgtcctggtgcgaggagccggcccaagccaacatggacatctccacgggacacatgattctggcatacatggaggatcacctgcggaaccgggaccgccttgccaaggagtggcaggccctctgtgcctaccaagcagagccaaacacctgtgccaccgcgcagggggagggcaacatcaaaaagaaccggcatcctgacttcctgccctatgaccatgcccgcataaaactgaaggtggagagcagcccttctcggagcgattacatcaacgccagccccattattgagcatgaccctcggatgccagcctacatagccacgcagggcccgctgtcccataccatcgcagacttctggcagatggtgtgggagagcggctgcaccgtcatcgtcatgctgaccccgctggtggaggatggtgtcaagcagtgtgaccgctactggccagatgagggtgcctccctctaccacgtatatgaggtgaacctggtgtcggagcacatctggtgcgaggacttcctggtgcggagcttctacctgaagaacgtgcagacccaggagacgcgcacgctcacgcagttccacttcctcagctggccggcagagggcacaccggcctccacgcggcccctgctggacttccgcaggaaggtgaacaagtgctaccggggccgctcctgccccatcatcgtgcactgcagtgatggtgcggggaggaccggcacctacatcctcatcgacatggtcctgaaccgcatggcaaaaggagtgaaggagattgacatcgctgccaccctggagcatgtccgtgaccagcggcctggccttgtccgctctaaggaccagtttgagtttgccctgacagccgtggcggaggaagtgaatgccatcctcaaggccctgccccagtga

SEQ ID NO: 3 - DNA, 2844 bp, synthetic construct
  source 1..2844: mol_type = other DNA; note = Dual NLuc IA-2ic
atggagcggcagcaagacaaggagcgcctggcagccctggggcctgagggggcccatggtgacactacctttgagtaccaggacctgtgccgccagcacatggccacgaagtccttgttcaaccgggcagagggtccaccggagccttcacgggtgagcagtgtgtcctcccagttcagcgacgcagcccagaccagccccagctcccacagcagcaccccgtcctggtgcgaggagccggcccaagccaacatggacatctccacgggacacatgattctggcatacatggaggatcacctgcggaaccgggaccgccttgccaaggagtggcaggccctctgtgcctaccaagcagagccaaacacctgtgccaccgcgcagggggagggcaacatcaaaaagaaccggcatcctgacttcctgccctatgaccatgcccgcataaaactgaaggtggagagcagcccttctcggagcgattacatcaacgccagccccattattgagcatgaccctcggatgccagcctacatagccacgcagggcccgctgtcccataccatcgcagacttctggcagatggtgtgggagagcggctgcaccgtcatcgtcatgctgaccccgctggtggaggatggtgtcaagcagtgtgaccgctactggccagatgagggtgcctccctctaccacgtatatgaggtgaacctggtgtcggagcacatctggtgcgaggacttcctggtgcggagcttctacctgaagaacgtgcagacccaggagacgcgcacgctcacgcagttccacttcctcagctggccggcagagggcacaccggcctccacgcggcccctgctggacttccgcaggaaggtgaacaagtgctaccggggccgctcctgccccatcatcgtgcactgcagtgatggtgcggggaggaccggcacctacatcctcatcgacatggtcctgaaccgcatggcaaaaggagtgaaggagattgacatcgctgccaccctggagcatgtccgtgaccagcggcctggccttgtccgctctaaggaccagtttgagtttgccctgacagccgtggcggaggaagtgaatgccatcctcaaggccctgccccagggtaccggcgggggtatggtcttcacactcgaagatttcgttggggactggcgacagacagccggctacaacctggaccaagtccttgaacagggaggtgtgtccagtttgtttcagaatctcggggtgtccgtaactccgatccaaaggattgtcctgagcggtgaaaatgggctgaagatcgacatccatgtcatcatcccgtatgaaggtctgagcggcgaccaaatgggccagatcgaaaaaatttttaaggtggtgtaccctgtggatgatcatcactttaaggtgatcctgcactatggcacactggtaatcgacggggttacgccgaacatgatcgactatttcggacggccgtatgaaggcatcgccgtgttcgacggcaaaaagatcactgtaacagggaccctgtggaacggcaacaaaattatcgacgagcgcctgatcaaccccgacggctccctgctgttccgagtaaccatcaacggagtgaccggctggcggctgtgcgaacgcattctggcgggcgcgagcggtggtggcgggagcggaggtggagggtcgtcaggtgcggccgcagagcggcagcaagacaaggagcgcctggcagccctggggcctgagggggcccatggtgacactacctttgagtaccaggacctgtgccgccagcacatggccacgaagtccttgttcaaccgggcagagggtccaccggagccttcacgggtgagcagtgtgtcctcccagttcagcgacgcagcccagaccagccccagctcccacagcagcaccccgtcctggtgcgaggagccggcccaagccaacatggacatctccacgggacacatgattctggcatacatggaggatcacctgcggaaccgggaccgccttgccaaggagtggcaggccctctgtgcctaccaagcagagccaaacacctgtgccaccgcgcagggggagggcaacatcaaaaagaaccggcatcctgacttcctgccctatgaccatgcccgcataaaactgaaggtggagagcagcccttctcggagcgattacatcaacgccagccccattattgagcatgaccctcggatgccagcctacatagccacgcagggcccgctgtcccataccatcgcagacttctggcagatggtgtgggagagcggctgcaccgtcatcgtcatgctgaccccgctggtggaggatggtgtcaagcagtgtgaccgctactggccagatgagggtgcctccctctaccacgtatatgaggtgaacctggtgtcggagcacatctggtgcgaggacttcctggtgcggagcttctacctgaagaacgtgcagacccaggagacgcgcacgctcacgcagttccacttcctcagctggccggcagagggcacaccggcctccacgcggcccctgctggacttccgcaggaaggtgaacaagtgctaccggggccgctcctgccccatcatcgtgcactgcagtgatggtgcggggaggaccggcacctacatcctcatcgacatggtcctgaaccgcatggcaaaaggagtgaaggagattgacatcgctgccaccctggagcatgtccgtgaccagcggcctggccttgtccgctctaaggaccagtttgagtttgccctgacagccgtggcggaggaagtgaatgccatcctcaaggccctgccccagtaa

SEQ ID NO: 4 - DNA, 1779 bp, synthetic construct
  source 1..1779: mol_type = other DNA; note = NLuc IA-2ic trimeric
atggagcggcagcaagacaaggagcgcctggcagccctggggcctgagggggcccatggtgacactacctttgagtaccaggacctgtgccgccagcacatggccacgaagtccttgttcaaccgggcagagggtccaccggagccttcacgggtgagcagtgtgtcctcccagttcagcgacgcagcccaggccagccccagctcccacagcagcaccccgtcctggtgcgaggagccggcccaagccaacatggacatctccacgggacacatgattctggcatacatggaggatcacctgcggaaccgggaccgccttgccaaggagtggcaggccctctgtgcctaccaagcagagccaaacacctgtgccaccgcgcagggggagggcaacatcaaaaagaaccggcatcctgacttcctgccctatgaccatgcccgcataaaactgaaggtggagagcagcccttctcggagcgattacatcaacgccagccccattattgagcatgaccctcggatgccagcctacatagccacgcagggcccgctgtcccataccatcgcagacttctggcagatggtgtgggagagcggctgcaccgtcatcgtcatgctgaccccgctggtggaggatggtgtcaagcagtgtgaccgctactggccagatgagggtgcctccctctaccacgtatatgaggtgaacctggtgtcggagcacatctggtgcgaggacttcctggtgcggagcttctacctgaagaacgtgcagacccaggagacgcgcacgctcacgcagttccacttcctcagctggccggcagagggcacaccggcctccacgcggcccctgctggacttccgcaggaaggtgaacaagtgctaccggggccgctcctgccccatcatcgtgcactgcagtgatggtgcggggaggaccggcacctacatcctcatcgacatggtcctgaaccgcatggcaaaaggagtgaaggagattgacatcgctgccaccctggagcatgtccgtgaccagcggcctggccttgtccgctctaaggaccagtttgaatttgccctgacagccgtggcggaggaagtgaatgccatcctcaaggccctgccccagggtacctctagagtcgacccgggcggccgcggtggaggcatggtcttcacactcgaagatttcgttggggactggcgacagacagccggctacaacctggaccaagtccttgaacagggaggtgtgtccagtttgtttcagaatctcggggtgtccgtaactccgatccaaaggattgtcctgagcggtgaaaatgggctgaagatcgacatccatgtcatcatcccgtatgaaggtctgagcggcgaccaaatgggccagatcgaaaaaatttttaaggtggtgtaccctgtggatgatcatcactttaaggtgatcctgcactatggcacactggtaatcgacggggttacgccgaacatgatcgactatttcggacggccgtatgaaggcatcgccgtgttcgacggcaaaaagatcactgtaacagggaccctgtggaacggcaacaaaattatcgacgagcgcctgatcaaccccgacggctccctgctgttccgagtaaccatcaacggagtgaccggctggcggctgtgcgaacgcattctggcggctgctgctgcgggctacatccccgaggcccccagggacggccaggcctacgtgaggaaggacggcgagtgggtgctgctgagcaccttcctgtaa

SEQ ID NO: 5 - DNA, 1854 bp, synthetic construct
  source 1..1854: mol_type = other DNA; note = Dual NLuc ZnT8 dimer
atggagaaggacttctccatcttactcatggaaggtgtgccaaagagcctgaattacagtggtgtgaaagagcttattttagcagtcgacggggtgctgtctgtgcacagcctgcacatctggtctctaacaatgaatcaagtaattctctcagctcatgttgctacagcagccagctgggacagccaagtggttcggagagaaattgctaaagcccttagcaaaagctttacgatgcactcactcaccattcagatggaatctccagttgaccaggaccccgactgccttttctgtgaagacccctgtgacggcggcggcaaggacttctccatcttactcatggaaggtgtgccaaagagcctgaattacagtggtgtgaaagagcttattttagcagtcgacggggtgctgtctgtgcacagcctgcacatctggtctctaacaatgaatcaagtaattctctcagctcatgttgctacagcagccagccgggacagccaagtggttcggagagaaattgctaaagcccttagcaaaagctttacgatgcactcactcaccattcagatggaatctccagttgaccaggaccccgactgccttttctgtgaagacccctgtgacggtaccggcgggggtatggtcttcacactcgaagatttcgttggggactggcgacagacagccggctacaacctggaccaagtccttgaacagggaggtgtgtccagtttgtttcagaatctcggggtgtccgtaactccgatccaaaggattgtcctgagcggtgaaaatgggctgaagatcgacatccatgtcatcatcccgtatgaaggtctgagcggcgaccaaatgggccagatcgaaaaaatttttaaggtggtgtaccctgtggatgatcatcactttaaggtgatcctgcactatggcacactggtaatcgacggggttacgccgaacatgatcgactatttcggacggccgtatgaaggcatcgccgtgttcgacggcaaaaagatcactgtaacagggaccctgtggaacggcaacaaaattatcgacgagcgcctgatcaaccccgacggctccctgctgttccgagtaaccatcaacggagtgaccggctggcggctgtgcgaacgcattctggcgggcgcgagcggtggtggcgggagcggaggtggagggtcgtcaggtgcggccgcggaattcgccgccaccatggagaaggacttctccatcttactcatggaaggtgtgccaaagagcctgaattacagtggtgtgaaagagcttattttagcagtcgacggggtgctgtctgtgcacagcctgcacatctggtctctaacaatgaatcaagtaattctctcagctcatgttgctacagcagccagctgggacagccaagtggttcggagagaaattgctaaagcccttagcaaaagctttacgatgcactcactcaccattcagatggaatctccagttgaccaggaccccgactgccttttctgtgaagacccctgtgacggcggcggcaaggacttctccatcttactcatggaaggtgtgccaaagagcctgaattacagtggtgtgaaagagcttattttagcagtcgacggggtgctgtctgtgcacagcctgcacatctggtctctaacaatgaatcaagtaattctctcagctcatgttgctacagcagccagccgggacagccaagtggttcggagagaaattgctaaagcccttagcaaaagctttacgatgcactcactcaccattcagatggaatctccagttgaccaggaccccgactgccttttctgtgaagacccctgtgactag

SEQ ID NO: 6 - DNA, 2031 bp, synthetic construct
  source 1..2031: mol_type = other DNA; note = NLuc GAD65 aa96_585
atggtcttcacactcgaagatttcgttggggactggcgacagacagccggctacaacctggaccaagtccttgaacagggaggtgtgtccagtttgtttcagaatctcggggtgtccgtaactccgatccaaaggattgtcctgagcggtgaaaatgggctgaagatcgacatccatgtcatcatcccgtatgaaggtctgagcggcgaccaaatgggccagatcgaaaaaatttttaaggtggtgtaccctgtggatgatcatcactttaaggtgatcctgcactatggcacactggtaatcgacggggttacgccgaacatgatcgactatttcggacggccgtatgaaggcatcgccgtgttcgacggcaaaaagatcactgtaacagggaccctgtggaacggcaacaaaattatcgacgagcgcctgatcaaccccgacggctccctgctgttccgagtaaccatcaacggagtgaccggctggcggctgtgcgaacgcattctggcgggtggaggctctagagaattcacgcgtggtaccgccgccaccatggacctgctgccggcgtgtgatggagaaaggcccactttggcgtttctgcaagatgttatgaacattttacttcagtatgtggtgaaaagtttcgatagatcaaccaaagtgattgatttccattatcctaatgagcttctccaagaatataattgggaattggcagaccaaccacaaaatttggaggaaattttgatgcattgccaaacaactctaaaatatgcaattaaaacagggcatcctagatacttcaatcaactttctactggtttggatatggttggattagcagcagactggctgacatcaacagcaaatactaacatgttcacctatgaaattgctccagtatttgtgcttttggaatatgtcacactaaagaaaatgagagaaatcattggctggccagggggctctggcgatgggatattttctcccggtggcgccatatctaacatgtatgccatgatgatcgcacgctttaagatgttcccagaagtcaaggagaaaggaatggctgctcttcccaggctcattgccttcacgtctgaacatagtcatttttctctcaagaagggagctgcagccttagggattggaacagacagcgtgattctgattaaatgtgatgagagagggaaaatgattccatctgatcttgaaagaaggattcttgaagccaaacagaaagggtttgttcctttcctcgtgagtgccacagctggaaccaccgtgtacggagcatttgaccccctcttagctgtcgctgacatttgcaaaaagtataagatctggatgcatgtggatgcagcttggggtgggggattactgatgtcccgaaaacacaagtggaaactgagtggcgtggagagggccaactctgtgacgtggaatccacacaagatgatgggagtccctttgcagtgctctgctctcctggttagagaagagggattgatgcagaattgcaaccaaatgcatgcctcctacctctttcagcaagataaacattatgacctgtcctatgacactggagacaaggccttacagtgcggacgccacgttgatgtttttaaactatggctgatgtggagggcaaaggggactaccgggtttgaagcgcatgttgataaatgtttggagttggcagagtatttatacaacatcataaaaaaccgagaaggatatgagatggtgtttgatgggaagcctcagcacacaaatgtctgcttctggtacattcctccaagcttgcgtactctggaagacaatgaagagagaatgagtcgcctctcgaaggtggctccagtgattaaagccagaatgatggagtatggaaccacaatggtcagctaccaacccttgggagacaaggtcaatttcttccgcatggtcatctcaaacccagcggcaactcaccaagacattgacttcctgattgaagaaatagaacgccttggacaagatttataa

SEQ ID NO: 7 - DNA, 1476 bp, synthetic construct
  source 1..1476: mol_type = other DNA; note = GAD65aa96-585 competitor
atggacctgctgccggcgtgtgatggagaaaggcccactttggcgtttctgcaagatgttatgaacattttacttcagtatgtggtgaaaagtttcgatagatcaaccaaagtgattgatttccattatcctaatgagcttctccaagaatataattgggaattggcagaccaaccacaaaatttggaggaaattttgatgcattgccaaacaactctaaaatatgcaattaaaacagggcatcctagatacttcaatcaactttctactggtttggatatggttggattagcagcagactggctgacatcaacagcaaatactaacatgttcacctatgaaattgctccagtatttgtgcttttggaatatgtcacactaaagaaaatgagagaaatcattggctggccagggggctctggcgatgggatattttctcccggtggcgccatatctaacatgtatgccatgatgatcgcacgctttaagatgttcccagaagtcaaggagaaaggaatggctgctcttcccaggctcattgccttcacgtctgaacatagtcatttttctctcaagaagggagctgcagccttagggattggaacagacagcgtgattctgattaaatgtgatgagagagggaaaatgattccatctgatcttgaaagaaggattcttgaagccaaacagaaagggtttgttcctttcctcgtgagtgccacagctggaaccaccgtgtacggagcatttgaccccctcttagctgtcgctgacatttgcaaaaagtataagatctggatgcatgtggatgcagcttggggtgggggattactgatgtcccgaaaacacaagtggaaactgagtggcgtggagagggccaactctgtgacgtggaatccacacaagatgatgggagtccctttgcagtgctctgctctcctggttagagaagagggattgatgcagaattgcaaccaaatgcatgcctcctacctctttcagcaagataaacattatgacctgtcctatgacactggagacaaggccttacagtgcggacgccacgttgatgtttttaaactatggctgatgtggagggcaaaggggactaccgggtttgaagcgcatgttgataaatgtttggagttggcagagtatttatacaacatcataaaaaaccgagaaggatatgagatggtgtttgatgggaagcctcagcacacaaatgtctgcttctggtacattcctccaagcttgcgtactctggaagacaatgaagagagaatgagtcgcctctcgaaggtggctccagtgattaaagccagaatgatggagtatggaaccacaatggtcagctaccaacccttgggagacaaggtcaatttcttccgcatggtcatctcaaacccagcggcaactcaccaagacattgacttcctgattgaagaaatagaacgccttggacaagatttataa

SEQ ID NO: 8 - DNA, 333 bp, synthetic construct
  source 1..333: mol_type = other DNA; note = proinsulin competitor
atggccctgtggatgcgcctcctgcccctgctggcgctgctggccctctggggacctgacccagccgcagcctttgtgaaccaacacctgtgcggctcacacctggtggaagctctctacctagtgtgcggggaacgaggcttcttctacacacccaagacccgccgggaggcagaggacctgcaggtggggcaggtggagctgggcgggggccctggtgcaggcagcctgcagcccttggccctggaggggtccctgcagaagcgtggcattgtggaacaatgctgtaccagcatctgctccctctaccagctggagaactactgcaactag

SEQ ID NO: 9 - DNA, 333 bp, synthetic construct; identical to SEQ ID NO: 8
  source 1..333: mol_type = other DNA; note = hPPI COMPETITOR_ CDS

SEQ ID NO: 10 - DNA, 513 bp, synthetic construct
  source 1..513: mol_type = other DNA; note = Nanoluc luciferase reporter sequence
atggtcttcacactcgaagatttcgttggggactggcgacagacagccggctacaacctggaccaagtccttgaacagggaggtgtgtccagtttgtttcagaatctcggggtgtccgtaactccgatccaaaggattgtcctgagcggtgaaaatgggctgaagatcgacatccatgtcatcatcccgtatgaaggtctgagcggcgaccaaatgggccagatcgaaaaaatttttaaggtggtgtaccctgtggatgatcatcactttaaggtgatcctgcactatggcacactggtaatcgacggggttacgccgaacatgatcgactatttcggacggccgtatgaaggcatcgccgtgttcgacggcaaaaagatcactgtaacagggaccctgtggaacggcaacaaaattatcgacgagcgcctgatcaaccccgacggctccctgctgttccgagtaaccatcaacggagtgaccggctggcggctgtgcgaacgcattctggcg

SEQ ID NO: 11 - DNA, 837 bp, synthetic construct
  source 1..837: mol_type = other DNA; note = Insulin B NLuc Delta B24-30
atggccctgtggatgcgcctcctgcccctgctggcgctgctggccctctggggacctgacccagccgcagcctttgtgaaccaacacctgtgcggctcacacctggtggaagctctctacctagtgtgcggggaacgaggcatggtcttcacactcgaagatttcgttggggactggcgacagacagccggctacaacctggaccaagtccttgaacagggaggtgtgtccagtttgtttcagaatctcggggtgtccgtaactccgatccaaaggattgtcctgagcggtgaaaatgggctgaagatcgacatccatgtcatcatcccgtatgaaggtctgagcggcgaccaaatgggccagatcgaaaaaatttttaaggtggtgtaccctgtggatgatcatcactttaaggtgatcctgcactatggcacactggtaatcgacggggttacgccgaacatgatcgactatttcggacggccgtatgaaggcatcgccgtgttcgacggcaaaaagatcactgtaacagggaccctgtggaacggcaacaaaattatcgacgagcgcctgatcaaccccgacggctccctgctgttccgagtaaccatcaacggagtgaccggctggcggctgtgcgaacgcattctggcggctgctgctgcgcgccggaagcgggaggacctgcaggtggggcaggtggagctgggcgggggcccaggcgcaggcagcctgcagcccttggccctggaggggtcccgacgcaagcgtggcattgtggaacaatgctgtaccagcatctgctccctctaccagctggagaactactgcaactag

SEQ ID NO: 12 - DNA, 840 bp, synthetic construct
  source 1..840: mol_type = other DNA; note = Insulin B NLuc Delta B25-30
atggccctgtggatgcgcctcctgcccctgctggcgctgctggccctctggggacctgacccagccgcagcctttgtgaaccaacacctgtgcggctcacacctggtggaagctctctacctagtgtgcggggaacgaggcttcatggtcttcacactcgaagatttcgttggggactggcgacagacagccggctacaacctggaccaagtccttgaacagggaggtgtgtccagtttgtttcagaatctcggggtgtccgtaactccgatccaaaggattgtcctgagcggtgaaaatgggctgaagatcgacatccatgtcatcatcccgtatgaaggtctgagcggcgaccaaatgggccagatcgaaaaaatttttaaggtggtgtaccctgtggatgatcatcactttaaggtgatcctgcactatggcacactggtaatcgacggggttacgccgaacatgatcgactatttcggacggccgtatgaaggcatcgccgtgttcgacggcaaaaagatcactgtaacagggaccctgtggaacggcaacaaaattatcgacgagcgcctgatcaaccccgacggctccctgctgttccgagtaaccatcaacggagtgaccggctggcggctgtgcgaacgcattctggcggctgctgctgcgcgccggaagcgggaggacctgcaggtggggcaggtggagctgggcgggggcccaggcgcaggcagcctgcagcccttggccctggaggggtcccgacgcaagcgtggcattgtggaacaatgctgtaccagcatctgctccctctaccagctggagaactactgcaactag

SEQ ID NO: 13 - DNA, 843 bp, synthetic construct
  source 1..843: mol_type = other DNA; note = Insulin B NLuc Delta B26-30
atggccctgtggatgcgcctcctgcccctgctggcgctgctggccctctggggacctgacccagccgcagcctttgtgaaccaacacctgtgcggctcacacctggtggaagctctctacctagtgtgcggggaacgaggcttcttcatggtcttcacactcgaagatttcgttggggactggcgacagacagccggctacaacctggaccaagtccttgaacagggaggtgtgtccagtttgtttcagaatctcggggtgtccgtaactccgatccaaaggattgtcctgagcggtgaaaatgggctgaagatcgacatccatgtcatcatcccgtatgaaggtctgagcggcgaccaaatgggccagatcgaaaaaatttttaaggtggtgtaccctgtggatgatcatcactttaaggtgatcctgcactatggcacactggtaatcgacggggttacgccgaacatgatcgactatttcggacggccgtatgaaggcatcgccgtgttcgacggcaaaaagatcactgtaacagggaccctgtggaacggcaacaaaattatcgacgagcgcctgatcaaccccgacggctccctgctgttccgagtaaccatcaacggagtgaccggctggcggctgtgcgaacgcattctggcggctgctgctgcgcgccggaagcgggaggacctgcaggtggggcaggtggagctgggcgggggcccaggcgcaggcagcctgcagcccttggccctggaggggtcccgacgcaagcgtggcattgtggaacaatgctgtaccagcatctgctccctctaccagctggagaactactgcaactag

SEQ ID NO: 14 - DNA, 846 bp, synthetic construct
  source 1..846: mol_type = other DNA; note = Insulin B NLuc Delta B27-30
atggccctgtggatgcgcctcctgcccctgctggcgctgctggccctctggggacctgacccagccgcagcctttgtgaaccaacacctgtgcggctcacacctggtggaagctctctacctagtgtgcggggaacgaggcttcttctacatggtcttcacactcgaagatttcgttggggactggcgacagacagccggctacaacctggaccaagtccttgaacagggaggtgtgtccagtttgtttcagaatctcggggtgtccgtaactccgatccaaaggattgtcctgagcggtgaaaatgggctgaagatcgacatccatgtcatcatcccgtatgaaggtctgagcggcgaccaaatgggccagatcgaaaaaatttttaaggtggtgtaccctgtggatgatcatcactttaaggtgatcctgcactatggcacactggtaatcgacggggttacgccgaacatgatcgactatttcggacggccgtatgaaggcatcgccgtgttcgacggcaaaaagatcactgtaacagggaccctgtggaacggcaacaaaattatcgacgagcgcctgatcaaccccgacggctccctgctgttccgagtaaccatcaacggagtgaccggctggcggctgtgcgaacgcattctggcggctgctgctgcgcgccggaagcgggaggacctgcaggtggggcaggtggagctgggcgggggcccaggcgcaggcagcctgcagcccttggccctggaggggtcccgacgcaagcgtggcattgtggaacaatgctgtaccagcatctgctccctctaccagctggagaactactgcaactag

SEQ ID NO: 15 - DNA, 849 bp, synthetic construct
  source 1..849: mol_type = other DNA; note = Insulin B NLuc Delta B28-30
atggccctgtggatgcgcctcctgcccctgctggcgctgctggccctctggggacctgacccagccgcagcctttgtgaaccaacacctgtgcggctcacacctggtggaagctctctacctagtgtgcggggaacgaggcttcttctacacaatggtcttcacactcgaagatttcgttggggactggcgacagacagccggctacaacctggaccaagtccttgaacagggaggtgtgtccagtttgtttcagaatctcggggtgtccgtaactccgatccaaaggattgtcctgagcggtgaaaatgggctgaagatcgacatccatgtcatcatcccgtatgaaggtctgagcggcgaccaaatgggccagatcgaaaaaatttttaaggtggtgtaccctgtggatgatcatcactttaaggtgatcctgcactatggcacactggtaatcgacggggttacgccgaacatgatcgactatttcggacggccgtatgaaggcatcgccgtgttcgacggcaaaaagatcactgtaacagggaccctgtggaacggcaacaaaattatcgacgagcgcctgatcaaccccgacggctccctgctgttccgagtaaccatcaacggagtgaccggctggcggctgtgcgaacgcattctggcggctgctgctgcgcgccggaagcgggaggacctgcaggtggggcaggtggagctgggcgggggcccaggcgcaggcagcctgcagcccttggccctggaggggtcccgacgcaagcgtggcattgtggaacaatgctgtaccagcatctgctccctctaccagctggagaactactgcaactag

SEQ ID NO: 16 - DNA, 864 bp, synthetic construct
  source 1..864: mol_type = other DNA; note = Insulin B NLuc mut A E17A
atggccctgtggatgcgcctcctgcccctgctggcgctgctggccctctggggacctgacccagccgcagcctttgtgaaccaacacctgtgcggctcacacctggtggaagctctctacctagtgtgcggggaacgaggcttcttctacacacccaagaccatggtcttcacactcgaagatttcgttggggactggcgacagacagccggctacaacctggaccaagtccttgaacagggaggtgtgtccagtttgtttcagaatctcggggtgtccgtaactccgatccaaaggattgtcctgagcggtgaaaatgggctgaagatcgacatccatgtcatcatcccgtatgaaggtctgagcggcgaccaaatgggccagatcgaaaaaatttttaaggtggtgtaccctgtggatgatcatcactttaaggtgatcctgcactatggcacactggtaatcgacggggttacgccgaacatgatcgactatttcggacggccgtatgaaggcatcgccgtgttcgacggcaaaaagatcactgtaacagggaccctgtggaacggcaacaaaattatcgacgagcgcctgatcaaccccgacggctccctgctgttccgagtaaccatcaacggagtgaccggctggcggctgtgcgaacgcattctggcggctgctgctgcgcgccggaagcgggaggacctgcaggtggggcaggtggagctgggcgggggcccaggccctggtgcaggcagcctgcagcccttggccctggaggggtcccgacgcaagcgtggcattgtggaacaatgctgtaccagcatctgctccctctaccagctggcgaactactgcaactag

SEQ ID NO: 17 - DNA, 864 bp, synthetic construct
  source 1..864: mol_type = other DNA; note = Insulin B NLuc mut A L13A
atggccctgtggatgcgcctcctgcccctgctggcgctgctggccctctggggacctgacccagccgcagcctttgtgaaccaacacctgtgcggctcacacctggtggaagctctctacctagtgtgcggggaacgaggcttcttctacacacccaagaccatggtcttcacactcgaagatttcgttggggactggcgacagacagccggctacaacctggaccaagtccttgaacagggaggtgtgtccagtttgtttcagaatctcggggtgtccgtaactccgatccaaaggattgtcctgagcggtgaaaatgggctgaagatcgacatccatgtcatcatcccgtatgaaggtctgagcggcgaccaaatgggccagatcgaaaaaatttttaaggtggtgtaccctgtggatgatcatcactttaaggtgatcctgcactatggcacactggtaatcgacggggttacgccgaacatgatcgactatttcggacggccgtatgaaggcatcgccgtgttcgacggcaaaaagatcactgtaacagggaccctgtggaacggcaacaaaattatcgacgagcgcctgatcaaccccgacggctccctgctgttccgagtaaccatcaacggagtgaccggctggcggctgtgcgaacgcattctggcggctgctgctgcgcgccggaagcgggaggacctgcaggtggggcaggtggagctgggcgggggcccaggccctggtgcaggcagcctgcagcccttggccctggaggggtcccgacgcaagcgtggcattgtggaacaatgctgtaccagcatctgctccgcctaccagctggagaactactgcaactag

SEQ ID NO: 18 - DNA, 864 bp, synthetic construct
  source 1..864: mol_type = other DNA; note = Insulin B NLuc mut A L13W
atggccctgtggatgcgcctcctgcccctgctggcgctgctggccctctggggacctgacccagccgcagcctttgtgaaccaacacctgtgcggctcacacctggtggaagctctctacctagtgtgcggggaacgaggcttcttctacacacccaagaccatggtcttcacactcgaagatttcgttggggactggcgacagacagccggctacaacctggaccaagtccttgaacagggaggtgtgtccagtttgtttcagaatctcggggtgtccgtaactccgatccaaaggattgtcctgagcggtgaaaatgggctgaagatcgacatccatgtcatcatcccgtatgaaggtctgagcggcgaccaaatgggccagatcgaaaaaatttttaaggtggtgtaccctgtggatgatcatcactttaaggtgatcctgcactatggcacactggtaatcgacggggttacgccgaacatgatcgactatttcggacggccgtatgaaggcatcgccgtgttcgacggcaaaaagatcactgtaacagggaccctgtggaacggcaacaaaattatcgacgagcgcctgatcaaccccgacggctccctgctgttccgagtaaccatcaacggagtgaccggctggcggctgtgcgaacgcattctggcggctgctgctgcgcgccggaagcgggaggacctgcaggtggggcaggtggagctgggcgggggcccaggccctggtgcaggcagcctgcagcccttggccctggaggggtcccgacgcaagcgtggcattgtggaacaatgctgtaccagcatctgctcctggtaccagctggagaactactgcaactag

SEQ ID NO: 19 - DNA, 864 bp, synthetic construct
  source 1..864: mol_type = other DNA; note = Insulin B NLuc mut A Y14A
atggccctgtggatgcgcctcctgcccctgctggcgctgctggccctctggggacctgacccagccgcagcctttgtgaaccaacacctgtgcggctcacacctggtggaagctctctacctagtgtgcggggaacgaggcttcttctacacacccaagaccatggtcttcacactcgaagatttcgttggggactggcgacagacagccggctacaacctggaccaagtccttgaacagggaggtgtgtccagtttgtttcagaatctcggggtgtccgtaactccgatccaaaggattgtcctgagcggtgaaaatgggctgaagatcgacatccatgtcatcatcccgtatgaaggtctgagcggcgaccaaatgggccagatcgaaaaaatttttaaggtggtgtaccctgtggatgatcatcactttaaggtgatcctgcactatggcacactggtaatcgacggggttacgccgaacatgatcgactatttcggacggccgtatgaaggcatcgccgtgttcgacggcaaaaagatcactgtaacagggaccctgtggaacggcaacaaaattatcgacgagcgcctgatcaaccccgacggctccctgctgttccgagtaaccatcaacggagtgaccggctggcggctgtgcgaacgcattctggcggctgctgctgcgcgccggaagcgggaggacctgcaggtggggcaggtggagctgggcgggggcccaggccctggtgcaggcagcctgcagcccttggccctggaggggtcccgacgcaagcgtggcattgtggaacaatgctgtaccagcatctgctccctcgcccagctggagaactactgcaactag

SEQ ID NO: 20 - DNA, 864 bp, synthetic construct
  source 1..864: mol_type = other DNA; note = Insulin B NLuc mut B F1A
atggccctgtggatgcgcctcctgcccctgctggcgctgctggccctctggggacctgacccagccgcagccgctgtgaaccaacacctgtgcggctcacacctggtggaagctctctacctagtgtgcggggaacgaggcttcttctacacacccaagaccatggtcttcacactcgaagatttcgttggggactggcgacagacagccggctacaacctggaccaagtccttgaacagggaggtgtgtccagtttgtttcagaatctcggggtgtccgtaactccgatccaaaggattgtcctgagcggtgaaaatgggctgaagatcgacatccatgtcatcatcccgtatgaaggtctgagcggcgaccaaatgggccagatcgaaaaaatttttaaggtggtgtaccctgtggatgatcatcactttaaggtgatcctgcactatggcacactggtaatcgacggggttacgccgaacatgatcgactatttcggacggccgtatgaaggcatcgccgtgttcgacggcaaaaagatcactgtaacagggaccctgtggaacggcaacaaaattatcgacgagcgcctgatcaaccccgacggctccctgctgttccgagtaaccatcaacggagtgaccggctggcggctgtgcgaacgcattctggcggctgctgctgcgcgccggaagcgggaggacctgcaggtggggcaggtggagctgggcgggggcccaggccctggtgcaggcagcctgcagcccttggccctggaggggtcccgacgcaagcgtggcattgtggaacaatgctgtaccagcatctgctccctctaccagctggagaactactgcaactag

SEQ ID NO: 21 - DNA, 864 bp, synthetic construct
  source 1..864: mol_type = other DNA; note = Insulin B NLuc mut B F25D
atggccctgtggatgcgcctcctgcccctgctggcgctgctggccctctggggacctgacccagccgcagcctttgtgaaccaacacctgtgcggctcacacctggtggaagctctctacctagtgtgcggggaacgaggcttcgactacacacccaagaccatggtcttcacactcgaagatttcgttggggactggcgacagacagccggctacaacctggaccaagtccttgaacagggaggtgtgtccagtttgtttcagaatctcggggtgtccgtaactccgatccaaaggattgtcctgagcggtgaaaatgggctgaagatcgacatccatgtcatcatcccgtatgaaggtctgagcggcgaccaaatgggccagatcgaaaaaatttttaaggtggtgtaccctgtggatgatcatcactttaaggtgatcctgcactatggcacactggtaatcgacggggttacgccgaacatgatcgactatttcggacggccgtatgaaggcatcgccgtgttcgacggcaaaaagatcactgtaacagggaccctgtggaacggcaacaaaattatcgacgagcgcctgatcaaccccgacggctccctgctgttccgagtaaccatcaacggagtgaccggctggcggctgtgcgaacgcattctggcggctgctgctgcgcgccggaagcgggaggacctgcaggtggggcaggtggagctgggcgggggcccaggccctggtgcaggcagcctgcagcccttggccctggaggggtcccgacgcaagcgtggcattgtggaacaatgctgtaccagcatctgctccctctaccagctggagaactactgcaactag

SEQ ID NO: 22 - DNA, 864 bp, synthetic construct
  source 1..864: mol_type = other DNA; note = Insulin B NLuc mut B L17A V18A
atggccctgtggatgcgcctcctgcccctgctggcgctgctggccctctggggacctgacccagccgcagcctttgtgaaccaacacctgtgcggctcacacctggtggaagctctctacgcagcgtgcggggaacgaggcttcttctacacacccaagaccatggtcttcacactcgaagatttcgttggggactggcgacagacagccggctacaacctggaccaagtccttgaacagggaggtgtgtccagtttgtttcagaatctcggggtgtccgtaactccgatccaaaggattgtcctgagcggtgaaaatgggctgaagatcgacatccatgtcatcatcccgtatgaaggtctgagcggcgaccaaatgggccagatcgaaaaaatttttaaggtggtgtaccctgtggatgatcatcactttaaggtgatcctgcactatggcacactggtaatcgacggggttacgccgaacatgatcgactatttcggacggccgtatgaaggcatcgccgtgttcgacggcaaaaagatcactgtaacagggaccctgtggaacggcaacaaaattatcgacgagcgcctgatcaaccccgacggctccctgctgttccgagtaaccatcaacggagtgaccggctggcggctgtgcgaacgcattctggcggctgctgctgcgcgccggaagcgggaggacctgcaggtggggcaggtggagctgggcgggggcccaggccctggtgcaggcagcctgcagcccttggccctggaggggtcccgacgcaagcgtggcattgtggaacaatgctgtaccagcatctgctccctctaccagctggagaactactgcaactag

SEQ ID NO: 23 - DNA, 864 bp, synthetic construct
  source 1..864: mol_type = other DNA; note = Insulin B NLuc mut B L17A
atggccctgtggatgcgcctcctgcccctgctggcgctgctggccctctggggacctgacccagccgcagcctttgtgaaccaacacctgtgcggctcacacctggtggaagctctctacgcagtgtgcggggaacgaggcttcttctacacacccaagaccatggtcttcacactcgaagatttcgttggggactggcgacagacagccggctacaacctggaccaagtccttgaacagggaggtgtgtccagtttgtttcagaatctcggggtgtccgtaactccgatccaaaggattgtcctgagcggtgaaaatgggctgaagatcgacatccatgtcatcatcccgtatgaaggtctgagcggcgaccaaatgggccagatcgaaaaaatttttaaggtggtgtaccctgtggatgatcatcactttaaggtgatcctgcactatggcacactggtaatcgacggggttacgccgaacatgatcgactatttcggacggccgtatgaaggcatcgccgtgttcgacggcaaaaagatcactgtaacagggaccctgtggaacggcaacaaaattatcgacgagcgcctgatcaaccccgacggctccctgctgttccgagtaaccatcaacggagtgaccggctggcggctgtgcgaacgcattctggcggctgctgctgcgcgccggaagcgggaggacctgcaggtggggcaggtggagctgggcgggggcccaggccctggtgcaggcagcctgcagcccttggccctggaggggtcccgacgcaagcgtggcattgtggaacaatgctgtaccagcatctgctccctctaccagctggagaactactgcaactag

SEQ ID NO: 24 - DNA, 864 bp, synthetic construct
  source 1..864: mol_type = other DNA; note = Insulin B NLuc mut B R22A
atggccctgtggatgcgcctcctgcccctgctggcgctgctggccctctggggacctgacccagccgcagcctttgtgaaccaacacctgtgcggctcacacctggtggaagctctctacctagtgtgcggggaagcaggcttcttctacacacccaagaccatggtcttcacactcgaagatttcgttggggactggcgacagacagccggctacaacctggaccaagtccttgaacagggaggtgtgtccagtttgtttcagaatctcggggtgtccgtaactccgatccaaaggattgtcctgagcggtgaaaatgggctgaagatcgacatccatgtcatcatcccgtatgaaggtctgagcggcgaccaaatgggccagatcgaaaaaatttttaaggtggtgtaccctgtggatgatcatcactttaaggtgatcctgcactatggcacactggtaatcgacggggttacgccgaacatgatcgactatttcggacggccgtatgaaggcatcgccgtgttcgacggcaaaaagatcactgtaacagggaccctgtggaacggcaacaaaattatcgacgagcgcctgatcaaccccgacggctccctgctgttccgagtaaccatcaacggagtgaccggctggcggctgtgcgaacgcattctggcggctgctgctgcgcgccggaagcgggaggacctgcaggtggggcaggtggagctgggcgggggcccaggccctggtgcaggcagcctgcagcccttggccctggaggggtcccgacgcaagcgtggcattgtggaacaatgctgtaccagcatctgctccctctaccagctggagaactactgcaactag

SEQ ID NO: 25 - DNA, 864 bp, synthetic construct
  source 1..864: mol_type = other DNA; note = Insulin B NLuc mut B S9P
atggccctgtggatgcgcctcctgcccctgctggcgctgctggccctctggggacctgacccagccgcagcctttgtgaaccaacacctgtgcggcccccacctggtggaagctctctacctagtgtgcggggaacgaggcttcttctacacacccaagaccatggtcttcacactcgaagatttcgttggggactggcgacagacagccggctacaacctggaccaagtccttgaacagggaggtgtgtccagtttgtttcagaatctcggggtgtccgtaactccgatccaaaggattgtcctgagcggtgaaaatgggctgaagatcgacatccatgtcatcatcccgtatgaaggtctgagcggcgaccaaatgggccagatcgaaaaaatttttaaggtggtgtaccctgtggatgatcatcactttaaggtgatcctgcactatggcacactggtaatcgacggggttacgccgaacatgatcgactatttcggacggccgtatgaaggcatcgccgtgttcgacggcaaaaagatcactgtaacagggaccctgtggaacggcaacaaaattatcgacgagcgcctgatcaaccccgacggctccctgctgttccgagtaaccatcaacggagtgaccggctggcggctgtgcgaacgcattctggcggctgctgctgcgcgccggaagcgggaggacctgcaggtggggcaggtggagctgggcgggggcccaggccctggtgcaggcagcctgcagcccttggccctggaggggtcccgacgcaagcgtggcattgtggaacaatgctgtaccagcatctgctccctctaccagctggagaactactgcaactag

SEQ ID NO: 26 - DNA, 864 bp, synthetic construct
  source 1..864: mol_type = other DNA; note = Insulin B NLuc mut B V18A
atggccctgtggatgcgcctcctgcccctgctggcgctgctggccctctggggacctgacccagccgcagcctttgtgaaccaacacctgtgcggctcacacctggtggaagctctctacctagcgtgcggggaacgaggcttcttctacacacccaagaccatggtcttcacactcgaagatttcgttggggactggcgacagacagccggctacaacctggaccaagtccttgaacagggaggtgtgtccagtttgtttcagaatctcggggtgtccgtaactccgatccaaaggattgtcctgagcggtgaaaatgggctgaagatcgacatccatgtcatcatcccgtatgaaggtctgagcggcgaccaaatgggccagatcgaaaaaatttttaaggtggtgtaccctgtggatgatcatcactttaaggtgatcctgcactatggcacactggtaatcgacggggttacgccgaacatgatcgactatttcggacggccgtatgaaggcatcgccgtgttcgacggcaaaaagatcactgtaacagggaccctgtggaacggcaacaaaattatcgacgagcgcctgatcaaccccgacggctccctgctgttccgagtaaccatcaacggagtgaccggctggcggctgtgcgaacgcattctggcggctgctgctgcgcgccggaagcgggaggacctgcaggtggggcaggtggagctgggcgggggcccaggccctggtgcaggcagcctgcagcccttggccctggaggggtcccgacgcaagcgtggcattgtggaacaatgctgtaccagcatctgctccctctaccagctggagaactactgcaactag

SEQ ID NO: 27 - DNA, 864 bp, synthetic construct
  source 1..864: mol_type = other DNA; note = Insulin B NLuc mut B V2G
atggccctgtggatgcgcctcctgcccctgctggcgctgctggccctctggggacctgacccagccgcagcctttgggaaccaacacctgtgcggctcacacctggtggaagctctctacctagtgtgcggggaacgaggcttcttctacacacccaagaccatggtcttcacactcgaagatttcgttggggactggcgacagacagccggctacaacctggaccaagtccttgaacagggaggtgtgtccagtttgtttcagaatctcggggtgtccgtaactccgatccaaaggattgtcctgagcggtgaaaatgggctgaagatcgacatccatgtcatcatcccgtatgaaggtctgagcggcgaccaaatgggccagatcgaaaaaatttttaaggtggtgtaccctgtggatgatcatcactttaaggtgatcctgcactatggcacactggtaatcgacggggttacgccgaacatgatcgactatttcggacggccgtatgaaggcatcgccgtgttcgacggcaaaaagatcactgtaacagggaccctgtggaacggcaacaaaattatcgacgagcgcctgatcaaccccgacggctccctgctgttccgagtaaccatcaacggagtgaccggctggcggctgtgcgaacgcattctggcggctgctgctgcgcgccggaagcgggaggacctgcaggtggggcaggtggagctgggcgggggcccaggccctggtgcaggcagcctgcagcccttggccctggaggggtcccgacgcaagcgtggcattgtggaacaatgctgtaccagcatctgctccctctaccagctggagaactactgcaactag

SEQ ID NO: 28 - DNA, 840 bp, synthetic construct
  source 1..840: mol_type = other DNA; note = Insulin NLuc A Delta B25-30
atggccctgtggatgcgcctcctgcccctgctggcgctgctggccctctggggacctgacccagccgcagcctttgtgaaccaacacctgtgcggctcacacctggtggaagctctctacctagtgtgcggggaacgaggcttccgccggaagcgggaggacctgcaggtggggcaggtggagctgggcgggggcccaggcgcaggcagcctgcagcccttggccctggaggggtcccgacgcaagcgtatggtcttcacactcgaagatttcgttggggactggcgacagacagccggctacaacctggaccaagtccttgaacagggaggtgtgtccagtttgtttcagaatctcggggtgtccgtaactccgatccaaaggattgtcctgagcggtgaaaatgggctgaagatcgacatccatgtcatcatcccgtatgaaggtctgagcggcgaccaaatgggccagatcgaaaaaatttttaaggtggtgtaccctgtggatgatcatcactttaaggtgatcctgcactatggcacactggtaatcgacggggttacgccgaacatgatcgactatttcggacggccgtatgaaggcatcgccgtgttcgacggcaaaaagatcactgtaacagggaccctgtggaacggcaacaaaattatcgacgagcgcctgatcaaccccgacggctccctgctgttccgagtaaccatcaacggagtgaccggctggcggctgtgcgaacgcattctggcggctgctgctgcgggcattgtggaacaatgctgtaccagcatctgctccctctaccagctggagaactactgcaactag

SEQ ID NO: 29 - DNA, 849 bp, synthetic construct
  source 1..849: mol_type = other DNA; note = Insulin NLuc A Delta B26-30
atggccctgtggatgcgcctcctgcccctgctggcgctgctggccctctggggacctgacccagccgcagcctttgtgaaccaacacctgtgcggctcacacctggtggaagctctctacctagtgtgcggggaacgaggcttcttccgccggaagcgggaggacctgcaggtggggcaggtggagctgggcgggggcccaggccctggtgcaggcagcctgcagcccttggccctggaggggtcccgacgcaagcgtatggtcttcacactcgaagatttcgttggggactggcgacagacagccggctacaacctggaccaagtccttgaacagggaggtgtgtccagtttgtttcagaatctcggggtgtccgtaactccgatccaaaggattgtcctgagcggtgaaaatgggctgaagatcgacatccatgtcatcatcccgtatgaaggtctgagcggcgaccaaatgggccagatcgaaaaaatttttaaggtggtgtaccctgtggatgatcatcactttaaggtgatcctgcactatggcacactggtaatcgacggggttacgccgaacatgatcgactatttcggacggccgtatgaaggcatcgccgtgttcgacggcaaaaagatcactgtaacagggaccctgtggaacggcaacaaaattatcgacgagcgcctgatcaaccccgacggctccctgctgttccgagtaaccatcaacggagtgaccggctggcggctgtgcgaacgcattctggcggctgctgctgcgggcattgtggaacaatgctgtaccagcatctgctccctctaccagctggagaactactgcaactag

SEQ ID NO: 30 - DNA, 852 bp, synthetic construct
  source 1..852: mol_type = other DNA; note = Insulin NLuc A Delta B27-30
atggccctgtggatgcgcctcctgcccctgctggcgctgctggccctctggggacctgacccagccgcagcctttgtgaaccaacacctgtgcggctcacacctggtggaagctctctacctagtgtgcggggaacgaggcttcttctaccgccggaagcgggaggacctgcaggtggggcaggtggagctgggcgggggcccaggccctggtgcaggcagcctgcagcccttggccctggaggggtcccgacgcaagcgtatggtcttcacactcgaagatttcgttggggactggcgacagacagccggctacaacctggaccaagtccttgaacagggaggtgtgtccagtttgtttcagaatctcggggtgtccgtaactccgatccaaaggattgtcctgagcggtgaaaatgggctgaagatcgacatccatgtcatcatcccgtatgaaggtctgagcggcgaccaaatgggccagatcgaaaaaatttttaaggtggtgtaccctgtggatgatcatcactttaaggtgatcctgcactatggcacactggtaatcgacggggttacgccgaacatgatcgactatttcggacggccgtatgaaggcatcgccgtgttcgacggcaaaaagatcactgtaacagggaccctgtggaacggcaacaaaattatcgacgagcgcctgatcaaccccgacggctccctgctgttccgagtaaccatcaacggagtgaccggctggcggctgtgcgaacgcattctggcggctgctgctgcgggcattgtggaacaatgctgtaccagcatctgctccctctaccagctggagaactactgcaactag

SEQ ID NO: 31 - DNA, 855 bp, synthetic construct
  source 1..855: mol_type = other DNA; note = Insulin NLuc A Delta B28-30
atggccctgtggatgcgcctcctgcccctgctggcgctgctggccctctggggacctgacccagccgcagcctttgtgaaccaacacctgtgcggctcacacctggtggaagctctctacctagtgtgcggggaacgaggcttcttctacacacgccggaagcgggaggacctgcaggtggggcaggtggagctgggcgggggcccaggccctggtgcaggcagcctgcagcccttggccctggaggggtcccgacgcaagcgtatggtcttcacactcgaagatttcgttggggactggcgacagacagccggctacaacctggaccaagtccttgaacagggaggtgtgtccagtttgtttcagaatctcggggtgtccgtaactccgatccaaaggattgtcctgagcggtgaaaatgggctgaagatcgacatccatgtcatcatcccgtatgaaggtctgagcggcgaccaaatgggccagatcgaaaaaatttttaaggtggtgtaccctgtggatgatcatcactttaaggtgatcctgcactatggcacactggtaatcgacggggttacgccgaacatgatcgactatttcggacggccgtatgaaggcatcgccgtgttcgacggcaaaaagatcactgtaacagggaccctgtggaacggcaacaaaattatcgacgagcgcctgatcaaccccgacggctccctgctgttccgagtaaccatcaacggagtgaccggctggcggctgtgcgaacgcattctggcggctgctgctgcgggcattgtggaacaatgctgtaccagcatctgctccctctaccagctggagaactactgcaactag

SEQ ID NO: 32 - DNA, 861 bp, synthetic construct
  source 1..861: mol_type = other DNA; note = Insulin NLuc A Delta B30
atggccctgtggatgcgcctcctgcccctgctggcgctgctggccctctggggacctgacccagccgcagcctttgtgaaccaacacctgtgcggctcacacctggtggaagctctctacctagtgtgcggggaacgaggcttcttctacacacccaagcgccggaagcgggaggacctgcaggtggggcaggtggagctgggcgggggcccaggccctggtgcaggcagcctgcagcccttggccctggaggggtcccgacgcaagcgtatggtcttcacactcgaagatttcgttggggactggcgacagacagccggctacaacctggaccaagtccttgaacagggaggtgtgtccagtttgtttcagaatctcggggtgtccgtaactccgatccaaaggattgtcctgagcggtgaaaatgggctgaagatcgacatccatgtcatcatcccgtatgaaggtctgagcggcgaccaaatgggccagatcgaaaaaatttttaaggtggtgtaccctgtggatgatcatcactttaaggtgatcctgcactatggcacactggtaatcgacggggttacgccgaacatgatcgactatttcggacggccgtatgaaggcatcgccgtgttcgacggcaaaaagatcactgtaacagggaccctgtggaacggcaacaaaattatcgacgagcgcctgatcaaccccgacggctccctgctgttccgagtaaccatcaacggagtgaccggctggcggctgtgcgaacgcattctggcggctgctgctgcgggcattgtggaacaatgctgtaccagcatctgctccctctaccagctggagaactactgcaactag

SEQ ID NO: 33 - DNA, 864 bp, synthetic construct
  source 1..864: mol_type = other DNA; note = Insulin NLuc A mut A L13A
atggccctgtggatgcgcctcctgcccctgctggcgctgctggccctctggggacctgacccagccgcagcctttgtgaaccaacacctgtgcggctcacacctggtggaagctctctacctagtgtgcggggaacgaggcttcttctacacacccaagacccgccggaagcgggaggacctgcaggtggggcaggtggagctgggcgggggcccaggccctggtgcaggcagcctgcagcccttggccctggaggggtcccgacgcaagcgtatggtcttcacactcgaagatttcgttggggactggcgacagacagccggctacaacctggaccaagtccttgaacagggaggtgtgtccagtttgtttcagaatctcggggtgtccgtaactccgatccaaaggattgtcctgagcggtgaaaatgggctgaagatcgacatccatgtcatcatcccgtatgaaggtctgagcggcgaccaaatgggccagatcgaaaaaatttttaaggtggtgtaccctgtggatgatcatcactttaaggtgatcctgcactatggcacactggtaatcgacggggttacgccgaacatgatcgactatttcggacggccgtatgaaggcatcgccgtgttcgacggcaaaaagatcactgtaacagggaccctgtggaacggcaacaaaattatcgacgagcgcctgatcaaccccgacggctccctgctgttccgagtaaccatcaacggagtgaccggctggcggctgtgcgaacgcattctggcggctgctgctgcgggcattgtggaacaatgctgtaccagcatctgctccgcctaccagctggagaactactgcaactag

SEQ ID NO: 34 - DNA, 864 bp, synthetic construct
  source 1..864: mol_type = other DNA; note = Insulin NLuc A mut A L13W
atggccctgtggatgcgcctcctgcccctgctggcgctgctggccctctggggacctgacccagccgcagcctttgtgaaccaacacctgtgcggctcacacctggtggaagctctctacctagtgtgcggggaacgaggcttcttctacacacccaagacccgccggaagcgggaggacctgcaggtggggcaggtggagctgggcgggggcccaggccctggtgcaggcagcctgcagcccttggccctggaggggtcccgacgcaagcgtatggtcttcacactcgaagatttcgttggggactggcgacagacagccggctacaacctggaccaagtccttgaacagggaggtgtgtccagtttgtttcagaatctcggggtgtccgtaactccgatccaaaggattgtcctgagcggtgaaaatgggctgaagatcgacatccatgtcatcatcccgtatgaaggtctgagcggcgaccaaatgggccagatcgaaaaaatttttaaggtggtgtaccctgtggatgatcatcactttaaggtgatcctgcactatggcacactggtaatcgacggggttacgccgaacatgatcgactatttcggacggccgtatgaaggcatcgccgtgttcgacggcaaaaagatcactgtaacagggaccctgtggaacggcaacaaaattatcgacgagcgcctgatcaaccccgacggctccctgctgttccgagtaaccatcaacggagtgaccggctggcggctgtgcgaacgcattctggcggctgctgctgcgggcattgtggaacaatgctgtaccagcatctgctcctggtaccagctggagaactactgcaactag

SEQ ID NO: 35 - DNA, 864 bp, synthetic construct
  source 1..864: mol_type = other DNA; note = Insulin NLuc A mut B F1A
atggccctgtggatgcgcctcctgcccctgctggcgctgctggccctctggggacctgacccagccgcagccgctgtgaaccaacacctgtgcggctcacacctggtggaagctctctacctagtgtgcggggaacgaggcttcttctacacacccaagacccgccggaagcgggaggacctgcaggtggggcaggtggagctgggcgggggcccaggccctggtgcaggcagcctgcagcccttggccctggaggggtcccgacgcaagcgtatggtcttcacactcgaagatttcgttggggactggcgacagacagccggctacaacctggaccaagtccttgaacagggaggtgtgtccagtttgtttcagaatctcggggtgtccgtaactccgatccaaaggattgtcctgagcggtgaaaatgggctgaagatcgacatccatgtcatcatcccgtatgaaggtctgagcggcgaccaaatgggccagatcgaaaaaatttttaaggtggtgtaccctgtggatgatcatcactttaaggtgatcctgcactatggcacactggtaatcgacggggttacgccgaacatgatcgactatttcggacggccgtatgaaggcatcgccgtgttcgacggcaaaaagatcactgtaacagggaccctgtggaacggcaacaaaattatcgacgagcgcctgatcaaccccgacggctccctgctgttccgagtaaccatcaacggagtgaccggctggcggctgtgcgaacgcattctggcggctgctgctgcgggcattgtggaacaatgctgtaccagcatctgctccctctaccagctggagaactactgcaactag

SEQ ID NO: 36 - DNA, 864 bp, synthetic construct
  source 1..864: mol_type = other DNA; note = Insulin NLuc A mut B F25D
atggccctgtggatgcgcctcctgcccctgctggcgctgctggccctctggggacctgacccagccgcagcctttgtgaaccaacacctgtgcggctcacacctggtggaagctctctacctagtgtgcggggaacgaggcttcgactacacacccaagacccgccggaagcgggaggacctgcaggtggggcaggtggagctgggcgggggcccaggccctggtgcaggcagcctgcagcccttggccctggaggggtcccgacgcaagcgtatggtcttcacactcgaagatttcgttggggactggcgacagacagccggctacaacctggaccaagtccttgaacagggaggtgtgtccagtttgtttcagaatctcggggtgtccgtaactccgatccaaaggattgtcctgagcggtgaaaatgggctgaagatcgacatccatgtcatcatcccgtatgaaggtctgagcggcgaccaaatgggccagatcgaaaaaatttttaaggtggtgtaccctgtggatgatcatcactttaaggtgatcctgcactatggcacactggtaatcgacggggttacgccgaacatgatcgactatttcggacggccgtatgaaggcatcgccgtgttcgacggcaaaaagatcactgtaacagggaccctgtggaacggcaacaaaattatcgacgagcgcctgatcaaccccgacggctccctgctgttccgagtaaccatcaacggagtgaccggctggcggctgtgcgaacgcattctggcggctgctgctgcgggcattgtggaacaatgctgtaccagcatctgctccctctaccagctggagaactactgcaactag

SEQ ID NO: 37 - DNA, 864 bp, synthetic construct
  source 1..864: mol_type = other DNA; note = Insulin NLuc A mut B L17A V18A
atggccctgtggatgcgcctcctgcccctgctggcgctgctggccctctggggacctgacccagccgcagcctttgtgaaccaacacctgtgcggctcacacctggtggaagctctctacgcagcgtgcggggaacgaggcttcttctacacacccaagacccgccggaagcgggaggacctgcaggtggggcaggtggagctgggcgggggcccaggccctggtgcaggcagcctgcagcccttggccctggaggggtcccgacgcaagcgtatggtcttcacactcgaagatttcgttggggactggcgacagacagccggctacaacctggaccaagtccttgaacagggaggtgtgtccagtttgtttcagaatctcggggtgtccgtaactccgatccaaaggattgtcctgagcggtgaaaatgggctgaagatcgacatccatgtcatcatcccgtatgaaggtctgagcggcgaccaaatgggccagatcgaaaaaatttttaaggtggtgtaccctgtggatgatcatcactttaaggtgatcctgcactatggcacactggtaatcgacggggttacgccgaacatgatcgactatttcggacggccgtatgaaggcatcgccgtgttcgacggcaaaaagatcactgtaacagggaccctgtggaacggcaacaaaattatcgacgagcgcctgatcaaccccgacggctccctgctgttccgagtaaccatcaacggagtgaccggctggcggctgtgcgaacgcattctggcggctgctgctgcgggcattgtggaacaatgctgtaccagcatctgctccctctaccagctggagaactactgcaactag

SEQ ID NO: 38 - DNA, 864 bp, synthetic construct
  source 1..864: mol_type = other DNA; note = Insulin NLuc A mut B L17A
atggccctgtggatgcgcctcctgcccctgctggcgctgctggccctctggggacctgacccagccgcagcctttgtgaaccaacacctgtgcggctcacacctggtggaagctctctacgcagtgtgcggggaacgaggcttcttctacacacccaagacccgccggaagcgggaggacctgcaggtggggcaggtggagctgggcgggggcccaggccctggtgcaggcagcctgcagcccttggccctggaggggtcccgacgcaagcgtatggtcttcacactcgaagatttcgttggggactggcgacagacagccggctacaacctggaccaagtccttgaacagggaggtgtgtccagtttgtttcagaatctcggggtgtccgtaactccgatccaaaggattgtcctgagcggtgaaaatgggctgaagatcgacatccatgtcatcatcccgtatgaaggtctgagcggcgaccaaatgggccagatcgaaaaaatttttaaggtggtgtaccctgtggatgatcatcactttaaggtgatcctgcactatggcacactggtaatcgacggggttacgccgaacatgatcgactatttcggacggccgtatgaaggcatcgccgtgttcgacggcaaaaagatcactgtaacagggaccctgtggaacggcaacaaaattatcgacgagcgcctgatcaaccccgacggctccctgctgttccgagtaaccatcaacggagtgaccggctggcggctgtgcgaacgcattctggcggctgctgctgcgggcattgtggaacaatgctgtaccagcatctgctccctctaccagctggagaactactgcaactag

SEQ ID NO: 39 - DNA, 864 bp, synthetic construct
  source 1..864: mol_type = other DNA; note = Insulin NLuc A mut B R22A
atggccctgtggatgcgcctcctgcccctgctggcgctgctggccctctggggacctgacccagccgcagcctttgtgaaccaacacctgtgcggctcacacctggtggaagctctctacctagtgtgcggggaacgaggcttcttctacacacccaagacccgccggaagcgggaggacctgcaggtggggcaggtggagctgggcgggggcccaggccctggtgcaggcagcctgcagcccttggccctggaggggtcccgacgcaagcgtatggtcttcacactcgaagatttcgttggggactggcgacagacagccggctacaacctggaccaagtccttgaacagggaggtgtgtccagtttgtttcagaatctcggggtgtccgtaactccgatccaaaggattgtcctgagcggtgaaaatgggctgaagatcgacatccatgtcatcatcccgtatgaaggtctgagcggcgaccaaatgggccagatcgaaaaaatttttaaggtggtgtaccctgtggatgatcatcactttaaggtgatcctgcactatggcacactggtaatcgacggggttacgccgaacatgatcgactatttcggacggccgtatgaaggcatcgccgtgttcgacggcaaaaagatcactgtaacagggaccctgtggaacggcaacaaaattatcgacgagcgcctgatcaaccccgacggctccctgctgttccgagtaaccatcaacggagtgaccggctggcggctgtgcgaacgcattctggcggctgctgctgcgggcattgtggaacaatgctgtaccagcatctgctccctctaccagctggagaactactgcaactag

SEQ ID NO: 40 - DNA, 864 bp, synthetic construct
  source 1..864: mol_type = other DNA; note = Insulin NLuc A mut B V18A
atggccctgtggatgcgcctcctgcccctgctggcgctgctggccctctggggacctgacccagccgcagcctttgtgaaccaacacctgtgcggctcacacctggtggaagctctctacctagcgtgcggggaacgaggcttcttctacacacccaagacccgccggaagcgggaggacctgcaggtggggcaggtggagctgggcgggggcccaggccctggtgcaggcagcctgcagcccttggccctggaggggtcccgacgcaagcgtatggtcttcacactcgaagatttcgttggggactggcgacagacagccggctacaacctggaccaagtccttgaacagggaggtgtgtccagtttgtttcagaatctcggggtgtccgtaactccgatccaaaggattgtcctgagcggtgaaaatgggctgaagatcgacatccatgtcatcatcccgtatgaaggtctgagcggcgaccaaatgggccagatcgaaaaaatttttaaggtggtgtaccctgtggatgatcatcactttaaggtgatcctgcactatggcacactggtaatcgacggggttacgccgaacatgatcgactatttcggacggccgtatgaaggcatcgccgtgttcgacggcaaaaagatcactgtaacagggaccctgtggaacggcaacaaaattatcgacgagcgcctgatcaaccccgacggctccctgctgttccgagtaaccatcaacggagtgaccggctggcggctgtgcgaacgcattctggcggctgctgctgcgggcattgtggaacaatgctgtaccagcatctgctccctctaccagctggagaactactgcaactag

SEQ ID NO: 41 - DNA, 864 bp, synthetic construct
  source 1..864: mol_type = other DNA; note = Insulin NLuc A mut B V2G
atggccctgtggatgcgcctcctgcccctgctggcgctgctggccctctggggacctgacccagccgcagcctttgggaaccaacacctgtgcggctcacacctggtggaagctctctacctagtgtgcggggaacgaggcttcttctacacacccaagacccgccggaagcgggaggacctgcaggtggggcaggtggagctgggcgggggcccaggccctggtgcaggcagcctgcagcccttggccctggaggggtcccgacgcaagcgtatggtcttcacactcgaagatttcgttggggactggcgacagacagccggctacaacctggaccaagtccttgaacagggaggtgtgtccagtttgtttcagaatctcggggtgtccgtaactccgatccaaaggattgtcctgagcggtgaaaatgggctgaagatcgacatccatgtcatcatcccgtatgaaggtctgagcggcgaccaaatgggccagatcgaaaaaatttttaaggtggtgtaccctgtggatgatcatcactttaaggtgatcctgcactatggcacactggtaatcgacggggttacgccgaacatgatcgactatttcggacggccgtatgaaggcatcgccgtgttcgacggcaaaaagatcactgtaacagggaccctgtggaacggcaacaaaattatcgacgagcgcctgatcaaccccgacggctccctgctgttccgagtaaccatcaacggagtgaccggctggcggctgtgcgaacgcattctggcggctgctgctgcgggcattgtggaacaatgctgtaccagcatctgctccctctaccagctggagaactactgcaactag

SEQ ID NO: 42 - DNA, 864 bp, synthetic construct
  source 1..864: mol_type = other DNA; note = Insulin NLuc A mut BR22A
atggccctgtggatgcgcctcctgcccctgctggcgctgctggccctctggggacctgacccagccgcagcctttgtgaaccaacacctgtgcggctcacacctggtggaagctctctacctagtgtgcggggaagcaggcttcttctacacacccaagacccgccggaagcgggaggacctgcaggtggggcaggtggagctgggcgggggcccaggccctggtgcaggcagcctgcagcccttggccctggaggggtcccgacgcaagcgtatggtcttcacactcgaagatttcgttggggactggcgacagacagccggctacaacctggaccaagtccttgaacagggaggtgtgtccagtttgtttcagaatctcggggtgtccgtaactccgatccaaaggattgtcctgagcggtgaaaatgggctgaagatcgacatccatgtcatcatcccgtatgaaggtctgagcggcgaccaaatgggccagatcgaaaaaatttttaaggtggtgtaccctgtggatgatcatcactttaaggtgatcctgcactatggcacactggtaatcgacggggttacgccgaacatgatcgactatttcggacggccgtatgaaggcatcgccgtgttcgacggcaaaaagatcactgtaacagggaccctgtggaacggcaacaaaattatcgacgagcgcctgatcaaccccgacggctccctgctgttccgagtaaccatcaacggagtgaccggctggcggctgtgcgaacgcattctggcggctgctgctgcgggcattgtggaacaatgctgtaccagcatctgctccctctaccagctggagaactactgcaactag

SEQ ID NO: 43 - DNA, 861 bp, synthetic construct
  source 1..861: mol_type = other DNA; note = Insulin A NLuc
atggccctgtggatgcgcctcctgcccctgctggcgctgctggccctctggggacctgacccagccgcagcctttgtgaaccaacacctgtgcggctcacacctggtggaagctctctacctagtgtgcggggaacgaggcttcttctacacacccaagacccgccggaagcgggaggacctgcaggtggggcaggtggagctgggcgggggcccaggccctggtgcaggcagcctgcagcccttggccctggaggggtcccgacgcaagcgtggcattgtggaacaatgctgtaccagcatctgctccctctaccagctggagaactactgcaacggtggaggcatggtcttcacactcgaagatttcgttggggactggcgacagacagccggctacaacctggaccaagtccttgaacagggaggtgtgtccagtttgtttcagaatctcggggtgtccgtaactccgatccaaaggattgtcctgagcggtgaaaatgggctgaagatcgacatccatgtcatcatcccgtatgaaggtctgagcggcgaccaaatgggccagatcgaaaaaatttttaaggtggtgtaccctgtggatgatcatcactttaaggtgatcctgcactatggcacactggtaatcgacggggttacgccgaacatgatcgactatttcggacggccgtatgaaggcatcgccgtgttcgacggcaaaaagatcactgtaacagggaccctgtggaacggcaacaaaattatcgacgagcgcctgatcaaccccgacggctccctgctgttccgagtaaccatcaacggagtgaccggctggcggctgtgcgaacgcattctggcgtag

SEQ ID NO: 44 - DNA, 864 bp, synthetic construct; identical to SEQ ID NO: 1
  source 1..864: mol_type = other DNA; note = Insulin B NLuc

SEQ ID NO: 45 - DNA, 864 bp, synthetic construct; identical to SEQ ID NO: 39
  source 1..864: mol_type = other DNA; note = Insulin NLuc A

SEQ ID NO: 46 - DNA, 873 bp, synthetic construct
  source 1..873: mol_type = other DNA; note = secNLuc insulin
atgaactccttctccacaagcgccttcggtccagttgccttctccctgggcctgctcctggtgttgcctgctgccttccctgccccagtcttcacactcgaagatttcgttggggactggcgacagacagccggctacaacctggaccaagtccttgaacagggaggtgtgtccagtttgtttcagaatctcggggtgtccgtaactccgatccaaaggattgtcctgagcggtgaaaatgggctgaagatcgacatccatgtcatcatcccgtatgaaggtctgagcggcgaccaaatgggccagatcgaaaaaatttttaaggtggtgtaccctgtggatgatcatcactttaaggtgatcctgcactatggcacactggtaatcgacggggttacgccgaacatgatcgactatttcggacggccgtatgaaggcatcgccgtgttcgacggcaaaaagatcactgtaacagggaccctgtggaacggcaacaaaattatcgacgagcgcctgatcaaccccgacggctccctgctgttccgagtaaccatcaacggagtgaccggctggcggctgtgcgaacgcattctggcgggtggaggctttgtgaaccaacacctgtgcggctcacacctggtggaagctctctacctagtgtgcggggaacgaggcttcttctacacacccaagacccgccggaagcgggaggacctgcaggtggggcaggtggagctgggcgggggcccaggccctggtgcaggcagcctgcagcccttggccctggaggggtcccgacgcaagcgtggcattgtggaacaatgctgtaccagcatctgctccctctaccagctggagaactactgcaactag

SEQ ID NO: 47 - DNA, 4893 bp, synthetic construct
  source 1..4893: mol_type = other DNA; note = pCMVTnT INS Bchaindel24-30Nluc
tcaatattggccattagccatattattcattggttatatagcataaatcaatattggctattggccattgcatacgttgtatctatatcataatatgtacatttatattggctcatgtccaatatgaccgccatgttggcattgattattgactagttattaatagtaatcaattacggggtcattagttcatagcccatatatggagttccgcgttacataacttacggtaaatggcccgcctggctgaccgcccaacgacccccgcccattgacgtcaataatgacgtatgttcccatagtaacgccaatagggactttccattgacgtcaatgggtggagtatttacggtaaactgcccacttggcagtacatcaagtgtatcatatgccaagtccgccccctattgacgtcaatgacggtaaatggcccgcctggcattatgcccagtacatgaccttacgggactttcctacttggcagtacatctacgtattagtcatcgctattaccatggtgatgcggttttggcagtacaccaatgggcgtggatagcggtttgactcacggggatttccaagtctccaccccattgacgtcaatgggagtttgttttggcaccaaaatcaacgggactttccaaaatgtcgtaataaccccgccccgttgacgcaaatgggcggtaggcgtgtacggtgggaggtctatataagcagagctcgtttagtgaaccgtcagatcactagaagctttattgcggtagtttatcacagttaaattgctaacgcagtcagtgcttctgacacaacagtctcgaacttaagctgcagaagttggtcgtgaggcactgggcaggtaagtatcaaggttacaagacaggtttaaggagaccaatagaaactgggcttgtcgagacagagaagactcttgcgtttctgataggcacctattggtcttactgacatccactttgcctttctctccacaggtgtccactcccagttcaattacagctcttaaggctagagtacttaatacgactcactataggctagcatttaggtgacactatagaatacaagctacttgttctttttgcactcgagaattcatggccctgtggatgcgcctcctgcccctgctggcgctgctggccctctggggacctgacccagccgcagcctttgtgaaccaacacctgtgcggctcacacctggtggaagctctctacctagtgtgcggggaacgaggcatggtcttcacactcgaagatttcgttggggactggcgacagacagccggctacaacctggaccaagtccttgaacagggaggtgtgtccagtttgtttcagaatctcggggtgtccgtaactccgatccaaaggattgtcctgagcggtgaaaatgggctgaagatcgacatccatgtcatcatcccgtatgaaggtctgagcggcgaccaaatgggccagatcgaaaaaatttttaaggtggtgtaccctgtggatgatcatcactttaaggtgatcctgcactatggcacactggtaatcgacggggttacgccgaacatgatcgactatttcggacggccgtatgaaggcatcgccgtgttcgacggcaaaaagatcactgtaacagggaccctgtggaacggcaacaaaattatcgacgagcgcctgatcaaccccgacggctccctgctgttccgagtaaccatcaacggagtgaccggctggcggctgtgcgaacgcattctggcggctgctgctgcgcgccggaagcgggaggacctgcaggtggggcaggtggagctgggcgggggcccaggcgcaggcagcctgcagcccttggccctggaggggtcccgacgcaagcgtggcattgtggaacaatgctgtaccagcatctgctccctctaccagctggagaactactgcaactaggaattcacgcgtggtacctctagagtcgacccgggcggccgcttcgagcagacatgataagatacattgatgagtttggacaaaccacaactagaatgcagtgaaaaaaatgctttatttgtgaaatttgtgatgctattgctttatttgtaaccattataagctgcaataaacaagttaacaacaacaattgcattcattttatgtttcaggttcagggggagatgtgggaggttttttaaagcaagtaaaacctctacaaatgtggtaaaatcgataaggatccgggctggcgtaatagcgaagaggcccgcaccgatcgcccttcccaacagttgcgcagcctgaatggcgaatggacgcgccctgtagcggcgcattaagcgcggcgggtgtggtggttacgcgcagcgtgaccgctacacttgccagcgccctagcgcccgctcctttcgctttcttcccttcctttctcgccacgttcgccggctttccccgtcaagctctaaatcgggggctccctttagggttccgatttagtgctttacggcacctcgaccccaaaaaacttgattagggtgatggttcacgtagtgggccatcgccctgatagacggtttttcgccctttgacgttggagtccacgttctttaatagtggactcttgttccaaactggaacaacactcaaccctatctcggtctattcttttgatttataagggattttgccgatttcggcctattggttaaaaaatgagctgatttaacaaaaatttaacgcgaattttaacaaaatattaacgcttacaatttcctgatgcggtattttctccttacgcatctgtgcggtatttcacaccgcatatggtgcactctcagtacaatctgctctgatgccgcatagttaagccagccccgacacccgccaacacccgctgacgcgccctgacgggcttgtctgctcccggcatccgcttacagacaagctgtgaccgtctccgggagctgcatgtgtcagaggttttcaccgtcatcaccgaaacgcgcgagacgaaagggcctcgtgatacgcctatttttataggttaatgtcatgataataatggtttcttagacgtcaggtggcacttttcggggaaatgtgcgcggaacccctatttgtttatttttctaaatacattcaaatatgtatccgctcatgagacaataaccctgataaatgcttcaataatattgaaaaaggaagagtatgagtattcaacatttccgtgtcgcccttattcccttttttgcggcattttgccttcctgtttttgctcacccagaaacgctggtgaaagtaaaagatgctgaagatcagttgggtgcacgagtgggttacatcgaactggatctcaacagcggtaagatccttgagagttttcgccccgaagaacgttttccaatgatgagcacttttaaagttctgctatgtggcgcggtattatcccgtattgacgccgggcaagagcaactcggtcgccgcatacactattctcagaatgacttggttgagtactcaccagtcacagaaaagcatcttacggatggcatgacagtaagagaattatgcagtgctgccataaccatgagtgataacactgcggccaacttacttctgacaacgatcggaggaccgaaggagctaaccgcttttttgcacaacatgggggatcatgtaactcgccttgatcgttgggaaccggagctgaatgaagccataccaaacgacgagcgtgacaccacgatgcctgtagcaatggcaacaacgttgcgcaaactattaactggcgaactacttactctagcttcccggcaacaattaatagactggatggaggcggataaagttgcaggaccacttctgcgctcggcccttccggctggctggtttattgctgataaatctggagccggtgagcgtgggtctcgcggtatcattgcagcactggggccagatggtaagccctcccgtatcgtagttatctacacgacggggagtcaggcaactatggatgaacgaaatagacagatcgctgagataggtgcctcactgattaagcattggtaactgtcagaccaagtttactcatatatactttagattgatttaaaacttcatttttaatttaaaaggatctaggtgaagatcctttttgataatctcatgaccaaaatcccttaacgtgagttttcgttccactgagcgtcagaccccgtagaaaagatcaaaggatcttcttgagatcctttttttctgcgcgtaatctgctgcttgcaaacaaaaaaaccaccgctaccagcggtggtttgtttgccggatcaagagctaccaactctttttccgaaggtaactggcttcagcagagcgcagataccaaatactgttcttctagtgtagccgtagttaggccaccacttcaagaactctgtagcaccgcctacatacctcgctctgctaatcctgttaccagtggctgctgccagtggcgataagtcgtgtcttaccgggttggactcaagacgatagttaccggataaggcgcagcggtcgggctgaacggggggttcgtgcacacagcccagcttggagcgaacgacctacaccgaactgagatacctacagcgtgagctatgagaaagcgccacgcttcccgaagggagaaaggcggacaggtatccggtaagcggcagggtcggaacaggagagcgcacgagggagcttccagggggaaacgcctggtatctttatagtcctgtcgggtttcgccacctctgacttgagcgtcgatttttgtgatgctcgtcaggggggcggagcctatggaaaaacgccagcaacgcggcctttttacggttcctggccttttgctggccttttgctcacatggctcgacagatct

SEQ ID NO: 48 - DNA, 4896 bp, synthetic construct
  source 1..4896: mol_type = other DNA; note = pCMVTnT INS Bchaindel25-30Nluc
tcaatattggccattagccatattattcattggttatatagcataaatcaatattggctattggccattgcatacgttgtatctatatcataatatgtacatttatattggctcatgtccaatatgaccgccatgttggcattgattattgactagttattaatagtaatcaattacggggtcattagttcatagcccatatatggagttccgcgttacataacttacggtaaatggcccgcctggctgaccgcccaacgacccccgcccattgacgtcaataatgacgtatgttcccatagtaacgccaatagggactttccattgacgtcaatgggtggagtatttacggtaaactgcccacttggcagtacatcaagtgtatcatatgccaagtccgccccctattgacgtcaatgacggtaaatggcccgcctggcattatgcccagtacatgaccttacgggactttcctacttggcagtacatctacgtattagtcatcgctattaccatggtgatgcggttttggcagtacaccaatgggcgtggatagcggtttgactcacggggatttccaagtctccaccccattgacgtcaatgggagtttgttttggcaccaaaatcaacgggactttccaaaatgtcgtaataaccccgccccgttgacgcaaatgggcggtaggcgtgtacggtgggaggtctatataagcagagctcgtttagtgaaccgtcagatcactagaagctttattgcggtagtttatcacagttaaattgctaacgcagtcagtgcttctgacacaacagtctcgaacttaagctgcagaagttggtcgtgaggcactgggcaggtaagtatcaaggttacaagacaggtttaaggagaccaatagaaactgggcttgtcgagacagagaagactcttgcgtttctgataggcacctattggtcttactgacatccactttgcctttctctccacaggtgtccactcccagttcaattacagctcttaaggctagagtacttaatacgactcactataggctagcatttaggtgacactatagaatacaagctacttgttctttttgcactcgagaattcatggccctgtggatgcgcctcctgcccctgctggcgctgctggccctctggggacctgacccagccgcagcctttgtgaaccaacacctgtgcggctcacacctggtggaagctctctacctagtgtgcggggaacgaggcttcatggtcttcacactcgaagatttcgttggggactggcgacagacagccggctacaacctggaccaagtccttgaacagggaggtgtgtccagtttgtttcagaatctcggggtgtccgtaactccgatccaaaggattgtcctgagcggtgaaaatgggctgaagatcgacatccatgtcatcatcccgtatgaaggtctgagcggcgaccaaatgggccagatcgaaaaaatttttaaggtggtgtaccctgtggatgatcatcactttaaggtgatcctgcactatggcacactggtaatcgacggggttacgccgaacatgatcgactatttcggacggccgtatgaaggcatcgccgtgttcgacggcaaaaagatcactgtaacagggaccctgtggaacggcaacaaaattatcgacgagcgcctgatcaaccccgacggctccctgctgttccgagtaaccatcaacggagtgaccggctggcggctgtgcgaacgcattctggcggctgctgctgcgcgccggaagcgggaggacctgcaggtggggcaggtggagctgggcgggggcccaggcgcaggcagcctgcagcccttggccctggaggggtcccgacgcaagcgtggcattgtggaacaatgctgtaccagcatctgctccctctaccagctggagaactactgcaactaggaattcacgcgtggtacctctagagtcgacccgggcggccgcttcgagcagacatgataagatacattgatgagtttggacaaaccacaactagaatgcagtgaaaaaaatgctttatttgtgaaatttgtgatgctattgctttatttgtaaccattataagctgcaataaacaagttaacaacaacaattgcattcattttatgtttcaggttcagggggagatgtgggaggttttttaaagcaagtaaaacctctacaaatgtggtaaaatcgataaggatccgggctggcgtaatagcgaagaggcccgcaccgatcgcccttcccaacagttgcgcagcctgaatggcgaatggacgcgccctgtagcggcgcattaagcgcggcgggtgtggtggttacgcgcagcgtgaccgctacacttgccagcgccctagcgcccgctcctttcgctttcttcccttcctttctcgccacgttcgccggctttccccgtcaagctctaaatcgggggctccctttagggttccgatttagtgctttacggcacctcgaccccaaaaaacttgattagggtgatggttcacgtagtgggccatcgccctgatagacggtttttcgccctttgacgttggagtccacgttctttaatagtggactcttgttccaaactggaacaacactcaaccctatctcggtctattcttttgatttataagggattttgccgatttcggcctattggttaaaaaatgagctgatttaacaaaaatttaacgcgaattttaacaaaatattaacgcttacaatttcctgatgcggtattttctccttacgcatctgtgcggtatttcacaccgcatatggtgcactctcagtacaatctgctctgatgccgcatagttaagccagccccgacacccgccaacacccgctgacgcgccctgacgggcttgtctgctcccggcatccgcttacagacaagctgtgaccgtctccgggagctgcatgtgtcagaggttttcaccgtcatcaccgaaacgcgcgagacgaaagggcctcgtgatacgcctatttttataggttaatgtcatgataataatggtttcttagacgtcaggtggcacttttcggggaaatgtgcgcggaacccctatttgtttatttttctaaatacattcaaatatgtatccgctcatgagacaataaccctgataaatgcttcaataatattgaaaaaggaagagtatgagtattcaacatttccgtgtcgcccttattcccttttttgcggcattttgccttcctgtttttgctcacccagaaacgctggtgaaagtaaaagatgctgaagatcagttgggtgcacgagtgggttacatcgaactggatctcaacagcggtaagatccttgagagttttcgccccgaagaacgttttccaatgatgagcacttttaaagttctgctatgtggcgcggtattatcccgtattgacgccgggcaagagcaactcggtcgccgcatacactattctcagaatgacttggttgagtactcaccagtcacagaaaagcatcttacggatggcatgacagtaagagaattatgcagtgctgccataaccatgagtgataacactgcggccaacttacttctgacaacgatcggaggaccgaaggagctaaccgcttttttgcacaacatgggggatcatgtaactcgccttgatcgttgggaaccggagctgaatgaagccataccaaacgacgagcgtgacaccacgatgcctgtagcaatggcaacaacgttgcgcaaactattaactggcgaactacttactctagcttcccggcaacaattaatagactggatggaggcggataaagttgcaggaccacttctgcgctcggcccttccggctggctggtttattgctgataaatctggagccggtgagcgtgggtctcgcggtatcattgcagcactggggccagatggtaagccctcccgtatcgtagttatctacacgacggggagtcaggcaactatggatgaacgaaatagacagatcgctgagataggtgcctcactgattaagcattggtaactgtcagaccaagtttactcatatatactttagattgatttaaaacttcatttttaatttaaaaggatctaggtgaagatcctttttgataatctcatgaccaaaatcccttaacgtgagttttcgttccactgagcgtcagaccccgtagaaaagatcaaaggatcttcttgagatcctttttttctgcgcgtaatctgctgcttgcaaacaaaaaaaccaccgctaccagcggtggtttgtttgccggatcaagagctaccaactctttttccgaaggtaactggcttcagcagagcgcagataccaaatactgttcttctagtgtagccgtagttaggccaccacttcaagaactctgtagcaccgcctacatacctcgctctgctaatcctgttaccagtggctgctgccagtggcgataagtcgtgtcttaccgggttggactcaagacgatagttaccggataaggcgcagcggtcgggctgaacggggggttcgtgcacacagcccagcttggagcgaacgacctacaccgaactgagatacctacagcgtgagctatgagaaagcgccacgcttcccgaagggagaaaggcggacaggtatccggtaagcggcagggtcggaacaggagagcgcacgagggagcttccagggggaaacgcctggtatctttatagtcctgtcgggtttcgccacctctgacttgagcgtcgatttttgtgatgctcgtcaggggggcggagcctatggaaaaacgccagcaacgcggcctttttacggttcctggccttttgctggccttttgctcacatggctcgacagatct

SEQ ID NO: 49 - DNA, 4899 bp, synthetic construct
  source 1..4899: mol_type = other DNA; note = pCMVTnT INS Bchaindel26-30Nluc
tcaatattggccattagccatattattcattggttatatagcataaatcaatattggctattggccattgcatacgttgtatctatatcataatatgtacatttatattggctcatgtccaatatgaccgccatgttggcattgattattgactagttattaatagtaatcaattacggggtcattagttcatagcccatatatggagttccgcgttacataacttacggtaaatggcccgcctggctgaccgcccaacgacccccgcccattgacgtcaataatgacgtatgttcccatagtaacgccaatagggactttccattgacgtcaatgggtggagtatttacggtaaactgcccacttggcagtacatcaagtgtatcatatgccaagtccgccccctattgacgtcaatgacggtaaatggcccgcctggcattatgcccagtacatgaccttacgggactttcctacttggcagtacatctacgtattagtcatcgctattaccatggtgatgcggttttggcagtacaccaatgggcgtggatagcggtttgactcacggggatttccaagtctccaccccattgacgtcaatgggagtttgttttggcaccaaaatcaacgggactttccaaaatgtcgtaataaccccgccccgttgacgcaaatgggcggtaggcgtgtacggtgggaggtctatataagcagagctcgtttagtgaaccgtcagatcactagaagctttattgcggtagtttatcacagttaaattgctaacgcagtcagtgcttctgacacaacagtctcgaacttaagctgcagaagttggtcgtgaggcactgggcaggtaagtatcaaggttacaagacaggtttaaggagaccaatagaaactgggcttgtcgagacagagaagactcttgcgtttctgataggcacctattggtcttactgacatccactttgcctttctctccacaggtgtccactcccagttcaattacagctcttaaggctagagtacttaatacgactcactataggctagcatttaggtgacactatagaatacaagctacttgttctttttgcactcgagaattcatggccctgtggatgcgcctcctgcccctgctggcgctgctggccctctggggacctgacccagccgcagcctttgtgaaccaacacctgtgcggctcacacctggtggaagctctctacctagtgtgcggggaacgaggcttcttcatggtcttcacactcgaagatttcgttggggactggcgacagacagccggctacaacctggaccaagtccttgaacagggaggtgtgtccagtttgtttcagaatctcggggtgtccgtaactccgatccaaaggattgtcctgagcggtgaaaatgggctgaagatcgacatccatgtcatcatcccgtatgaaggtctgagcggcgaccaaatgggccagatcgaaaaaatttttaaggtggtgtaccctgtggatgatcatcactttaaggtgatcctgcactatggcacactggtaatcgacggggttacgccgaacatgatcgactatttcggacggccgtatgaaggcatcgccgtgttcgacggcaaaaagatcactgtaacagggaccctgtggaacggcaacaaaattatcgacgagcgcctgatcaaccccgacggctccctgctgttccgagtaaccatcaacggagtgaccggctggcggctgtgcgaacgcattctggcggctgctgctgcgcgccggaagcgggaggacctgcaggtggggcaggtggagctgggcgggggcccaggcgcaggcagcctgcagcccttggccctggaggggtcccgacgcaagcgtggcattgtggaacaatgctgtaccagcatctgctccctctaccagctggagaactactgcaactaggaattcacgcgtggtacctctagagtcgacccgggcggccgcttcgagcagacatgataagatacattgatgagtttggacaaaccacaactagaatgcagtgaaaaaaatgctttatttgtgaaatttgtgatgctattgctttatttgtaaccattataagctgcaataaacaagttaacaacaacaattgcattcattttatgtttcaggttcagggggagatgtgggaggttttttaaagcaagtaaaacctctacaaatgtggtaaaatcgataaggatccgggctggcgtaatagcgaagaggcccgcaccgatcgcccttcccaacagttgcgcagcctgaatggcgaatggacgcgccctgtagcggcgcattaagcgcggcgggtgtggtggttacgcgcagcgtgaccgctacacttgccagcgccctagcgcccgctcctttcgctttcttcccttcctttctcgccacgttcgccggctttccccgtcaagctctaaatcgggggctccctttagggttccgatttagtgctttacggcacctcgaccccaaaaaacttgattagggtgatggttcacgtagtgggccatcgccctgatagacggtttttcgccctttgacgttggagtccacgttctttaatagtggactcttgttccaaactggaacaacactcaaccctatctcggtctattcttttgatttataagggattttgccgatttcggcctattggttaaaaaatgagctgatttaacaaaaatttaacgcgaattttaacaaaatattaacgcttacaatttcctgatgcggtattttctccttacgcatctgtgcggtatttcacaccgcatatggtgcactctcagtacaatctgctctgatgccgcatagttaagccagccccgacacccgccaacacccgctgacgcgccctgacgggcttgtctgctcccggcatccgcttacagacaagctgtgaccgtctccgggagctgcatgtgtcagaggttttcaccgtcatcaccgaaacgcgcgagacgaaagggcctcgtgatacgcctatttttataggttaatgtcatgataataatggtttcttagacgtcaggtggcacttttcggggaaatgtgcgcggaacccctatttgtttatttttctaaatacattcaaatatgtatccgctcatgagacaataaccctgataaatgcttcaataatattgaaaaaggaagagtatgagtattcaacatttccgtgtcgcccttattcccttttttgcggcattttgccttcctgtttttgctcacccagaaacgctggtgaaagtaaaagatgctgaagatcagttgggtgcacgagtgggttacatcgaactggatctcaacagcggtaagatccttgagagttttcgccccgaagaacgttttccaatgatgagcacttttaaagttctgctatgtggcgcggtattatcccgtattgacgccgggcaagagcaactcggtcgccgcatacactattctcagaatgacttggttgagtactcaccagtcacagaaaagcatcttacggatggcatgacagtaagagaattatgcagtgctgccataaccatgagtgataacactgcggccaacttacttctgacaacgatcggaggaccgaaggagctaaccgcttttttgcacaacatgggggatcatgtaactcgccttgatcgttgggaaccggagctgaatgaagccataccaaacgacgagcgtgacaccacgatgcctgtagcaatggcaacaacgttgcgcaaactattaactggcgaactacttactctagcttcccggcaacaattaatagactggatggaggcggataaagttgcaggaccacttctgcgctcggcccttccggctggctggtttattgctgataaatctggagccggtgagcgtgggtctcgcggtatcattgcagcactggggccagatggtaagccctcccgtatcgtagttatctacacgacggggagtcaggcaactatggatgaacgaaatagacagatcgctgagataggtgcctcactgattaagcattggtaactgtcagaccaagtttactcatatatactttagattgatttaaaacttcatttttaatttaaaaggatctaggtgaagatcctttttgataatctcatgaccaaaatcccttaacgtgagttttcgttccactgagcgtcagaccccgtagaaaagatcaaaggatcttcttgagatcctttttttctgcgcgtaatctgctgcttgcaaacaaaaaaaccaccgctaccagcggtggtttgtttgccggatcaagagctaccaactctttttccgaaggtaactggcttcagcagagcgcagataccaaatactgttcttctagtgtagccgtagttaggccaccacttcaagaactctgtagcaccgcctacatacctcgctctgctaatcctgttaccagtggctgctgccagtggcgataagtcgtgtcttaccgggttggactcaagacgatagttaccggataaggcgcagcggtcgggctgaacggggggttcgtgcacacagcccagcttggagcgaacgacctacaccgaactgagatacctacagcgtgagctatgagaaagcgccacgcttcccgaagggagaaaggcggacaggtatccggtaagcggcagggtcggaacaggagagcgcacgagggagcttccagggggaaacgcctggtatctttatagtcctgtcgggtttcgccacctctgacttgagcgtcgatttttgtgatgctcgtcaggggggcggagcctatggaaaaacgccagcaacgcggcctttttacggttcctggccttttgctggccttttgctcacatggctcgacagatct

SEQ ID NO: 50 - DNA, 4902 bp, synthetic construct
  source 1..4902: mol_type = other DNA; note = pCMVTnT INS Bchaindel27-30Nluc
tcaatattggccattagccatattattcattggttatatagcataaatcaatattggctattggccattgcatacgttgtatctatatcataatatgtacatttatattggctcatgtccaatatgaccgccatgttggcattgattattgactagttattaatagtaatcaattacggggtcattagttcatagcccatatatggagttccgcgttacataacttacggtaaatggcccgcctggctgaccgcccaacgacccccgcccattgacgtcaataatgacgtatgttcccatagtaacgccaatagggactttccattgacgtcaatgggtggagtatttacggtaaactgcccacttggcagtacatcaagtgtatcatatgccaagtccgccccctattgacgtcaatgacggtaaatggcccgcctggcattatgcccagtacatgaccttacgggactttcctacttggcagtacatctacgtattagtcatcgctattaccatggtgatgcggttttggcagtacaccaatgggcgtggatagcggtttgactcacggggatttccaagtctccaccccattgacgtcaatgggagtttgttttggcaccaaaatcaacgggactttccaaaatgtcgtaataaccccgccccgttgacgcaaatgggcggtaggcgtgtacggtgggaggtctatataagcagagctcgtttagtgaaccgtcagatcactagaagctttattgcggtagtttatcacagttaaattgctaacgcagtcagtgcttctgacacaacagtctcgaacttaagctgcagaagttggtcgtgaggcactgggcaggtaagtatcaaggttacaagacaggtttaaggagaccaatagaaactgggcttgtcgagacagagaagactcttgcgtttctgataggcacctattggtcttactgacatccactttgcctttctctccacaggtgtccactcccagttcaattacagctcttaaggctagagtacttaatacgactcactataggctagcatttaggtgacactatagaatacaagctacttgttctttttgcactcgagaattcatggccctgtggatgcgcctcctgcccctgctggcgctgctggccctctggggacctgacccagccgcagcctttgtgaaccaacacctgtgcggctcacacctggtggaagctctctacctagtgtgcggggaacgaggcttcttctacatggtcttcacactcgaagatttcgttggggactggcgacagacagccggctacaacctggaccaagtccttgaacagggaggtgtgtccagtttgtttcagaatctcggggtgtccgtaactccgatccaaaggattgtcctgagcggtgaaaatgggctgaagatcgacatccatgtcatcatcccgtatgaaggtctgagcggcgaccaaatgggccagatcgaaaaaatttttaaggtggtgtaccctgtggatgatcatcactttaaggtgatcctgcactatggcacactggtaatcgacggggttacgccgaacatgatcgactatttcggacggccgtatgaaggcatcgccgtgttcgacggcaaaaagatcactgtaacagggaccctgtggaacggcaacaaaattatcgacgagcgcctgatcaaccccgacggctccctgctgttccgagtaaccatcaacggagtgaccggctggcggctgtgcgaacgcattctggcggctgctgctgcgcgccggaagcgggaggacctgcaggtggggcaggtggagctgggcgggggcccaggcgcaggcagcctgcagcccttggccctggaggggtcccgacgcaagcgtggcattgtggaacaatgctgtaccagcatctgctccctctaccagctggagaactactgcaactaggaattcacgcgtggtacctctagagtcgacccgggcggccgcttcgagcagacatgataagatacattgatgagtttggacaaaccacaactagaatgcagtgaaaaaaatgctttatttgtgaaatttgtgatgctattgctttatttgtaaccattataagctgcaataaacaagttaacaacaacaattgcattcattttatgtttcaggttcagggggagatgtgggaggttttttaaagcaagtaaaacctctacaaatgtggtaaaatcgataaggatccgggctggcgtaatagcgaagaggcccgcaccgatcgcccttcccaacagttgcgcagcctgaatggcgaatggacgcgccctgtagcggcgcattaagcgcggcgggtgtggtggttacgcgcagcgtgaccgctacacttgccagcgccctagcgcccgctcctttcgctttcttcccttcctttctcgccacgttcgccggctttccccgtcaagctctaaatcgggggctccctttagggttccgatttagtgctttacggcacctcgaccccaaaaaacttgattagggtgatggttcacgtagtgggccatcgccctgatagacggtttttcgccctttgacgttggagtccacgttctttaatagtggactcttgttccaaactggaacaacactcaaccctatctcggtctattcttttgatttataagggattttgccgatttcggcctattggttaaaaaatgagctgatttaacaaaaatttaacgcgaattttaacaaaatattaacgcttacaatttcctgatgcggtattttctccttacgcatctgtgcggtatttcacaccgcatatggtgcactctcagtacaatctgctctgatgccgcatagttaagccagccccgacacccgccaacacccgctgacgcgccctgacgggcttgtctgctcccggcatccgcttacagacaagctgtgaccgtctccgggagctgcatgtgtcagaggttttcaccgtcatcaccgaaacgcgcgagacgaaagggcctcgtgatacgcctatttttataggttaatgtcatgataataatggtttcttagacgtcaggtggcacttttcggggaaatgtgcgcggaacccctatttgtttatttttctaaatacattcaaatatgtatccgctcatgagacaataaccctgataaatgcttcaataatattgaaaaaggaagagtatgagtattcaacatttccgtgtcgcccttattcccttttttgcggcattttgccttcctgtttttgctcacccagaaacgctggtgaaagtaaaagatgctgaagatcagttgggtgcacgagtgggttacatcgaactggatctcaacagcggtaagatccttgagagttttcgccccgaagaacgttttccaatgatgagcacttttaaagttctgctatgtggcgcggtattatcccgtattgacgccgggcaagagcaactcggtcgccgcatacactattctcagaatgacttggttgagtactcaccagtcacagaaaagcatcttacggatggcatgacagtaagagaattatgcagtgctgccataaccatgagtgataacactgcggccaacttacttctgacaacgatcggaggaccgaaggagctaaccgcttttttgcacaacatgggggatcatgtaactcgccttgatcgttgggaaccggagctgaatgaagccataccaaacgacgagcgtgacaccacgatgcctgtagcaatggcaacaacgttgcgcaaactattaactggcgaactacttactctagcttcccggcaacaattaatagactggatggaggcggataaagttgcaggaccacttctgcgctcggcccttccggctggctggtttattgctgataaatctggagccggtgagcgtgggtctcgcggtatcattgcagcactggggccagatggtaagccctcccgtatcgtagttatctacacgacggggagtcaggcaactatggatgaacgaaatagacagatcgctgagataggtgcctcactgattaagcattggtaactgtcagaccaagtttactcatatatactttagattgatttaaaacttcatttttaatttaaaaggatctaggtgaagatcctttttgataatctcatgaccaaaatcccttaacgtgagttttcgttccactgagcgtcagaccccgtagaaaagatcaaaggatcttcttgagatcctttttttctgcgcgtaatctgctgcttgcaaacaaaaaaaccaccgctaccagcggtggtttgtttgccggatcaagagctaccaactctttttccgaaggtaactggcttcagcagagcgcagataccaaatactgttcttctagtgtagccgtagttaggccaccacttcaagaactctgtagcaccgcctacatacctcgctctgctaatcctgttaccagtggctgctgccagtggcgataagtcgtgtcttaccgggttggactcaagacgatagttaccggataaggcgcagcggtcgggctgaacggggggttcgtgcacacagcccagcttggagcgaacgacctacaccgaactgagatacctacagcgtgagctatgagaaagcgccacgcttcccgaagggagaaaggcggacaggtatccggtaagcggcagggtcggaacaggagagcgcacgagggagcttccagggggaaacgcctggtatctttatagtcctgtcgggtttcgccacctctgacttgagcgtcgatttttgtgatgctcgtcaggggggcggagcctatggaaaaacgccagcaacgcggcctttttacggttcctggccttttgctggccttttgctcacatggctcgacagatct

SEQ ID NO: 51 - DNA, 4905 bp, synthetic construct
  source 1..4905: mol_type = other DNA; note = pCMVTnT INS Bchaindel28-30Nluc
tcaatattggccattagccatattattcattggttatatagcataaatcaatattggctattggccattgcatacgttgtatctatatcataatatgtacatttatattggctcatgtccaatatgaccgccatgttggcattgattattgactagttattaatagtaatcaattacggggtcattagttcatagcccatatatggagttccgcgttacataacttacggtaaatggcccgcctggctgaccgcccaacgacccccgcccattgacgtcaataatgacgtatgttcccatagtaacgccaatagggactttccattgacgtcaatgggtggagtatttacggtaaactgcccacttggcagtacatcaagtgtatcatatgccaagtccgccccctattgacgtcaatgacggtaaatggcccgcctggcattatgcccagtacatgaccttacgggactttcctacttggcagtacatctacgtattagtcatcgctattaccatggtgatgcggttttggcagtacaccaatgggcgtggatagcggtttgactcacggggatttccaagtctccaccccattgacgtcaatgggagtttgttttggcaccaaaatcaacgggactttccaaaatgtcgtaataaccccgccccgttgacgcaaatgggcggtaggcgtgtacggtgggaggtctatataagcagagctcgtttagtgaaccgtcagatcactagaagctttattgcggtagtttatcacagttaaattgctaacgcagtcagtgcttctgacacaacagtctcgaacttaagctgcagaagttggtcgtgaggcactgggcaggtaagtatcaaggttacaagacaggtttaaggagaccaatagaaactgggcttgtcgagacagagaagactcttgcgtttctgataggcacctattggtcttactgacatccactttgcctttctctccacaggtgtccactcccagttcaattacagctcttaaggctagagtacttaatacgactcactataggctagcatttaggtgacactatagaatacaagctacttgttctttttgcactcgagaattcatggccctgtggatgcgcctcctgcccctgctggcgctgctggccctctggggacctgacccagccgcagcctttgtgaaccaacacctgtgcggctcacacctggtggaagctctctacctagtgtgcggggaacgaggcttcttctacacaatggtcttcacactcgaagatttcgttggggactggcgacagacagccggctacaacctggaccaagtccttgaacagggaggtgtgtccagtttgtttcagaatctcggggtgtccgtaactccgatccaaaggattgtcctgagcggtgaaaatgggctgaagatcgacatccatgtcatcatcccgtatgaaggtctgagcggcgaccaaatgggccagatcgaaaaaatttttaaggtggtgtaccctgtggatgatcatcactttaaggtgatcctgcactatggcacactggtaatcgacggggttacgccgaacatgatcgactatttcggacggccgtatgaaggcatcgccgtgttcgacggcaaaaagatcactgtaacagggaccctgtggaacggcaacaaaattatcgacgagcgcctgatcaaccccgacggctccctgctgttccgagtaaccatcaacggagtgaccggctggcggctgtgcgaacgcattctggcggctgctgctgcgcgccggaagcgggaggacctgcaggtggggcaggtggagctgggcgggggcccaggcgcaggcagcctgcagcccttggccctggaggggtcccgacgcaagcgtggcattgtggaacaatgctgtaccagcatctgctccctctaccagctggagaactactgcaactaggaattcacgcgtggtacctctagagtcgacccgggcggccgcttcgagcagacatgataagatacattgatgagtttggacaaaccacaactagaatgcagtgaaaaaaatgctttatttgtgaaatttgtgatgctattgctttatttgtaaccattataagctgcaataaacaagttaacaacaacaattgcattcattttatgtttcaggttcagggggagatgtgggaggttttttaaagcaagtaaaacctctacaaatgtggtaaaatcgataaggatccgggctggcgtaatagcgaagaggcccgcaccgatcgcccttcccaacagttgcgcagcctgaatggcgaatggacgcgccctgtagcggcgcattaagcgcggcgggtgtggtggttacgcgcagcgtgaccgctacacttgccagcgccctagcgcccgctcctttcgctttcttcccttcctttctcgccacgttcgccggctttccccgtcaagctctaaatcgggggctccctttagggttccgatttagtgctttacggcacctcgaccccaaaaaacttgattagggtgatggttcacgtagtgggccatcgccctgatagacggtttttcgccctttgacgttggagtccacgttctttaatagtggactcttgttccaaactggaacaacactcaaccctatctcggtctattcttttgatttataagggattttgccgatttcggcctattggttaaaaaatgagctgatttaacaaaaatttaacgcgaattttaacaaaatattaacgcttacaatttcctgatgcggtattttctccttacgcatctgtgcggtatttcacaccgcatatggtgcactctcagtacaatctgctctgatgccgcatagttaagccagccccgacacccgccaacacccgctgacgcgccctgacgggcttgtctgctcccggcatccgcttacagacaagctgtgaccgtctccgggagctgcatgtgtcagaggttttcaccgtcatcaccgaaacgcgcgagacgaaagggcctcgtgatacgcctatttttataggttaatgtcatgataataatggtttcttagacgtcaggtggcacttttcggggaaatgtgcgcggaacccctatttgtttatttttctaaatacattcaaatatgtatccgctcatgagacaataaccctgataaatgcttcaataatattgaaaaaggaagagtatgagtattcaacatttccgtgtcgcccttattcccttttttgcggcattttgccttcctgtttttgctcacccagaaacgctggtgaaagtaaaagatgctgaagatcagttgggtgcacgagtgggttacatcgaactggatctcaacagcggtaagatccttgagagttttcgccccgaagaacgttttccaatgatgagcacttttaaagttctgctatgtggcgcggtattatcccgtattgacgccgggcaagagcaactcggtcgccgcatacactattctcagaatgacttggttgagtactcaccagtcacagaaaagcatcttacggatggcatgacagtaagagaattatgcagtgctgccataaccatgagtgataacactgcggccaacttacttctgacaacgatcggaggaccgaaggagctaaccgcttttttgcacaacatgggggatcatgtaactcgccttgatcgttgggaaccggagctgaatgaagccataccaaacgacgagcgtgacaccacgatgcctgtagcaatggcaacaacgttgcgcaaactattaactggcgaactacttactctagcttcccggcaacaattaatagactggatggaggcggataaagttgcaggaccacttctgcgctcggcccttccggctggctggtttattgctgataaatctggagccggtgagcgtgggtctcgcggtatcattgcagcactggggccagatggtaagccctcccgtatcgtagttatctacacgacggggagtcaggcaactatggatgaacgaaatagacagatcgctgagataggtgcctcactgattaagcattggtaactgtcagaccaagtttactcatatatactttagattgatttaaaacttcatttttaatttaaaaggatctaggtgaagatcctttttgataatctcatgaccaaaatcccttaacgtgagttttcgttccactgagcgtcagaccccgtagaaaagatcaaaggatcttcttgagatcctttttttctgcgcgtaatctgctgcttgcaaacaaaaaaaccaccgctaccagcggtggtttgtttgccggatcaagagctaccaactctttttccgaaggtaactggcttcagcagagcgcagataccaaatactgttcttctagtgtagccgtagttaggccaccacttcaagaactctgtagcaccgcctacatacctcgctctgctaatcctgttaccagtggctgctgccagtggcgataagtcgtgtcttaccgggttggactcaagacgatagttaccggataaggcgcagcggtcgggctgaacggggggttcgtgcacacagcccagcttggagcgaacgacctacaccgaactgagatacctacagcgtgagctatgagaaagcgccacgcttcccgaagggagaaaggcggacaggtatccggtaagcggcagggtcggaacaggagagcgcacgagggagcttccagggggaaacgcctggtatctttatagtcctgtcgggtttcgccacctctgacttgagcgtcgatttttgtgatgctcgtcaggggggcggagcctatggaaaaacgccagcaacgcggcctttttacggttcctggccttttgctggccttttgctcacatggctcgacagatct

SEQ ID NO: 52 - DNA, 4920 bp, synthetic construct
  source 1..4920: mol_type = other DNA; note = pCMVTnT insulin Nluc-Achain A L13A
tcaatattggccattagccatattattcattggttatatagcataaatcaatattggctattggccattgcatacgttgtatctatatcataatatgtacatttatattggctcatgtccaatatgaccgccatgttggcattgattattgactagttattaatagtaatcaattacggggtcattagttcatagcccatatatggagttccgcgttacataacttacggtaaatggcccgcctggctgaccgcccaacgacccccgcccattgacgtcaataatgacgtatgttcccatagtaacgccaatagggactttccattgacgtcaatgggtggagtatttacggtaaactgcccacttggcagtacatcaagtgtatcatatgccaagtccgccccctattgacgtcaatgacggtaaatggcccgcctggcattatgcccagtacatgaccttacgggactttcctacttggcagtacatctacgtattagtcatcgctattaccatggtgatgcggttttggcagtacaccaatgggcgtggatagcggtttgactcacggggatttccaagtctccaccccattgacgtcaatgggagtttgttttggcaccaaaatcaacgggactttccaaaatgtcgtaataaccccgccccgttgacgcaaatgggcggtaggcgtgtacggtgggaggtctatataagcagagctcgtttagtgaaccgtcagatcactagaagctttattgcggtagtttatcacagttaaattgctaacgcagtcagtgcttctgacacaacagtctcgaacttaagctgcagaagttggtcgtgaggcactgggcaggtaagtatcaaggttacaagacaggtttaaggagaccaatagaaactgggcttgtcgagacagagaagactcttgcgtttctgataggcacctattggtcttactgacatccactttgcctttctctccacaggtgtccactcccagttcaattacagctcttaaggctagagtacttaatacgactcactataggctagcatttaggtgacactatagaatacaagctacttgttctttttgcactcgagaattcatggccctgtggatgcgcctcctgcccctgctggcgctgctggccctctggggacctgacccagccgcagcctttgtgaaccaacacctgtgcggctcacacctggtggaagctctctacctagtgtgcggggaacgaggcttcttctacacacccaagacccgccggaagcgggaggacctgcaggtggggcaggtggagctgggcgggggcccaggccctggtgcaggcagcctgcagcccttggccctggaggggtcccgacgcaagcgtatggtcttcacactcgaagatttcgttggggactggcgacagacagccggctacaacctggaccaagtccttgaacagggaggtgtgtccagtttgtttcagaatctcggggtgtccgtaactccgatccaaaggattgtcctgagcggtgaaaatgggctgaagatcgacatccatgtcatcatcccgtatgaaggtctgagcggcgaccaaatgggccagatcgaaaaaatttttaaggtggtgtaccctgtggatgatcatcactttaaggtgatcctgcactatggcacactggtaatcgacggggttacgccgaacatgatcgactatttcggacggccgtatgaaggcatcgccgtgttcgacggcaaaaagatcactgtaacagggaccctgtggaacggcaacaaaattatcgacgagcgcctgatcaaccccgacggctccctgctgttccgagtaaccatcaacggagtgaccggctggcggctgtgcgaacgcattctggcggctgctgctgcgggcattgtggaacaatgctgtaccagcatctgctccgcctaccagctggagaactactgcaactaggaattcacgcgtggtacctctagagtcgacccgggcggccgcttcgagcagacatgataagatacattgatgagtttggacaaaccacaactagaatgcagtgaaaaaaatgctttatttgtgaaatttgtgatgctattgctttatttgtaaccattataagctgcaataaacaagttaacaacaacaattgcattcattttatgtttcaggttcagggggagatgtgggaggttttttaaagcaagtaaaacctctacaaatgtggtaaaatcgataaggatccgggctggcgtaatagcgaagaggcccgcaccgatcgcccttcccaacagttgcgcagcctgaatggcgaatggacgcgccctgtagcggcgcattaagcgcggcgggtgtggtggttacgcgcagcgtgaccgctacacttgccagcgccctagcgcccgctcctttcgctttcttcccttcctttctcgccacgttcgccggctttccccgtcaagctctaaatcgggggctccctttagggttccgatttagtgctttacggcacctcgaccccaaaaaacttgattagggtgatggttcacgtagtgggccatcgccctgatagacggtttttcgccctttgacgttggagtccacgttctttaatagtggactcttgttccaaactggaacaacactcaaccctatctcggtctattcttttgatttataagggattttgccgatttcggcctattggttaaaaaatgagctgatttaacaaaaatttaacgcgaattttaacaaaatattaacgcttacaatttcctgatgcggtattttctccttacgcatctgtgcggtatttcacaccgcatatggtgcactctcagtacaatctgctctgatgccgcatagttaagccagccccgacacccgccaacacccgctgacgcgccctgacgggcttgtctgctcccggcatccgcttacagacaagctgtgaccgtctccgggagctgcatgtgtcagaggttttcaccgtcatcaccgaaacgcgcgagacgaaagggcctcgtgatacgcctatttttataggttaatgtcatgataataatggtttcttagacgtcaggtggcacttttcggggaaatgtgcgcggaacccctatttgtttatttttctaaatacattcaaatatgtatccgctcatgagacaataaccctgataaatgcttcaataatattgaaaaaggaagagtatgagtattcaacatttccgtgtcgcccttattcccttttttgcggcattttgccttcctgtttttgctcacccagaaacgctggtgaaagtaaaagatgctgaagatcagttgggtgcacgagtgggttacatcgaactggatctcaacagcggtaagatccttgagagttttcgccccgaagaacgttttccaatgatgagcacttttaaagttctgctatgtggcgcggtattatcccgtattgacgccgggcaagagcaactcggtcgccgcatacactattctcagaatgacttggttgagtactcaccagtcacagaaaagcatcttacggatggcatgacagtaagagaattatgcagtgctgccataaccatgagtgataacactgcggccaacttacttctgacaacgatcggaggaccgaaggagctaaccgcttttttgcacaacatgggggatcatgtaactcgccttgatcgttgggaaccggagctgaatgaagccataccaaacgacgagcgtgacaccacgatgcctgtagcaatggcaacaacgttgcgcaaactattaactggcgaactacttactctagcttcccggcaacaattaatagactggatggaggcggataaagttgcaggaccacttctgcgctcggcccttccggctggctggtttattgctgataaatctggagccggtgagcgtgggtctcgcggtatcattgcagcactggggccagatggtaagccctcccgtatcgtagttatctacacgacggggagtcaggcaactatggatgaacgaaatagacagatcgctgagataggtgcctcactgattaagcattggtaactgtcagaccaagtttactcatatatactttagattgatttaaaacttcatttttaatttaaaaggatctaggtgaagatcctttttgataatctcatgaccaaaatcccttaacgtgagttttcgttccactgagcgtcagaccccgtagaaaagatcaaaggatcttcttgagatcctttttttctgcgcgtaatctgctgcttgcaaacaaaaaaaccaccgctaccagcggtggtttgtttgccggatcaagagctaccaactctttttccgaaggtaactggcttcagcagagcgcagataccaaatactgttcttctagtgtagccgtagttaggccaccacttcaagaactctgtagcaccgcctacatacctcgctctgctaatcctgttaccagtggctgctgccagtggcgataagtcgtgtcttaccgggttggactcaagacgatagttaccggataaggcgcagcggtcgggctgaacggggggttcgtgcacacagcccagcttggagcgaacgacctacaccgaactgagatacctacagcgtgagctatgagaaagcgccacgcttcccgaagggagaaaggcggacaggtatccggtaagcggcagggtcggaacaggagagcgcacgagggagcttccagggggaaacgcctggtatctttatagtcctgtcgggtttcgccacctctgacttgagcgtcgatttttgtgatgctcgtcaggggggcggagcctatggaaaaacgccagcaacgcggcctttttacggttcctggccttttgctggccttttgctcacatggctcgacagatct

SEQ ID NO: 53 - DNA, 4920 bp, synthetic construct
  source 1..4920: mol_type = other DNA; note = pCMVTnT insulin Nluc-Achain B chain F1A
tcaatattggccattagccatattattcattggttatatagcataaatcaatattggctattggccattgcatacgttgtatctatatcataatatgtacatttatattggctcatgtccaatatgaccgccatgttggcattgattattgactagttattaatagtaatcaattacggggtcattagttcatagcccatatatggagttccgcgttacataacttacggtaaatggcccgcctggctgaccgcccaacgacccccgcccattgacgtcaataatgacgtatgttcccatagtaacgccaatagggactttccattgacgtcaatgggtggagtatttacggtaaactgcccacttggcagtacatcaagtgtatcatatgccaagtccgccccctattgacgtcaatgacggtaaatggcccgcctggcattatgcccagtacatgaccttacgggactttcctacttggcagtacatctacgtattagtcatcgctattaccatggtgatgcggttttggcagtacaccaatgggcgtggatagcggtttgactcacggggatttccaagtctccaccccattgacgtcaatgggagtttgttttggcaccaaaatcaacgggactttccaaaatgtcgtaataaccccgccccgttgacgcaaatgggcggtaggcgtgtacggtgggaggtctatataagcagagctcgtttagtgaaccgtcagatcactagaagctttattgcggtagtttatcacagttaaattgctaacgcagtcagtgcttctgacacaacagtctcgaacttaagctgcagaagttggtcgtgaggcactgggcaggtaagtatcaaggttacaagacaggtttaaggagaccaatagaaactgggcttgtcgagacagagaagactcttgcgtttctgataggcacctattggtcttactgacatccactttgcctttctctccacaggtgtccactcccagttcaattacagctcttaaggctagagtacttaatacgactcactataggctagcatttaggtgacactatagaatacaagctacttgttctttttgcactcgagaattcatggccctgtggatgcgcctcctgcccctgctggcgctgctggccctctggggacctgacccagccgcagccgctgtgaaccaacacctgtgcggctcacacctggtggaagctctctacctagtgtgcggggaacgaggcttcttctacacacccaagacccgccggaagcgggaggacctgcaggtggggcaggtggagctgggcgggggcccaggccctggtgcaggcagcctgcagcccttggccctggaggggtcccgacgcaagcgtatggtcttcacactcgaagatttcgttggggactggcgacagacagccggctacaacctggaccaagtccttgaacagggaggtgtgtccagtttgtttcagaatctcggggtgtccgtaactccgatccaaaggattgtcctgagcggtgaaaatgggctgaagatcgacatccatgtcatcatcccgtatgaaggtctgagcggcgaccaaatgggccagatcgaaaaaatttttaaggtggtgtaccctgtggatgatcatcactttaaggtgatcctgcactatggcacactggtaatcgacggggttacgccgaacatgatcgactatttcggacggccgtatgaaggcatcgccgtgttcgacggcaaaaagatcactgtaacagggaccctgtggaacggcaacaaaattatcgacgagcgcctgatcaaccccgacggctccctgctgttccgagtaaccatcaacggagtgaccggctggcggctgtgcgaacgcattctggcggctgctgctgcgggcattgtggaacaatgctgtaccagcatctgctccctctaccagctggagaactactgcaactaggaattcacgcgtggtacctctagagtcgacccgggcggccgcttcgagcagacatgataagatacattgatgagtttggacaaaccacaactagaatgcagtgaaaaaaatgctttatttgtgaaatttgtgatgctattgctttatttgtaaccattataagctgcaataaacaagttaacaacaacaattgcattcattttatgtttcaggttcagggggagatgtgggaggttttttaaagcaagtaaaacctctacaaatgtggtaaaatcgataaggatccgggctggcgtaatagcgaagaggcccgcaccgatcgcccttcccaacagttgcgcagcctgaatggcgaatggacgcgccctgtagcggcgcattaagcgcggcgggtgtggtggttacgcgcagcgtgaccgctacacttgccagcgccctagcgcccgctcctttcgctttcttcccttcctttctcgccacgttcgccggctttccccgtcaagctctaaatcgggggctccctttagggttccgatttagtgctttacggcacctcgaccccaaaaaacttgattagggtgatggttcacgtagtgggccatcgccctgatagacggtttttcgccctttgacgttggagtccacgttctttaatagtggactcttgttccaaactggaacaacactcaaccctatctcggtctattcttttgatttataagggattttgccgatttcggcctattggttaaaaaatgagctgatttaacaaaaatttaacgcgaattttaacaaaatattaacgcttacaatttcctgatgcggtattttctccttacgcatctgtgcggtatttcacaccgcatatggtgcactctcagtacaatctgctctgatgccgcatagttaagccagccccgacacccgccaacacccgctgacgcgccctgacgggcttgtctgctcccggcatccgcttacagacaagctgtgaccgtctccgggagctgcatgtgtcagaggttttcaccgtcatcaccgaaacgcgcgagacgaaagggcctcgtgatacgcctatttttataggttaatgtcatgataataatggtttcttagacgtcaggtggcacttttcggggaaatgtgcgcggaacccctatttgtttatttttctaaatacattcaaatatgtatccgctcatgagacaataaccctgataaatgcttcaataatattgaaaaaggaagagtatgagtattcaacatttccgtgtcgcccttattcccttttttgcggcattttgccttcctgtttttgctcacccagaaacgctggtgaaagtaaaagatgctgaagatcagttgggtgcacgagtgggttacatcgaactggatctcaacagcggtaagatccttgagagttttcgccccgaagaacgttttccaatgatgagcacttttaaagttctgctatgtggcgcggtattatcccgtattgacgccgggcaagagcaactcggtcgccgcatacactattctcagaatgacttggttgagtactcaccagtcacagaaaagcatcttacggatggcatgacagtaagagaattatgcagtgctgccataaccatgagtgataacactgcggccaacttacttctgacaacgatcggaggaccgaaggagctaaccgcttttttgcacaacatgggggatcatgtaactcgccttgatcgttgggaaccggagctgaatgaagccataccaaacgacgagcgtgacaccacgatgcctgtagcaatggcaacaacgttgcgcaaactattaactggcgaactacttactctagcttcccggcaacaattaatagactggatggaggcggataaagttgcaggaccacttctgcgctcggcccttccggctggctggtttattgctgataaatctggagccggtgagcgtgggtctcgcggtatcattgcagcactggggccagatggtaagccctcccgtatcgtagttatctacacgacggggagtcaggcaactatggatgaacgaaatagacagatcgctgagataggtgcctcactgattaagcattggtaactgtcagaccaagtttactcatatatactttagattgatttaaaacttcatttttaatttaaaaggatctaggtgaagatcctttttgataatctcatgaccaaaatcccttaacgtgagttttcgttccactgagcgtcagaccccgtagaaaagatcaaaggatcttcttgagatcctttttttctgcgcgtaatctgctgcttgcaaacaaaaaaaccaccgctaccagcggtggtttgtttgccggatcaagagctaccaactctttttccgaaggtaactggcttcagcagagcgcagataccaaatactgttcttctagtgtagccgtagttaggccaccacttcaagaactctgtagcaccgcctacatacctcgctctgctaatcctgttaccagtggctgctgccagtggcgataagtcgtgtcttaccgggttggactcaagacgatagttaccggataaggcgcagcggtcgggctgaacggggggttcgtgcacacagcccagcttggagcgaacgacctacaccgaactgagatacctacagcgtgagctatgagaaagcgccacgcttcccgaagggagaaaggcggacaggtatccggtaagcggcagggtcggaacaggagagcgcacgagggagcttccagggggaaacgcctggtatctttatagtcctgtcgggtttcgccacctctgacttgagcgtcgatttttgtgatgctcgtcaggggggcggagcctatggaaaaacgccagcaacgcggcctttttacggttcctggccttttgctggccttttgctcacatggctcgacagatct

SEQ ID NO: 54 - DNA, 4920 bp, synthetic construct
  source 1..4920: mol_type = other DNA; note = pCMVTnT insulin Nluc-Achain B L17A
tcaatattggccattagccatattattcattggttatatagcataaatcaatattggctattggccattgcatacgttgtatctatatcataatatgtacatttatattggctcatgtccaatatgaccgccatgttggcattgattattgactagttattaatagtaatcaattacggggtcattagttcatagcccatatatggagttccgcgttacataacttacggtaaatggcccgcctggctgaccgcccaacgacccccgcccattgacgtcaataatgacgtatgttcccatagtaacgccaatagggactttccattgacgtcaatgggtggagtatttacggtaaactgcccacttggcagtacatcaagtgtatcatatgccaagtccgccccctattgacgtcaatgacggtaaatggcccgcctggcattatgcccagtacatgaccttacgggactttcctacttggcagtacatctacgtattagtcatcgctattaccatggtgatgcggttttggcagtacaccaatgggcgtggatagcggtttgactcacggggatttccaagtctccaccccattgacgtcaatgggagtttgttttggcaccaaaatcaacgggactttccaaaatgtcgtaataaccccgccccgttgacgcaaatgggcggtaggcgtgtacggtgggaggtctatataagcagagctcgtttagtgaaccgtcagatcactagaagctttattgcggtagtttatcacagttaaattgctaacgcagtcagtgcttctgacacaacagtctcgaacttaagctgcagaagttggtcgtgaggcactgggcaggtaagtatcaaggttacaagacaggtttaaggagaccaatagaaactgggcttgtcgagacagagaagactcttgcgtttctgataggcacctattggtcttactgacatccactttgcctttctctccacaggtgtccactcccagttcaattacagctcttaaggctagagtacttaatacgactcactataggctagcatttaggtgacactatagaatacaagctacttgttctttttgcactcgagaattcatggccctgtggatgcgcctcctgcccctgctggcgctgctggccctctggggacctgacccagccgcagcctttgtgaaccaacacctgtgcggctcacacctggtggaagctctctacgcagtgtgcggggaacgaggcttcttctacacacccaagacccgccggaagcgggaggacctgcaggtggggcaggtggagctgggcgggggcccaggccctggtgcaggcagcctgcagcccttggccctggaggggtcccgacgcaagcgtatggtcttcacactcgaagatttcgttggggactggcgacagacagccggctacaacctggaccaagtccttgaacagggaggtgtgtccagtttgtttcagaatctcggggtgtccgtaactccgatccaaaggattgtcctgagcggtgaaaatgggctgaagatcgacatccatgtcatcatcccgtatgaaggtctgagcggcgaccaaatgggccagatcgaaaaaatttttaaggtggtgtaccctgtggatgatcatcactttaaggtgatcctgcactatggcacactggtaatcgacggggttacgccgaacatgatcgactatttcggacggccgtatgaaggcatcgccgtgttcgacggcaaaaagatcactgtaacagggaccctgtggaacggcaacaaaattatcgacgagcgcctgatcaaccccgacggctccctgctgttccgagtaaccatcaacggagtgaccggctggcggctgtgcgaacgcattctggcggctgctgctgcgggcattgtggaacaatgctgtaccagcatctgctccctctaccagctggagaactactgcaactaggaattcacgcgtggtacctctagagtcgacccgggcggccgcttcgagcagacatgataagatacattgatgagtttggacaaaccacaactagaatgcagtgaaaaaaatgctttatttgtgaaatttgtgatgctattgctttatttgtaaccattataagctgcaataaacaagttaacaacaacaattgcattcattttatgtttcaggttcagggggagatgtgggaggttttttaaagcaagtaaaacctctacaaatgtggtaaaatcgataaggatccgggctggcgtaatagcgaagaggcccgcaccgatcgcccttcccaacagttgcgcagcctgaatggcgaatggacgcgccctgtagcggcgcattaagcgcggcgggtgtggtggttacgcgcagcgtgaccgctacacttgccagcgccctagcgcccgctcctttcgctttcttcccttcctttctcgccacgttcgccggctttccccgtcaagctctaaatcgggggctccctttagggttccgatttagtgctttacggcacctcgaccccaaaaaacttgattagggtgatggttcacgtagtgggccatcgccctgatagacggtttttcgccctttgacgttggagtccacgttctttaatagtggactcttgttccaaactggaacaacactcaaccctatctcggtctattcttttgatttataagggattttgccgatttcggcctattggttaaaaaatgagctgatttaacaaaaatttaacgcgaattttaacaaaatattaacgcttacaatttcctgatgcggtattttctccttacgcatctgtgcggtatttcacaccgcatatggtgcactctcagtacaatctgctctgatgccgcatagttaagccagccccgacacccgccaacacccgctgacgcgccctgacgggcttgtctgctcccggcatccgcttacagacaagctgtgaccgtctccgggagctgcatgtgtcagaggttttcaccgtcatcaccgaaacgcgcgagacgaaagggcctcgtgatacgcctatttttataggttaatgtcatgataataatggtttcttagacgtcaggtggcacttttcggggaaatgtgcgcggaacccctatttgtttatttttctaaatacattcaaatatgtatccgctcatgagacaataaccctgataaatgcttcaataatattgaaaaaggaagagtatgagtattcaacatttccgtgtcgcccttattcccttttttgcggcattttgccttcctgtttttgctcacccagaaacgctggtgaaagtaaaagatgctgaagatcagttgggtgcacgagtgggttacatcgaactggatctcaacagcggtaagatccttgagagttttcgccccgaagaacgttttccaatgatgagcacttttaaagttctgctatgtggcgcggtattatcccgtattgacgccgggcaagagcaactcggtcgccgcatacactattctcagaatgacttggttgagtactcaccagtcacagaaaagcatcttacggatggcatgacagtaagagaattatgcagtgctgccataaccatgagtgataacactgcggccaacttacttctgacaacgatcggaggaccgaaggagctaaccgcttttttgcacaacatgggggatcatgtaactcgccttgatcgttgggaaccggagctgaatgaagccataccaaacgacgagcgtgacaccacgatgcctgtagcaatggcaacaacgttgcgcaaactattaactggcgaactacttactctagcttcccggcaacaattaatagactggatggaggcggataaagttgcaggaccacttctgcgctcggcccttccggctggctggtttattgctgataaatctggagccggtgagcgtgggtctcgcggtatcattgcagcactggggccagatggtaagccctcccgtatcgtagttatctacacgacggggagtcaggcaactatggatgaacgaaatagacagatcgctgagataggtgcctcactgattaagcattggtaactgtcagaccaagtttactcatatatactttagattgatttaaaacttcatttttaatttaaaaggatctaggtgaagatcctttttgataatctcatgaccaaaatcccttaacgtgagttttcgttccactgagcgtcagaccccgtagaaaagatcaaaggatcttcttgagatcctttttttctgcgcgtaatctgctgcttgcaaacaaaaaaaccaccgctaccagcggtggtttgtttgccggatcaagagctaccaactctttttccgaaggtaactggcttcagcagagcgcagataccaaatactgttcttctagtgtagccgtagttaggccaccacttcaagaactctgtagcaccgcctacatacctcgctctgctaatcctgttaccagtggctgctgccagtggcgataagtcgtgtcttaccgggttggactcaagacgatagttaccggataaggcgcagcggtcgggctgaacggggggttcgtgcacacagcccagcttggagcgaacgacctacaccgaactgagatacctacagcgtgagctatgagaaagcgccacgcttcccgaagggagaaaggcggacaggtatccggtaagcggcagggtcggaacaggagagcgcacgagggagcttccagggggaaacgcctggtatctttatagtcctgtcgggtttcgccacctctgacttgagcgtcgatttttgtgatgctcgtcaggggggcggagcctatggaaaaacgccagcaacgcggcctttttacggttcctggccttttgctggccttttgctcacatggctcgacagatct

SEQ ID NO: 55 - DNA, 4920 bp, synthetic construct
  source 1..4920: mol_type = other DNA; note = pCMVTnT insulin Nluc-Achain B R22A
tcaatattggccattagccatattattcattggttatatagcataaatcaatattggctattggccattgcatacgttgtatctatatcataatatgtacatttatattggctcatgtccaatatgaccgccatgttggcattgattattgactagttattaatagtaatcaattacggggtcattagttcatagcccatatatggagttccgcgttacataacttacggtaaatggcccgcctggctgaccgcccaacgacccccgcccattgacgtcaataatgacgtatgttcccatagtaacgccaatagggactttccattgacgtcaatgggtggagtatttacggtaaactgcccacttggcagtacatcaagtgtatcatatgccaagtccgccccctattgacgtcaatgacggtaaatggcccgcctggcattatgcccagtacatgaccttacgggactttcctacttggcagtacatctacgtattagtcatcgctattaccatggtgatgcggttttggcagtacaccaatgggcgtggatagcggtttgactcacggggatttccaagtctccaccccattgacgtcaatgggagtttgttttggcaccaaaatcaacgggactttccaaaatgtcgtaataaccccgccccgttgacgcaaatgggcggtaggcgtgtacggtgggaggtctatataagcagagctcgtttagtgaaccgtcagatcactagaagctttattgcggtagtttatcacagttaaattgctaacgcagtcagtgcttctgacacaacagtctcgaacttaagctgcagaagttggtcgtgaggcactgggcaggtaagtatcaaggttacaagacaggtttaaggagaccaatagaaactgggcttgtcgagacagagaagactcttgcgtttctgataggcacctattggtcttactgacatccactttgcctttctctccacaggtgtccactcccagttcaattacagctcttaaggctagagtacttaatacgactcactataggctagcatttaggtgacactatagaatacaagctacttgttctttttgcactcgagaattcatggccctgtggatgcgcctcctgcccctgctggcgctgctggccctctggggacctgacccagccgcagcctttgtgaaccaacacctgtgcggctcacacctggtggaagctctctacctagtgtgcggggaacgaggcttcttctacacacccaagacccgccggaagcgggaggacctgcaggtggggcaggtggagctgggcgggggcccaggccctggtgcaggcagcctgcagcccttggccctggaggggtcccgacgcaagcgtatggtcttcacactcgaagatttcgttggggactggcgacagacagccggctacaacctggaccaagtccttgaacagggaggtgtgtccagtttgtttcagaatctcggggtgtccgtaactccgatccaaaggattgtcctgagcggtgaaaatgggctgaagatcgacatccatgtcatcatcccgtatgaaggtctgagcggcgaccaaatgggccagatcgaaaaaatttttaaggtggtgtaccctgtggatgatcatcactttaaggtgatcctgcactatggcacactggtaatcgacggggttacgccgaacatgatcgactatttcggacggccgtatgaaggcatcgccgtgttcgacggcaaaaagatcactgtaacagggaccctgtggaacggcaacaaaattatcgacgagcgcctgatcaaccccgacggctccctgctgttccgagtaaccatcaacggagtgaccggctggcggctgtgcgaacgcattctggcggctgctgctgcgggcattgtggaacaatgctgtaccagcatctgctccctctaccagctggagaactactgcaactaggaattcacgcgtggtacctctagagtcgacccgggcggccgcttcgagcagacatgataagatacattgatgagtttggacaaaccacaactagaatgcagtgaaaaaaatgctttatttgtgaaatttgtgatgctattgctttatttgtaaccattataagctgcaataaacaagttaacaacaacaattgcattcattttatgtttcaggttcagggggagatgtgggaggttttttaaagcaagtaaaacctctacaaatgtggtaaaatcgataaggatccgggctggcgtaatagcgaagaggcccgcaccgatcgcccttcccaacagttgcgcagcctgaatggcgaatggacgcgccctgtagcggcgcattaagcgcggcgggtgtggtggttacgcgcagcgtgaccgctacacttgccagcgccctagcgcccgctcctttcgctttcttcccttcctttctcgccacgttcgccggctttccccgtcaagctctaaatcgggggctccctttagggttccgatttagtgctttacggcacctcgaccccaaaaaacttgattagggtgatggttcacgtagtgggccatcgccctgatagacggtttttcgccctttgacgttggagtccacgttctttaatagtggactcttgttccaaactggaacaacactcaaccctatctcggtctattcttttgatttataagggattttgccgatttcggcctattggttaaaaaatgagctgatttaacaaaaatttaacgcgaattttaacaaaatattaacgcttacaatttcctgatgcggtattttctccttacgcatctgtgcggtatttcacaccgcatatggtgcactctcagtacaatctgctctgatgccgcatagttaagccagccccgacacccgccaacacccgctgacgcgccctgacgggcttgtctgctcccggcatccgcttacagacaagctgtgaccgtctccgggagctgcatgtgtcagaggttttcaccgtcatcaccgaaacgcgcgagacgaaagggcctcgtgatacgcctatttttataggttaatgtcatgataataatggtttcttagacgtcaggtggcacttttcggggaaatgtgcgcggaacccctatttgtttatttttctaaatacattcaaatatgtatccgctcatgagacaataaccctgataaatgcttcaataatattgaaaaaggaagagtatgagtattcaacatttccgtgtcgcccttattcccttttttgcggcattttgccttcctgtttttgctcacccagaaacgctggtgaaagtaaaagatgctgaagatcagttgggtgcacgagtgggttacatcgaactggatctcaacagcggtaagatccttgagagttttcgccccgaagaacgttttccaatgatgagcacttttaaagttctgctatgtggcgcggtattatcccgtattgacgccgggcaagagcaactcggtcgccgcatacactattctcagaatgacttggttgagtactcaccagtcacagaaaagcatcttacggatggcatgacagtaagagaattatgcagtgctgccataaccatgagtgataacactgcggccaacttacttctgacaacgatcggaggaccgaaggagctaaccgcttttttgcacaacatgggggatcatgtaactcgccttgatcgttgggaaccggagctgaatgaagccataccaaacgacgagcgtgacaccacgatgcctgtagcaatggcaacaacgttgcgcaaactattaactggcgaactacttactctagcttcccggcaacaattaatagactggatggaggcggataaagttgcaggaccacttctgcgctcggcccttccggctggctggtttattgctgataaatctggagccggtgagcgtgggtctcgcggtatcattgcagcactggggccagatggtaagccctcccgtatcgtagttatctacacgacggggagtcaggcaactatggatgaacgaaatagacagatcgctgagataggtgcctcactgattaagcattggtaactgtcagaccaagtttactcatatatactttagattgatttaaaacttcatttttaatttaaaaggatctaggtgaagatcctttttgataatctcatgaccaaaatcccttaacgtgagttttcgttccactgagcgtcagaccccgtagaaaagatcaaaggatcttcttgagatcctttttttctgcgcgtaatctgctgcttgcaaacaaaaaaaccaccgctaccagcggtggtttgtttgccggatcaagagctaccaactctttttccgaaggtaactggcttcagcagagcgcagataccaaatactgttcttctagtgtagccgtagttaggccaccacttcaagaactctgtagcaccgcctacatacctcgctctgctaatcctgttaccagtggctgctgccagtggcgataagtcgtgtcttaccgggttggactcaagacgatagttaccggataaggcgcagcggtcgggctgaacggggggttcgtgcacacagcccagcttggagcgaacgacctacaccgaactgagatacctacagcgtgagctatgagaaagcgccacgcttcccgaagggagaaaggcggacaggtatccggtaagcggcagggtcggaacaggagagcgcacgagggagcttccagggggaaacgcctggtatctttatagtcctgtcgggtttcgccacctctgacttgagcgtcgatttttgtgatgctcgtcaggggggcggagcctatggaaaaacgccagcaacgcggcctttttacggttcctggccttttgctggccttttgctcacatggctcgacagatct

SEQ ID NO: 56 - DNA, 4920 bp, synthetic construct
  source 1..4920: mol_type = other DNA; note = pCMVTnT insulin Nluc-Achain Bchain V2G
tcaatattggccattagccatattattcattggttatatagcataaatcaatattggctattggccattgcatacgttgtatctatatcataatatgtacatttatattggctcatgtccaatatgaccgccatgttggcattgattattgactagttattaatagtaatcaattacggggtcattagttcatagcccatatatggagttccgcgttacataacttacggtaaatggcccgcctggctgaccgcccaacgacccccgcccattgacgtcaataatgacgtatgttcccatagtaacgccaatagggactttccattgacgtcaatgggtggagtatttacggtaaactgcccacttggcagtacatcaagtgtatcatatgccaagtccgccccctattgacgtcaatgacggtaaatggcccgcctggcattatgcccagtacatgaccttacgggactttcctacttggcagtacatctacgtattagtcatcgctattaccatggtgatgcggttttggcagtacaccaatgggcgtggatagcggtttgactcacggggatttccaagtctccaccccattgacgtcaatgggagtttgttttggcaccaaaatcaacgggactttccaaaatgtcgtaataaccccgccccgttgacgcaaatgggcggtaggcgtgtacggtgggaggtctatataagcagagctcgtttagtgaaccgtcagatcactagaagctttattgcggtagtttatcacagttaaattgctaacgcagtcagtgcttctgacacaacagtctcgaacttaagctgcagaagttggtcgtgaggcactgggcaggtaagtatcaaggttacaagacaggtttaaggagaccaatagaaactgggcttgtcgagacagagaagactcttgcgtttctgataggcacctattggtcttactgacatccactttgcctttctctccacaggtgtccactcccagttcaattacagctcttaaggctagagtacttaatacgactcactataggctagcatttaggtgacactatagaatacaagctacttgttctttttgcactcgagaattcatggccctgtggatgcgcctcctgcccctgctggcgctgctggccctctggggacctgacccagccgcagcctttgggaaccaacacctgtgcggctcacacctggtggaagctctctacctagtgtgcggggaacgaggcttcttctacacacccaagacccgccggaagcgggaggacctgcaggtggggcaggtggagctgggcgggggcccaggccctggtgcaggcagcctgcagcccttggccctggaggggtcccgacgcaagcgtatggtcttcacactcgaagatttcgttggggactggcgacagacagccggctacaacctggaccaagtccttgaacagggaggtgtgtccagtttgtttcagaatctcggggtgtccgtaactccgatccaaaggattgtcctgagcggtgaaaatgggctgaagatcgacatccatgtcatcatcccgtatgaaggtctgagcggcgaccaaatgggccagatcgaaaaaatttttaaggtggtgtaccctgtggatgatcatcactttaaggtgatcctgcactatggcacactggtaatcgacggggttacgccgaacatgatcgactatttcggacggccgtatgaaggcatcgccgtgttcgacggcaaaaagatcactgtaacagggaccctgtggaacggcaacaaaattatcgacgagcgcctgatcaaccccgacggctccctgctgttccgagtaaccatcaacggagtgaccggctggcggctgtgcgaacgcattctggcggctgctgctgcgggcattgtggaacaatgctgtaccagcatctgctccctctaccagctggagaactactgcaactaggaattcacgcgtggtacctctagagtcgacccgggcggccgcttcgagcagacatgataagatacattgatgagtttggacaaaccacaactagaatgcagtgaaaaaaatgctttatttgtgaaatttgtgatgctattgctttatttgtaaccattataagctgcaataaacaagttaacaacaacaattgcattcattttatgtttcaggttcagggggagatgtgggaggttttttaaagcaagtaaaacctctacaaatgtggtaaaatcgataaggatccgggctggcgtaatagcgaagaggcccgcaccgatcgcccttcccaacagttgcgcagcctgaatggcgaatggacgcgccctgtagcggcgcattaagcgcggcgggtgtggtggttacgcgcagcgtgaccgctacacttgccagcgccctagcgcccgctcctttcgctttcttcccttcctttctcgccacgttcgccggctttccccgtcaagctctaaatcgggggctccctttagggttccgatttagtgctttacggcacctcgaccccaaaaaacttgattagggtgatggttcacgtagtgggccatcgccctgatagacggtttttcgccctttgacgttggagtccacgttctttaatagtggactcttgttccaaactggaacaacactcaaccctatctcggtctattcttttgatttataagggattttgccgatttcggcctattggttaaaaaatgagctgatttaacaaaaatttaacgcgaattttaacaaaatattaacgcttacaatttcctgatgcggtattttctccttacgcatctgtgcggtatttcacaccgcatatggtgcactctcagtacaatctgctctgatgccgcatagttaagccagccccgacacccgccaacacccgctgacgcgccctgacgggcttgtctgctcccggcatccgcttacagacaagctgtgaccgtctccgggagctgcatgtgtcagaggttttcaccgtcatcaccgaaacgcgcgagacgaaagggcctcgtgatacgcctatttttataggttaatgtcatgataataatggtttcttagacgtcaggtggcacttttcggggaaatgtgcgcggaacccctatttgtttatttttctaaatacattcaaatatgtatccgctcatgagacaataaccctgataaatgcttcaataatattgaaaaaggaagagtatgagtattcaacatttccgtgtcgcccttattcccttttttgcggcattttgccttcctgtttttgctcacccagaaacgctggtgaaagtaaaagatgctgaagatcagttgggtgcacgagtgggttacatcgaactggatctcaacagcggtaagatccttgagagttttcgccccgaagaacgttttccaatgatgagcacttttaaagttctgctatgtggcgcggtattatcccgtattgacgccgggcaagagcaactcggtcgccgcatacactattctcagaatgacttggttgagtactcaccagtcacagaaaagcatcttacggatggcatgacagtaagagaattatgcagtgctgccataaccatgagtgataacactgcggccaacttacttctgacaacgatcggaggaccgaaggagctaaccgcttttttgcacaacatgggggatcatgtaactcgccttgatcgttgggaaccggagctgaatgaagccataccaaacgacgagcgtgacaccacgatgcctgtagcaatggcaacaacgttgcgcaaactattaactggcgaactacttactctagcttcccggcaacaattaatagactggatggaggcggataaagttgcaggaccacttctgcgctcggcccttccggctggctggtttattgctgataaatctggagccggtgagcgtgggtctcgcggtatcattgcagcactggggccagatggtaagccctcccgtatcgtagttatctacacgacggggagtcaggcaactatggatgaacgaaatagacagatcgctgagataggtgcctcactgattaagcattggtaactgtcagaccaagtttactcatatatactttagattgatttaaaacttcatttttaatttaaaaggatctaggtgaagatcctttttgataatctcatgaccaaaatcccttaacgtgagttttcgttccactgagcgtcagaccccgtagaaaagatcaaaggatcttcttgagatcctttttttctgcgcgtaatctgctgcttgcaaacaaaaaaaccaccgctaccagcggtggtttgtttgccggatcaagagctaccaactctttttccgaaggtaactggcttcagcagagcgcagataccaaatactgttcttctagtgtagccgtagttaggccaccacttcaagaactctgtagcaccgcctacatacctcgctctgctaatcctgttaccagtggctgctgccagtggcgataagtcgtgtcttaccgggttggactcaagacgatagttaccggataaggcgcagcggtcgggctgaacggggggttcgtgcacacagcccagcttggagcgaacgacctacaccgaactgagatacctacagcgtgagctatgagaaagcgccacgcttcccgaagggagaaaggcggacaggtatccggtaagcggcagggtcggaacaggagagcgcacgagggagcttccagggggaaacgcctggtatctttatagtcctgtcgggtttcgccacctctgacttgagcgtcgatttttgtgatgctcgtcaggggggcggagcctatggaaaaacgccagcaacgcggcctttttacggttcctggccttttgctggccttttgctcacatggctcgacagatct

SEQ ID NO: 57 - DNA, 4905 bp, synthetic construct
  source 1..4905: mol_type = other DNA; note = pCMVTnT insulin Nluc-Achain del B26-30
tcaatattggccattagccatattattcattggttatatagcataaatcaatattggctattggccattgcatacgttgtatctatatcataatatgtacatttatattggctcatgtccaatatgaccgccatgttggcattgattattgactagttattaatagtaatcaattacggggtcattagttcatagcccatatatggagttccgcgttacataacttacggtaaatggcccgcctggctgaccgcccaacgacccccgcccattgacgtcaataatgacgtatgttcccatagtaacgccaatagggactttccattgacgtcaatgggtggagtatttacggtaaactgcccacttggcagtacatcaagtgtatcatatgccaagtccgccccctattgacgtcaatgacggtaaatggcccgcctggcattatgcccagtacatgaccttacgggactttcctacttggcagtacatctacgtattagtcatcgctattaccatggtgatgcggttttggcagtacaccaatgggcgtggatagcggtttgactcacggggatttccaagtctccaccccattgacgtcaatgggagtttgttttggcaccaaaatcaacgggactttccaaaatgtcgtaataaccccgccccgttgacgcaaatgggcggtaggcgtgtacggtgggaggtctatataagcagagctcgtttagtgaaccgtcagatcactagaagctttattgcggtagtttatcacagttaaattgctaacgcagtcagtgcttctgacacaacagtctcgaacttaagctgcagaagttggtcgtgaggcactgggcaggtaagtatcaaggttacaagacaggtttaaggagaccaatagaaactgggcttgtcgagacagagaagactcttgcgtttctgataggcacctattggtcttactgacatccactttgcctttctctccacaggtgtccactcccagttcaattacagctcttaaggctagagtacttaatacgactcactataggctagcatttaggtgacactatagaatacaagctacttgttctttttgcactcgagaattcatggccctgtggatgcgcctcctgcccctgctggcgctgctggccctctggggacctgacccagccgcagcctttgtgaaccaacacctgtgcggctcacacctggtggaagctctctacctagtgtgcggggaacgaggcttcttccgccggaagcgggaggacctgcaggtggggcaggtggagctgggcgggggcccaggccctggtgcaggcagcctgcagcccttggccctggaggggtcccgacgcaagcgtatggtcttcacactcgaagatttcgttggggactggcgacagacagccggctacaacctggaccaagtccttgaacagggaggtgtgtccagtttgtttcagaatctcggggtgtccgtaactccgatccaaaggattgtcctgagcggtgaaaatgggctgaagatcgacatccatgtcatcatcccgtatgaaggtctgagcggcgaccaaatgggccagatcgaaaaaatttttaaggtggtgtaccctgtggatgatcatcactttaaggtgatcctgcactatggcacactggtaatcgacggggttacgccgaacatgatcgactatttcggacggccgtatgaaggcatcgccgtgttcgacggcaaaaagatcactgtaacagggaccctgtggaacggcaacaaaattatcgacgagcgcctgatcaaccccgacggctccctgctgttccgagtaaccatcaacggagtgaccggctggcggctgtgcgaacgcattctggcggctgctgctgcgggcattgtggaacaatgctgtaccagcatctgctccctctaccagctggagaactactgcaactaggaattcacgcgtggtacctctagagtcgacccgggcggccgcttcgagcagacatgataagatacattgatgagtttggacaaaccacaactagaatgcagtgaaaaaaatgctttatttgtgaaatttgtgatgctattgctttatttgtaaccattataagctgcaataaacaagttaacaacaacaattgcattcattttatgtttcaggttcagggggagatgtgggaggttttttaaagcaagtaaaacctctacaaatgtggtaaaatcgataaggatccgggctggcgtaatagcgaagaggcccgcaccgatcgcccttcccaacagttgcgcagcctgaatggcgaatggacgcgccctgtagcggcgcattaagcgcggcgggtgtggtggttacgcgcagcgtgaccgctacacttgccagcgccctagcgcccgctcctttcgctttcttcccttcctttctcgccacgttcgccggctttccccgtcaagctctaaatcgggggctccctttagggttccgatttagtgctttacggcacctcgaccccaaaaaacttgattagggtgatggttcacgtagtgggccatcgccctgatagacggtttttcgccctttgacgttggagtccacgttctttaatagtggactcttgttccaaactggaacaacactcaaccctatctcggtctattcttttgatttataagggattttgccgatttcggcctattggttaaaaaatgagctgatttaacaaaaatttaacgcgaattttaacaaaatattaacgcttacaatttcctgatgcggtattttctccttacgcatctgtgcggtatttcacaccgcatatggtgcactctcagtacaatctgctctgatgccgcatagttaagccagccccgacacccgccaacacccgctgacgcgccctgacgggcttgtctgctcccggcatccgcttacagacaagctgtgaccgtctccgggagctgcatgtgtcagaggttttcaccgtcatcaccgaaacgcgcgagacgaaagggcctcgtgatacgcctatttttataggttaatgtcatgataataatggtttcttagacgtcaggtggcacttttcggggaaatgtgcgcggaacccctatttgtttatttttctaaatacattcaaatatgtatccgctcatgagacaataaccctgataaatgcttcaataatattgaaaaaggaagagtatgagtattcaacatttccgtgtcgcccttattcccttttttgcggcattttgccttcctgtttttgctcacccagaaacgctggtgaaagtaaaagatgctgaagatcagttgggtgcacgagtgggttacatcgaactggatctcaacagcggtaagatccttgagagttttcgccccgaagaacgttttccaatgatgagcacttttaaagttctgctatgtggcgcggtattatcccgtattgacgccgggcaagagcaactcggtcgccgcatacactattctcagaatgacttggttgagtactcaccagtcacagaaaagcatcttacggatggcatgacagtaagagaattatgcagtgctgccataaccatgagtgataacactgcggccaacttacttctgacaacgatcggaggaccgaaggagctaaccgcttttttgcacaacatgggggatcatgtaactcgccttgatcgttgggaaccggagctgaatgaagccataccaaacgacgagcgtgacaccacgatgcctgtagcaatggcaacaacgttgcgcaaactattaactggcgaactacttactctagcttcccggcaacaattaatagactggatggaggcggataaagttgcaggaccacttctgcgctcggcccttccggctggctggtttattgctgataaatctggagccggtgagcgtgggtctcgcggtatcattgcagcactggggccagatggtaagccctcccgtatcgtagttatctacacgacggggagtcaggcaactatggatgaacgaaatagacagatcgctgagataggtgcctcactgattaagcattggtaactgtcagaccaagtttactcatatatactttagattgatttaaaacttcatttttaatttaaaaggatctaggtgaagatcctttttgataatctcatgaccaaaatcccttaacgtgagttttcgttccactgagcgtcagaccccgtagaaaagatcaaaggatcttcttgagatcctttttttctgcgcgtaatctgctgcttgcaaacaaaaaaaccaccgctaccagcggtggtttgtttgccggatcaagagctaccaactctttttccgaaggtaactggcttcagcagagcgcagataccaaatactgttcttctagtgtagccgtagttaggccaccacttcaagaactctgtagcaccgcctacatacctcgctctgctaatcctgttaccagtggctgctgccagtggcgataagtcgtgtcttaccgggttggactcaagacgatagttaccggataaggcgcagcggtcgggctgaacggggggttcgtgcacacagcccagcttggagcgaacgacctacaccgaactgagatacctacagcgtgagctatgagaaagcgccacgcttcccgaagggagaaaggcggacaggtatccggtaagcggcagggtcggaacaggagagcgcacgagggagcttccagggggaaacgcctggtatctttatagtcctgtcgggtttcgccacctctgacttgagcgtcgatttttgtgatgctcgtcaggggggcggagcctatggaaaaacgccagcaacgcggcctttttacggttcctggccttttgctggccttttgctcacatggctcgacagatct

SEQ ID NO: 58 - DNA, 4908 bp, synthetic construct
  source 1..4908: mol_type = other DNA; note = pCMVTnT insulin Nluc-Achain del B27-30
tcaatattggccattagccatattattcattggttatatagcataaatcaatattggctattggccattgcatacgttgtatctatatcataatatgtacatttatattggctcatgtccaatatgaccgccatgttggcattgattattgactagttattaatagtaatcaattacggggtcattagttcatagcccatatatggagttccgcgttacataacttacggtaaatggcccgcctggctgaccgcccaacgacccccgcccattgacgtcaataatgacgtatgttcccatagtaacgccaatagggactttccattgacgtcaatgggtggagtatttacggtaaactgcccacttggcagtacatcaagtgtatcatatgccaagtccgccccctattgacgtcaatgacggtaaatggcccgcctggcattatgcccagtacatgaccttacgggactttcctacttggcagtacatctacgtattagtcatcgctattaccatggtgatgcggttttggcagtacaccaatgggcgtggatagcggtttgactcacggggatttccaagtctccaccccattgacgtcaatgggagtttgttttggcaccaaaatcaacgggactttccaaaatgtcgtaataaccccgccccgttgacgcaaatgggcggtaggcgtgtacggtgggaggtctatataagcagagctcgtttagtgaaccgtcagatcactagaagctttattgcggtagtttatcacagttaaattgctaacgcagtcagtgcttctgacacaacagtctcgaacttaagctgcagaagttggtcgtgaggcactgggcaggtaagtatcaaggttacaagacaggtttaaggagaccaatagaaactgggcttgtcgagacagagaagactcttgcgtttctgataggcacctattggtcttactgacatccactttgcctttctctccacaggtgtccactcccagttcaattacagctcttaaggctagagtacttaatacgactcactataggctagcatttaggtgacactatagaatacaagctacttgttctttttgcactcgagaattcatggccctgtggatgcgcctcctgcccctgctggcgctgctggccctctggggacctgacccagccgcagcctttgtgaaccaacacctgtgcggctcacacctggtggaagctctctacctagtgtgcggggaacgaggcttcttctaccgccggaagcgggaggacctgcaggtggggcaggtggagctgggcgggggcccaggccctggtgcaggcagcctgcagcccttggccctggaggggtcccgacgcaagcgtatggtcttcacactcgaagatttcgttggggactggcgacagacagccggctacaacctggaccaagtccttgaacagggaggtgtgtccagtttgtttcagaatctcggggtgtccgtaactccgatccaaaggattgtcctgagcggtgaaaatgggctgaagatcgacatccatgtcatcatcccgtatgaaggtctgagcggcgaccaaatgggccagatcgaaaaaatttttaaggtggtgtaccctgtggatgatcatcactttaaggtgatcctgcactatggcacactggtaatcgacggggttacgccgaacatgatcgactatttcggacggccgtatgaaggcatcgccgtgttcgacggcaaaaagatcactgtaacagggaccctgtggaacggcaacaaaattatcgacgagcgcctgatcaaccccgacggctccctgctgttccgagtaaccatcaacggagtgaccggctggcggctgtgcgaacgcattctggcggctgctgctgcgggcattgtggaacaatgctgtaccagcatctgctccctctaccagctggagaactactgcaactaggaattcacgcgtggtacctctagagtcgacccgggcggccgcttcgagcagacatgataagatacattgatgagtttggacaaaccacaactagaatgcagtgaaaaaaatgctttatttgtgaaatttgtgatgctattgctttatttgtaaccattataagctgcaataaacaagttaacaacaacaattgcattcattttatgtttcaggttcagggggagatgtgggaggttttttaaagcaagtaaaacctctacaaatgtggtaaaatcgataaggatccgggctggcgtaatagcgaagaggcccgcaccgatcgcccttcccaacagttgcgcagcctgaatggcgaatggacgcgccctgtagcggcgcattaagcgcggcgggtgtggtggttacgcgcagcgtgaccgctacacttgccagcgccctagcgcccgctcctttcgctttcttcccttcctttctcgccacgttcgccggctttccccgtcaagctctaaatcgggggctccctttagggttccgatttagtgctttacggcacctcgaccccaaaaaacttgattagggtgatggttcacgtagtgggccatcgccctgatagacggtttttcgccctttgacgttggagtccacgttctttaatagtggactcttgttccaaactggaacaacactcaaccctatctcggtctattcttttgatttataagggattttgccgatttcggcctattggttaaaaaatgagctgatttaacaaaaatttaacgcgaattttaacaaaatattaacgcttacaatttcctgatgcggtattttctccttacgcatctgtgcggtatttcacaccgcatatggtgcactctcagtacaatctgctctgatgccgcatagttaagccagccccgacacccgccaacacccgctgacgcgccctgacgggcttgtctgctcccggcatccgcttacagacaagctgtgaccgtctccgggagctgcatgtgtcagaggttttcaccgtcatcaccgaaacgcgcgagacgaaagggcctcgtgatacgcctatttttataggttaatgtcatgataataatggtttcttagacgtcaggtggcacttttcggggaaatgtgcgcggaacccctatttgtttatttttctaaatacattcaaatatgtatccgctcatgagacaataaccctgataaatgcttcaataatattgaaaaaggaagagtatgagtattcaacatttccgtgtcgcccttattcccttttttgcggcattttgccttcctgtttttgctcacccagaaacgctggtgaaagtaaaagatgctgaagatcagttgggtgcacgagtgggttacatcgaactggatctcaacagcggtaagatccttgagagttttcgccccgaagaacgttttccaatgatgagcacttttaaagttctgctatgtggcgcggtattatcccgtattgacgccgggcaagagcaactcggtcgccgcatacactattctcagaatgacttggttgagtactcaccagtcacagaaaagcatcttacggatggcatgacagtaagagaattatgcagtgctgccataaccatgagtgataacactgcggccaacttacttctgacaacgatcggaggaccgaaggagctaaccgcttttttgcacaacatgggggatcatgtaactcgccttgatcgttgggaaccggagctgaatgaagccataccaaacgacgagcgtgacaccacgatgcctgtagcaatggcaacaacgttgcgcaaactattaactggcgaactacttactctagcttcccggcaacaattaatagactggatggaggcggataaagttgcaggaccacttctgcgctcggcccttccggctggctggtttattgctgataaatctggagccggtgagcgtgggtctcgcggtatcattgcagcactggggccagatggtaagccctcccgtatcgtagttatctacacgacggggagtcaggcaactatggatgaacgaaatagacagatcgctgagataggtgcctcactgattaagcattggtaactgtcagaccaagtttactcatatatactttagattgatttaaaacttcatttttaatttaaaaggatctaggtgaagatcctttttgataatctcatgaccaaaatcccttaacgtgagttttcgttccactgagcgtcagaccccgtagaaaagatcaaaggatcttcttgagatcctttttttctgcgcgtaatctgctgcttgcaaacaaaaaaaccaccgctaccagcggtggtttgtttgccggatcaagagctaccaactctttttccgaaggtaactggcttcagcagagcgcagataccaaatactgttcttctagtgtagccgtagttaggccaccacttcaagaactctgtagcaccgcctacatacctcgctctgctaatcctgttaccagtggctgctgccagtggcgataagtcgtgtcttaccgggttggactcaagacgatagttaccggataaggcgcagcggtcgggctgaacggggggttcgtgcacacagcccagcttggagcgaacgacctacaccgaactgagatacctacagcgtgagctatgagaaagcgccacgcttcccgaagggagaaaggcggacaggtatccggtaagcggcagggtcggaacaggagagcgcacgagggagcttccagggggaaacgcctggtatctttatagtcctgtcgggtttcgccacctctgacttgagcgtcgatttttgtgatgctcgtcaggggggcggagcctatggaaaaacgccagcaacgcggcctttttacggttcctggccttttgctggccttttgctcacatggctcgacagatct

SEQ ID NO: 59 - DNA, 4911 bp, synthetic construct
  source 1..4911: mol_type = other DNA; note = pCMVTnT insulin Nluc-Achain del B28-30
tcaatattggccattagccatattattcattggttatatagcataaatcaatattggctattggccattgcatacgttgtatctatatcataatatgtacatttatattggctcatgtccaatatgaccgccatgttggcattgattattgactagttattaatagtaatcaattacggggtcattagttcatagcccatatatggagttccgcgttacataacttacggtaaatggcccgcctggctgaccgcccaacgacccccgcccattgacgtcaataatgacgtatgttcccatagtaacgccaatagggactttccattgacgtcaatgggtggagtatttacggtaaactgcccacttggcagtacatcaagtgtatcatatgccaagtccgccccctattgacgtcaatgacggtaaatggcccgcctggcattatgcccagtacatgaccttacgggactttcctacttggcagtacatctacgtattagtcatcgctattaccatggtgatgcggttttggcagtacaccaatgggcgtggatagcggtttgactcacggggatttccaagtctccaccccattgacgtcaatgggagtttgttttggcaccaaaatcaacgggactttccaaaatgtcgtaataaccccgccccgttgacgcaaatgggcggtaggcgtgtacggtgggaggtctatataagcagagctcgtttagtgaaccgtcagatcactagaagctttattgcggtagtttatcacagttaaattgctaacgcagtcagtgcttctgacacaacagtctcgaacttaagctgcagaagttggtcgtgaggcactgggcaggtaagtatcaaggttacaagacaggtttaaggagaccaatagaaactgggcttgtcgagacagagaagactcttgcgtttctgataggcacctattggtcttactgacatccactttgcctttctctccacaggtgtccactcccagttcaattacagctcttaaggctagagtacttaatacgactcactataggctagcatttaggtgacactatagaatacaagctacttgttctttttgcactcgagaattcatggccctgtggatgcgcctcctgcccctgctggcgctgctggccctctggggacctgacccagccgcagcctttgtgaaccaacacctgtgcggctcacacctggtggaagctctctacctagtgtgcggggaacgaggcttcttctacacacgccggaagcgggaggacctgcaggtggggcaggtggagctgggcgggggcccaggccctggtgcaggcagcctgcagcccttggccctggaggggtcccgacgcaagcgtatggtcttcacactcgaagatttcgttggggactggcgacagacagccggctacaacctggaccaagtccttgaacagggaggtgtgtccagtttgtttcagaatctcggggtgtccgtaactccgatccaaaggattgtcctgagcggtgaaaatgggctgaagatcgacatccatgtcatcatcccgtatgaaggtctgagcggcgaccaaatgggccagatcgaaaaaatttttaaggtggtgtaccctgtggatgatcatcactttaaggtgatcctgcactatggcacactggtaatcgacggggttacgccgaacatgatcgactatttcggacggccgtatgaaggcatcgccgtgttcgacggcaaaaagatcactgtaacagggaccctgtggaacggcaacaaaattatcgacgagcgcctgatcaaccccgacggctccctgctgttccgagtaaccatcaacggagtgaccggctggcggctgtgcgaacgcattctggcggctgctgctgcgggcattgtggaacaatgctgtaccagcatctgctccctctaccagctggagaactactgcaactaggaattcacgcgtggtacctctagagtcgacccgggcggccgcttcgagcagacatgataagatacattgatgagtttggacaaaccacaactagaatgcagtgaaaaaaatgctttatttgtgaaatttgtgatgctattgctttatttgtaaccattataagctgcaataaacaagttaacaacaacaattgcattcattttatgtttcaggttcagggggagatgtgggaggttttttaaagcaagtaaaacctctacaaatgtggtaaaatcgataaggatccgggctggcgtaatagcgaagaggcccgcaccgatcgcccttcccaacagttgcgcagcctgaatggcgaatggacgcgccctgtagcggcgcattaagcgcggcgggtgtggtggttacgcgcagcgtgaccgctacacttgccagcgccctagcgcccgctcctttcgctttcttcccttcctttctcgccacgttcgccggctttccccgtcaagctctaaatcgggggctccctttagggttccgatttagtgctttacggcacctcgaccccaaaaaacttgattagggtgatggttcacgtagtgggccatcgccctgatagacggtttttcgccctttgacgttggagtccacgttctttaatagtggactcttgttccaaactggaacaacactcaaccctatctcggtctattcttttgatttataagggattttgccgatttcggcctattggttaaaaaatgagctgatttaacaaaaatttaacgcgaattttaacaaaatattaacgcttacaatttcctgatgcggtattttctccttacgcatctgtgcggtatttcacaccgcatatggtgcactctcagtacaatctgctctgatgccgcatagttaagccagccccgacacccgccaacacccgctgacgcgccctgacgggcttgtctgctcccggcatccgcttacagacaagctgtgaccgtctccgggagctgcatgtgtcagaggttttcaccgtcatcaccgaaacgcgcgagacgaaagggcctcgtgatacgcctatttttataggttaatgtcatgataataatggtttcttagacgtcaggtggcacttttcggggaaatgtgcgcggaacccctatttgtttatttttctaaatacattcaaatatgtatccgctcatgagacaataaccctgataaatgcttcaataatattgaaaaaggaagagtatgagtattcaacatttccgtgtcgcccttattcccttttttgcggcattttgccttcctgtttttgctcacccagaaacgctggtgaaagtaaaagatgctgaagatcagttgggtgcacgagtgggttacatcgaactggatctcaacagcggtaagatccttgagagttttcgccccgaagaacgttttccaatgatgagcacttttaaagttctgctatgtggcgcggtattatcccgtattgacgccgggcaagagcaactcggtcgccgcatacactattctcagaatgacttggttgagtactcaccagtcacagaaaagcatcttacggatggcatgacagtaagagaattatgcagtgctgccataaccatgagtgataacactgcggccaacttacttctgacaacgatcggaggaccgaaggagctaaccgcttttttgcacaacatgggggatcatgtaactcgccttgatcgttgggaaccggagctgaatgaagccataccaaacgacgagcgtgacaccacgatgcctgtagcaatggcaacaacgttgcgcaaactattaactggcgaactacttactctagcttcccggcaacaattaatagactggatggaggcggataaagttgcaggaccacttctgcgctcggcccttccggctggctggtttattgctgataaatctggagccggtgagcgtgggtctcgcggtatcattgcagcactggggccagatggtaagccctcccgtatcgtagttatctacacgacggggagtcaggcaactatggatgaacgaaatagacagatcgctgagataggtgcctcactgattaagcattggtaactgtcagaccaagtttactcatatatactttagattgatttaaaacttcatttttaatttaaaaggatctaggtgaagatcctttttgataatctcatgaccaaaatcccttaacgtgagttttcgttccactgagcgtcagaccccgtagaaaagatcaaaggatcttcttgagatcctttttttctgcgcgtaatctgctgcttgcaaacaaaaaaaccaccgctaccagcggtggtttgtttgccggatcaagagctaccaactctttttccgaaggtaactggcttcagcagagcgcagataccaaatactgttcttctagtgtagccgtagttaggccaccacttcaagaactctgtagcaccgcctacatacctcgctctgctaatcctgttaccagtggctgctgccagtggcgataagtcgtgtcttaccgggttggactcaagacgatagttaccggataaggcgcagcggtcgggctgaacggggggttcgtgcacacagcccagcttggagcgaacgacctacaccgaactgagatacctacagcgtgagctatgagaaagcgccacgcttcccgaagggagaaaggcggacaggtatccggtaagcggcagggtcggaacaggagagcgcacgagggagcttccagggggaaacgcctggtatctttatagtcctgtcgggtttcgccacctctgacttgagcgtcgatttttgtgatgctcgtcaggggggcggagcctatggaaaaacgccagcaacgcggcctttttacggttcctggccttttgctggccttttgctcacatggctcgacagatct

SEQ ID NO: 60 - DNA, 4917 bp, synthetic construct
  source 1..4917: mol_type = other DNA; note = pCMVTnT insulin Nluc-Achain del B30
tcaatattggccattagccatattattcattggttatatagcataaatcaatattggctattggccattgcatacgttgtatctatatcataatatgtacatttatattggctcatgtccaatatgaccgccatgttggcattgattattgactagttattaatagtaatcaattacggggtcattagttcatagcccatatatggagttccgcgttacataacttacggtaaatggcccgcctggctgaccgcccaacgacccccgcccattgacgtcaataatgacgtatgttcccatagtaacgccaatagggactttccattgacgtcaatgggtggagtatttacggtaaactgcccacttggcagtacatcaagtgtatcatatgccaagtccgccccctattgacgtcaatgacggtaaatggcccgcctggcattatgcccagtacatgaccttacgggactttcctacttggcagtacatctacgtattagtcatcgctattaccatggtgatgcggttttggcagtacaccaatgggcgtggatagcggtttgactcacggggatttccaagtctccaccccattgacgtcaatgggagtttgttttggcaccaaaatcaacgggactttccaaaatgtcgtaataaccccgccccgttgacgcaaatgggcggtaggcgtgtacggtgggaggtctatataagcagagctcgtttagtgaaccgtcagatcactagaagctttattgcggtagtttatcacagttaaattgctaacgcagtcagtgcttctgacacaacagtctcgaacttaagctgcagaagttggtcgtgaggcactgggcaggtaagtatcaaggttacaagacaggtttaaggagaccaatagaaactgggcttgtcgagacagagaagactcttgcgtttctgataggcacctattggtcttactgacatccactttgcctttctctccacaggtgtccactcccagttcaattacagctcttaaggctagagtacttaatacgactcactataggctagcatttaggtgacactatagaatacaagctacttgttctttttgcactcgagaattcatggccctgtggatgcgcctcctgcccctgctggcgctgctggccctctggggacctgacccagccgcagcctttgtgaaccaacacctgtgcggctcacacctggtggaagctctctacctagtgtgcggggaacgaggcttcttctacacacccaagcgccggaagcgggaggacctgcaggtggggcaggtggagctgggcgggggcccaggccctggtgcaggcagcctgcagcccttggccctggaggggtcccgacgcaagcgtatggtcttcacactcgaagatttcgttggggactggcgacagacagccggctacaacctggaccaagtccttgaacagggaggtgtgtccagtttgtttcagaatctcggggtgtccgtaactccgatccaaaggattgtcctgagcggtgaaaatgggctgaagatcgacatccatgtcatcatcccgtatgaaggtctgagcggcgaccaaatgggccagatcgaaaaaatttttaaggtggtgtaccctgtggatgatcatcactttaaggtgatcctgcactatggcacactggtaatcgacggggttacgccgaacatgatcgactatttcggacggccgtatgaaggcatcgccgtgttcgacggcaaaaagatcactgtaacagggaccctgtggaacggcaacaaaattatcgacgagcgcctgatcaaccccgacggctccctgctgttccgagtaaccatcaacggagtgaccggctggcggctgtgcgaacgcattctggcggctgctgctgcgggcattgtggaacaatgctgtaccagcatctgctccctctaccagctggagaactactgcaactaggaattcacgcgtggtacctctagagtcgacccgggcggccgcttcgagcagacatgataagatacattgatgagtttggacaaaccacaactagaatgcagtgaaaaaaatgctttatttgtgaaatttgtgatgctattgctttatttgtaaccattataagctgcaataaacaagttaacaacaacaattgcattcattttatgtttcaggttcagggggagatgtgggaggttttttaaagcaagtaaaacctctacaaatgtggtaaaatcgataaggatccgggctggcgtaatagcgaagaggcccgcaccgatcgcccttcccaacagttgcgcagcctgaatggcgaatggacgcgccctgtagcggcgcattaagcgcggcgggtgtggtggttacgcgcagcgtgaccgctacacttgccagcgccctagcgcccgctcctttcgctttcttcccttcctttctcgccacgttcgccggctttccccgtcaagctctaaatcgggggctccctttagggttccgatttagtgctttacggcacctcgaccccaaaaaacttgattagggtgatggttcacgtagtgggccatcgccctgatagacggtttttcgccctttgacgttggagtccacgttctttaatagtggactcttgttccaaactggaacaacactcaaccctatctcggtctattcttttgatttataagggattttgccgatttcggcctattggttaaaaaatgagctgatttaacaaaaatttaacgcgaattttaacaaaatattaacgcttacaatttcctgatgcggtattttctccttacgcatctgtgcggtatttcacaccgcatatggtgcactctcagtacaatctgctctgatgccgcatagttaagccagccccgacacccgccaacacccgctgacgcgccctgacgggcttgtctgctcccggcatccgcttacagacaagctgtgaccgtctccgggagctgcatgtgtcagaggttttcaccgtcatcaccgaaacgcgcgagacgaaagggcctcgtgatacgcctatttttataggttaatgtcatgataataatggtttcttagacgtcaggtggcacttttcggggaaatgtgcgcggaacccctatttgtttatttttctaaatacattcaaatatgtatccgctcatgagacaataaccctgataaatgcttcaataatattgaaaaaggaagagtatgagtattcaacatttccgtgtcgcccttattcccttttttgcggcattttgccttcctgtttttgctcacccagaaacgctggtgaaagtaaaagatgctgaagatcagttgggtgcacgagtgggttacatcgaactggatctcaacagcggtaagatccttgagagttttcgccccgaagaacgttttccaatgatgagcacttttaaagttctgctatgtggcgcggtattatcccgtattgacgccgggcaagagcaactcggtcgccgcatacactattctcagaatgacttggttgagtactcaccagtcacagaaaagcatcttacggatggcatgacagtaagagaattatgcagtgctgccataaccatgagtgataacactgcggccaacttacttctgacaacgatcggaggaccgaaggagctaaccgcttttttgcacaacatgggggatcatgtaactcgccttgatcgttgggaaccggagctgaatgaagccataccaaacgacgagcgtgacaccacgatgcctgtagcaatggcaacaacgttgcgcaaactattaactggcgaactacttactctagcttcccggcaacaattaatagactggatggaggcggataaagttgcaggaccacttctgcgctcggcccttccggctggctggtttattgctgataaatctggagccggtgagcgtgggtctcgcggtatcattgcagcactggggccagatggtaagccctcccgtatcgtagttatctacacgacggggagtcaggcaactatggatgaacgaaatagacagatcgctgagataggtgcctcactgattaagcattggtaactgtcagaccaagtttactcatatatactttagattgatttaaaacttcatttttaatttaaaaggatctaggtgaagatcctttttgataatctcatgaccaaaatcccttaacgtgagttttcgttccactgagcgtcagaccccgtagaaaagatcaaaggatcttcttgagatcctttttttctgcgcgtaatctgctgcttgcaaacaaaaaaaccaccgctaccagcggtggtttgtttgccggatcaagagctaccaactctttttccgaaggtaactggcttcagcagagcgcagataccaaatactgttcttctagtgtagccgtagttaggccaccacttcaagaactctgtagcaccgcctacatacctcgctctgctaatcctgttaccagtggctgctgccagtggcgataagtcgtgtcttaccgggttggactcaagacgatagttaccggataaggcgcagcggtcgggctgaacggggggttcgtgcacacagcccagcttggagcgaacgacctacaccgaactgagatacctacagcgtgagctatgagaaagcgccacgcttcccgaagggagaaaggcggacaggtatccggtaagcggcagggtcggaacaggagagcgcacgagggagcttccagggggaaacgcctggtatctttatagtcctgtcgggtttcgccacctctgacttgagcgtcgatttttgtgatgctcgtcaggggggcggagcctatggaaaaacgccagcaacgcggcctttttacggttcctggccttttgctggccttttgctcacatggctcgacagatct

SEQ ID NO: 61 - DNA, 4917 bp, synthetic construct
  source 1..4917: mol_type = other DNA; note = pCMVTnT_hPPI furin-Nlucstop
tcaatattggccattagccatattattcattggttatatagcataaatcaatattggctattggccattgcatacgttgtatctatatcataatatgtacatttatattggctcatgtccaatatgaccgccatgttggcattgattattgactagttattaatagtaatcaattacggggtcattagttcatagcccatatatggagttccgcgttacataacttacggtaaatggcccgcctggctgaccgcccaacgacccccgcccattgacgtcaataatgacgtatgttcccatagtaacgccaatagggactttccattgacgtcaatgggtggagtatttacggtaaactgcccacttggcagtacatcaagtgtatcatatgccaagtccgccccctattgacgtcaatgacggtaaatggcccgcctggcattatgcccagtacatgaccttacgggactttcctacttggcagtacatctacgtattagtcatcgctattaccatggtgatgcggttttggcagtacaccaatgggcgtggatagcggtttgactcacggggatttccaagtctccaccccattgacgtcaatgggagtttgttttggcaccaaaatcaacgggactttccaaaatgtcgtaataaccccgccccgttgacgcaaatgggcggtaggcgtgtacggtgggaggtctatataagcagagctcgtttagtgaaccgtcagatcactagaagctttattgcggtagtttatcacagttaaattgctaacgcagtcagtgcttctgacacaacagtctcgaacttaagctgcagaagttggtcgtgaggcactgggcaggtaagtatcaaggttacaagacaggtttaaggagaccaatagaaactgggcttgtcgagacagagaagactcttgcgtttctgataggcacctattggtcttactgacatccactttgcctttctctccacaggtgtccactcccagttcaattacagctcttaaggctagagtacttaatacgactcactataggctagcatttaggtgacactatagaatacaagctacttgttctttttgcactcgagaattcatggccctgtggatgcgcctcctgcccctgctggcgctgctggccctctggggacctgacccagccgcagcctttgtgaaccaacacctgtgcggctcacacctggtggaagctctctacctagtgtgcggggaacgaggcttcttctacacacccaagacccgccggaagcgggaggacctgcaggtggggcaggtggagctgggcgggggcccaggccctggtgcaggcagcctgcagcccttggccctggaggggtcccgacgcaagcgtggcattgtggaacaatgctgtaccagcatctgctccctctaccagctggagaactactgcaacggtggaggcatggtcttcacactcgaagatttcgttggggactggcgacagacagccggctacaacctggaccaagtccttgaacagggaggtgtgtccagtttgtttcagaatctcggggtgtccgtaactccgatccaaaggattgtcctgagcggtgaaaatgggctgaagatcgacatccatgtcatcatcccgtatgaaggtctgagcggcgaccaaatgggccagatcgaaaaaatttttaaggtggtgtaccctgtggatgatcatcactttaaggtgatcctgcactatggcacactggtaatcgacggggttacgccgaacatgatcgactatttcggacggccgtatgaaggcatcgccgtgttcgacggcaaaaagatcactgtaacagggaccctgtggaacggcaacaaaattatcgacgagcgcctgatcaaccccgacggctccctgctgttccgagtaaccatcaacggagtgaccggctggcggctgtgcgaacgcattctggcgtaggaattcacgcgtggtacctctagagtcgacccgggcggccgcttcgagcagacatgataagatacattgatgagtttggacaaaccacaactagaatgcagtgaaaaaaatgctttatttgtgaaatttgtgatgctattgctttatttgtaaccattataagctgcaataaacaagttaacaacaacaattgcattcattttatgtttcaggttcagggggagatgtgggaggttttttaaagcaagtaaaacctctacaaatgtggtaaaatcgataaggatccgggctggcgtaatagcgaagaggcccgcaccgatcgcccttcccaacagttgcgcagcctgaatggcgaatggacgcgccctgtagcggcgcattaagcgcggcgggtgtggtggttacgcgcagcgtgaccgctacacttgccagcgccctagcgcccgctcctttcgctttcttcccttcctttctcgccacgttcgccggctttccccgtcaagctctaaatcgggggctccctttagggttccgatttagtgctttacggcacctcgaccccaaaaaacttgattagggtgatggttcacgtagtgggccatcgccctgatagacggtttttcgccctttgacgttggagtccacgttctttaatagtggactcttgttccaaactggaacaacactcaaccctatctcggtctattcttttgatttataagggattttgccgatttcggcctattggttaaaaaatgagctgatttaacaaaaatttaacgcgaattttaacaaaatattaacgcttacaatttcctgatgcggtattttctccttacgcatctgtgcggtatttcacaccgcatatggtgcactctcagtacaatctgctctgatgccgcatagttaagccagccccgacacccgccaacacccgctgacgcgccctgacgggcttgtctgctcccggcatccgcttacagacaagctgtgaccgtctccgggagctgcatgtgtcagaggttttcaccgtcatcaccgaaacgcgcgagacgaaagggcctcgtgatacgcctatttttataggttaatgtcatgataataatggtttcttagacgtcaggtggcacttttcggggaaatgtgcgcggaacccctatttgtttatttttctaaatacattcaaatatgtatccgctcatgagacaataaccctgataaatgcttcaataatattgaaaaaggaagagtatgagtattcaacatttccgtgtcgcccttattcccttttttgcggcattttgccttcctgtttttgctcacccagaaacgctggtgaaagtaaaagatgctgaagatcagttgggtgcacgagtgggttacatcgaactggatctcaacagcggtaagatccttgagagttttcgccccgaagaacgttttccaatgatgagcacttttaaagttctgctatgtggcgcggtattatcccgtattgacgccgggcaagagcaactcggtcgccgcatacactattctcagaatgacttggttgagtactcaccagtcacagaaaagcatcttacggatggcatgacagtaagagaattatgcagtgctgccataaccatgagtgataacactgcggccaacttacttctgacaacgatcggaggaccgaaggagctaaccgcttttttgcacaacatgggggatcatgtaactcgccttgatcgttgggaaccggagctgaatgaagccataccaaacgacgagcgtgacaccacgatgcctgtagcaatggcaacaacgttgcgcaaactattaactggcgaactacttactctagcttcccggcaacaattaatagactggatggaggcggataaagttgcaggaccacttctgcgctcggcccttccggctggctggtttattgctgataaatctggagccggtgagcgtgggtctcgcggtatcattgcagcactggggccagatggtaagccctcccgtatcgtagttatctacacgacggggagtcaggcaactatggatgaacgaaatagacagatcgctgagataggtgcctcactgattaagcattggtaactgtcagaccaagtttactcatatatactttagattgatttaaaacttcatttttaatttaaaaggatctaggtgaagatcctttttgataatctcatgaccaaaatcccttaacgtgagttttcgttccactgagcgtcagaccccgtagaaaagatcaaaggatcttcttgagatcctttttttctgcgcgtaatctgctgcttgcaaacaaaaaaaccaccgctaccagcggtggtttgtttgccggatcaagagctaccaactctttttccgaaggtaactggcttcagcagagcgcagataccaaatactgttcttctagtgtagccgtagttaggccaccacttcaagaactctgtagcaccgcctacatacctcgctctgctaatcctgttaccagtggctgctgccagtggcgataagtcgtgtcttaccgggttggactcaagacgatagttaccggataaggcgcagcggtcgggctgaacggggggttcgtgcacacagcccagcttggagcgaacgacctacaccgaactgagatacctacagcgtgagctatgagaaagcgccacgcttcccgaagggagaaaggcggacaggtatccggtaagcggcagggtcggaacaggagagcgcacgagggagcttccagggggaaacgcctggtatctttatagtcctgtcgggtttcgccacctctgacttgagcgtcgatttttgtgatgctcgtcaggggggcggagcctatggaaaaacgccagcaacgcggcctttttacggttcctggccttttgctggccttttgctcacatggctcgacagatct

SEQ ID NO: 62 - DNA, 4920 bp, synthetic construct
  source 1..4920: mol_type = other DNA; note = pCMVTnT_hPreProIns B chain Nluc furin
tcaatattggccattagccatattattcattggttatatagcataaatcaatattggctattggccattgcatacgttgtatctatatcataatatgtacatttatattggctcatgtccaatatgaccgccatgttggcattgattattgactagttattaatagtaatcaattacggggtcattagttcatagcccatatatggagttccgcgttacataacttacggtaaatggcccgcctggctgaccgcccaacgacccccgcccattgacgtcaataatgacgtatgttcccatagtaacgccaatagggactttccattgacgtcaatgggtggagtatttacggtaaactgcccacttggcagtacatcaagtgtatcatatgccaagtccgccccctattgacgtcaatgacggtaaatggcccgcctggcattatgcccagtacatgaccttacgggactttcctacttggcagtacatctacgtattagtcatcgctattaccatggtgatgcggttttggcagtacaccaatgggcgtggatagcggtttgactcacggggatttccaagtctccaccccattgacgtcaatgggagtttgttttggcaccaaaatcaacgggactttccaaaatgtcgtaataaccccgccccgttgacgcaaatgggcggtaggcgtgtacggtgggaggtctatataagcagagctcgtttagtgaaccgtcagatcactagaagctttattgcggtagtttatcacagttaaattgctaacgcagtcagtgcttctgacacaacagtctcgaacttaagctgcagaagttggtcgtgaggcactgggcaggtaagtatcaaggttacaagacaggtttaaggagaccaatagaaactgggcttgtcgagacagagaagactcttgcgtttctgataggcacctattggtcttactgacatccactttgcctttctctccacaggtgtccactcccagttcaattacagctcttaaggctagagtacttaatacgactcactataggctagcatttaggtgacactatagaatacaagctacttgttctttttgcactcgagaattcatggccctgtggatgcgcctcctgcccctgctggcgctgctggccctctggggacctgacccagccgcagcctttgtgaaccaacacctgtgcggctcacacctggtggaagctctctacctagtgtgcggggaacgaggcttcttctacacacccaagaccatggtcttcacactcgaagatttcgttggggactggcgacagacagccggctacaacctggaccaagtccttgaacagggaggtgtgtccagtttgtttcagaatctcggggtgtccgtaactccgatccaaaggattgtcctgagcggtgaaaatgggctgaagatcgacatccatgtcatcatcccgtatgaaggtctgagcggcgaccaaatgggccagatcgaaaaaatttttaaggtggtgtaccctgtggatgatcatcactttaaggtgatcctgcactatggcacactggtaatcgacggggttacgccgaacatgatcgactatttcggacggccgtatgaaggcatcgccgtgttcgacggcaaaaagatcactgtaacagggaccctgtggaacggcaacaaaattatcgacgagcgcctgatcaaccccgacggctccctgctgttccgagtaaccatcaacggagtgaccggctggcggctgtgcgaacgcattctggcggctgctgctgcgcgccggaagcgggaggacctgcaggtggggcaggtggagctgggcgggggcccaggccctggtgcaggcagcctgcagcccttggccctggaggggtcccgacgcaagcgtggcattgtggaacaatgctgtaccagcatctgctccctctaccagctggagaactactgcaactaggaattcacgcgtggtacctctagagtcgacccgggcggccgcttcgagcagacatgataagatacattgatgagtttggacaaaccacaactagaatgcagtgaaaaaaatgctttatttgtgaaatttgtgatgctattgctttatttgtaaccattataagctgcaataaacaagttaacaacaacaattgcattcattttatgtttcaggttcagggggagatgtgggaggttttttaaagcaagtaaaacctctacaaatgtggtaaaatcgataaggatccgggctggcgtaatagcgaagaggcccgcaccgatcgcccttcccaacagttgcgcagcctgaatggcgaatggacgcgccctgtagcggcgcattaagcgcggcgggtgtggtggttacgcgcagcgtgaccgctacacttgccagcgccctagcgcccgctcctttcgctttcttcccttcctttctcgccacgttcgccggctttccccgtcaagctctaaatcgggggctccctttagggttccgatttagtgctttacggcacctcgaccccaaaaaacttgattagggtgatggttcacgtagtgggccatcgccctgatagacggtttttcgccctttgacgttggagtccacgttctttaatagtggactcttgttccaaactggaacaacactcaaccctatctcggtctattcttttgatttataagggattttgccgatttcggcctattggttaaaaaatgagctgatttaacaaaaatttaacgcgaattttaacaaaatattaacgcttacaatttcctgatgcggtattttctccttacgcatctgtgcggtatttcacaccgcatatggtgcactctcagtacaatctgctctgatgccgcatagttaagccagccccgacacccgccaacacccgctgacgcgccctgacgggcttgtctgctcccggcatccgcttacagacaagctgtgaccgtctccgggagctgcatgtgtcagaggttttcaccgtcatcaccgaaacgcgcgagacgaaagggcctcgtgatacgcctatttttataggttaatgtcatgataataatggtttcttagacgtcaggtggcacttttcggggaaatgtgcgcggaacccctatttgtttatttttctaaatacattcaaatatgtatccgctcatgagacaataaccctgataaatgcttcaataatattgaaaaaggaagagtatgagtattcaacatttccgtgtcgcccttattcccttttttgcggcattttgccttcctgtttttgctcacccagaaacgctggtgaaagtaaaagatgctgaagatcagttgggtgcacgagtgggttacatcgaactggatctcaacagcggtaagatccttgagagttttcgccccgaagaacgttttccaatgatgagcacttttaaagttctgctatgtggcgcggtattatcccgtattgacgccgggcaagagcaactcggtcgccgcatacactattctcagaatgacttggttgagtactcaccagtcacagaaaagcatcttacggatggcatgacagtaagagaattatgcagtgctgccataaccatgagtgataacactgcggccaacttacttctgacaacgatcggaggaccgaaggagctaaccgcttttttgcacaacatgggggatcatgtaactcgccttgatcgttgggaaccggagctgaatgaagccataccaaacgacgagcgtgacaccacgatgcctgtagcaatggcaacaacgttgcgcaaactattaactggcgaactacttactctagcttcccggcaacaattaatagactggatggaggcggataaagttgcaggaccacttctgcgctcggcccttccggctggctggtttattgctgataaatctggagccggtgagcgtgggtctcgcggtatcattgcagcactggggccagatggtaagccctcccgtatcgtagttatctacacgacggggagtcaggcaactatggatgaacgaaatagacagatcgctgagataggtgcctcactgattaagcattggtaactgtcagaccaagtttactcatatatactttagattgatttaaaacttcatttttaatttaaaaggatctaggtgaagatcctttttgataatctcatgaccaaaatcccttaacgtgagttttcgttccactgagcgtcagaccccgtagaaaagatcaaaggatcttcttgagatcctttttttctgcgcgtaatctgctgcttgcaaacaaaaaaaccaccgctaccagcggtggtttgtttgccggatcaagagctaccaactctttttccgaaggtaactggcttcagcagagcgcagataccaaatactgttcttctagtgtagccgtagttaggccaccacttcaagaactctgtagcaccgcctacatacctcgctctgctaatcctgttaccagtggctgctgccagtggcgataagtcgtgtcttaccgggttggactcaagacgatagttaccggataaggcgcagcggtcgggctgaacggggggttcgtgcacacagcccagcttggagcgaacgacctacaccgaactgagatacctacagcgtgagctatgagaaagcgccacgcttcccgaagggagaaaggcggacaggtatccggtaagcggcagggtcggaacaggagagcgcacgagggagcttccagggggaaacgcctggtatctttatagtcctgtcgggtttcgccacctctgacttgagcgtcgatttttgtgatgctcgtcaggggggcggagcctatggaaaaacgccagcaacgcggcctttttacggttcctggccttttgctggccttttgctcacatggctcgacagatct

SEQ ID NO: 63 - DNA, 4920 bp, synthetic construct; identical to SEQ ID NO: 55
  source 1..4920: mol_type = other DNA

SEQ ID NO: 64 - DNA, 4934 bp, synthetic construct
  source 1..4934: mol_type = other DNA; note = pCMVTnT_sNluc_hPPI_furin_c-peptide
tcaatattggccattagccatattattcattggttatatagcataaatcaatattggctattggccattgcatacgttgtatctatatcataatatgtacatttatattggctcatgtccaatatgaccgccatgttggcattgattattgactagttattaatagtaatcaattacggggtcattagttcatagcccatatatggagttccgcgttacataacttacggtaaatggcccgcctggctgaccgcccaacgacccccgcccattgacgtcaataatgacgtatgttcccatagtaacgccaatagggactttccattgacgtcaatgggtggagtatttacggtaaactgcccacttggcagtacatcaagtgtatcatatgccaagtccgccccctattgacgtcaatgacggtaaatggcccgcctggcattatgcccagtacatgaccttacgggactttcctacttggcagtacatctacgtattagtcatcgctattaccatggtgatgcggttttggcagtacaccaatgggcgtggatagcggtttgactcacggggatttccaagtctccaccccattgacgtcaatgggagtttgttttggcaccaaaatcaacgggactttccaaaatgtcgtaataaccccgccccgttgacgcaaatgggcggtaggcgtgtacggtgggaggtctatataagcagagctcgtttagtgaaccgtcagatcactagaagctttattgcggtagtttatcacagttaaattgctaacgcagtcagtgcttctgacacaacagtctcgaacttaagctgcagaagttggtcgtgaggcactgggcaggtaagtatcaaggttacaagacaggtttaaggagaccaatagaaactgggcttgtcgagacagagaagactcttgcgtttctgataggcacctattggtcttactgacatccactttgcctttctctccacaggtgtccactcccagttcaattacagctcttaaggctagagtacttaatacgactcactataggctagcatttaggtgacactatagaatacaagctacttgttctttttgcactcgaggaattcgccgccaccatgaactccttctccacaagcgccttcggtccagttgccttctccctgggcctgctcctggtgttgcctgctgccttccctgccccagtcttcacactcgaagatttcgttggggactggcgacagacagccggctacaacctggaccaagtccttgaacagggaggtgtgtccagtttgtttcagaatctcggggtgtccgtaactccgatccaaaggattgtcctgagcggtgaaaatgggctgaagatcgacatccatgtcatcatcccgtatgaaggtctgagcggcgaccaaatgggccagatcgaaaaaatttttaaggtggtgtaccctgtggatgatcatcactttaaggtgatcctgcactatggcacactggtaatcgacggggttacgccgaacatgatcgactatttcggacggccgtatgaaggcatcgccgtgttcgacggcaaaaagatcactgtaacagggaccctgtggaacggcaacaaaattatcgacgagcgcctgatcaaccccgacggctccctgctgttccgagtaaccatcaacggagtgaccggctggcggctgtgcgaacgcattctggcgggtggaggctttgtgaaccaacacctgtgcggctcacacctggtggaagctctctacctagtgtgcggggaacgaggcttcttctacacacccaagacccgccggaagcgggaggacctgcaggtggggcaggtggagctgggcgggggcccaggccctggtgcaggcagcctgcagcccttggccctggaggggtcccgacgcaagcgtggcattgtggaacaatgctgtaccagcatctgctccctctaccagctggagaactactgcaactaggaattccggtacctctagagtcgacccgggcggccgcttcgagcagacatgataagatacattgatgagtttggacaaaccacaactagaatgcagtgaaaaaaatgctttatttgtgaaatttgtgatgctattgctttatttgtaaccattataagctgcaataaacaagttaacaacaacaattgcattcattttatgtttcaggttcagggggagatgtgggaggttttttaaagcaagtaaaacctctacaaatgtggtaaaatcgataaggatccgggctggcgtaatagcgaagaggcccgcaccgatcgcccttcccaacagttgcgcagcctgaatggcgaatggacgcgccctgtagcggcgcattaagcgcggcgggtgtggtggttacgcgcagcgtgaccgctacacttgccagcgccctagcgcccgctcctttcgctttcttcccttcctttctcgccacgttcgccggctttccccgtcaagctctaaatcgggggctccctttagggttccgatttagtgctttacggcacctcgaccccaaaaaacttgattagggtgatggttcacgtagtgggccatcgccctgatagacggtttttcgccctttgacgttggagtccacgttctttaatagtggactcttgttccaaactggaacaacactcaaccctatctcggtctattcttttgatttataagggattttgccgatttcggcctattggttaaaaaatgagctgatttaacaaaaatttaacgcgaattttaacaaaatattaacgcttacaatttcctgatgcggtattttctccttacgcatctgtgcggtatttcacaccgcatatggtgcactctcagtacaatctgctctgatgccgcatagttaagccagccccgacacccgccaacacccgctgacgcgccctgacgggcttgtctgctcccggcatccgcttacagacaagctgtgaccgtctccgggagctgcatgtgtcagaggttttcaccgtcatcaccgaaacgcgcgagacgaaagggcctcgtgatacgcctatttttataggttaatgtcatgataataatggtttcttagacgtcaggtggcacttttcggggaaatgtgcgcggaacccctatttgtttatttttctaaatacattcaaatatgtatccgctcatgagacaataaccctgataaatgcttcaataatattgaaaaaggaagagtatgagtattcaacatttccgtgtcgcccttattcccttttttgcggcattttgccttcctgtttttgctcacccagaaacgctggtgaaagtaaaagatgctgaagatcagttgggtgcacgagtgggttacatcgaactggatctcaacagcggtaagatccttgagagttttcgccccgaagaacgttttccaatgatgagcacttttaaagttctgctatgtggcgcggtattatcccgtattgacgccgggcaagagcaactcggtcgccgcatacactattctcagaatgacttggttgagtactcaccagtcacagaaaagcatcttacggatggcatgacagtaagagaattatgcagtgctgccataaccatgagtgataacactgcggccaacttacttctgacaacgatcggaggaccgaaggagctaaccgcttttttgcacaacatgggggatcatgtaactcgccttgatcgttgggaaccggagctgaatgaagccataccaaacgacgagcgtgacaccacgatgcctgtagcaatggcaacaacgttgcgcaaactattaactggcgaactacttactctagcttcccggcaacaattaatagactggatggaggcggataaagttgcaggaccacttctgcgctcggcccttccggctggctggtttattgctgataaatctggagccggtgagcgtgggtctcgcggtatcattgcagcactggggccagatggtaagccctcccgtatcgtagttatctacacgacggggagtcaggcaactatggatgaacgaaatagacagatcgctgagataggtgcctcactgattaagcattggtaactgtcagaccaagtttactcatatatactttagattgatttaaaacttcatttttaatttaaaaggatctaggtgaagatcctttttgataatctcatgaccaaaatcccttaacgtgagttttcgttccactgagcgtcagaccccgtagaaaagatcaaaggatcttcttgagatcctttttttctgcgcgtaatctgctgcttgcaaacaaaaaaaccaccgctaccagcggtggtttgtttgccggatcaagagctaccaactctttttccgaaggtaactggcttcagcagagcgcagataccaaatactgttcttctagtgtagccgtagttaggccaccacttcaagaactctgtagcaccgcctacatacctcgctctgctaatcctgttaccagtggctgctgccagtggcgataagtcgtgtcttaccgggttggactcaagacgatagttaccggataaggcgcagcggtcgggctgaacggggggttcgtgcacacagcccagcttggagcgaacgacctacaccgaactgagatacctacagcgtgagctatgagaaagcgccacgcttcccgaagggagaaaggcggacaggtatccggtaagcggcagggtcggaacaggagagcgcacgagggagcttccagggggaaacgcctggtatctttatagtcctgtcgggtttcgccacctctgacttgagcgtcgatttttgtgatgctcgtcaggggggcggagcctatggaaaaacgccagcaacgcggcctttttacggttcctggccttttgctggccttttgctcacatggctcgacagatct

SEQ ID NO: 65 - DNA, 837 bp, synthetic construct
  source 1..837: mol_type = other DNA; note = Proinsulin B NLuc Delta B24-30
atggccctgtggatgcgcctcctgcccctgctggcgctgctggccctctggggacctgacccagccgcagcctttgtgaaccaacacctgtgcggctcacacctggtggaagctctctacctagtgtgcggggaacgaggcatggtcttcacactcgaagatttcgttggggactggcgacagacagccggctacaacctggaccaagtccttgaacagggaggtgtgtccagtttgtttcagaatctcggggtgtccgtaactccgatccaaaggattgtcctgagcggtgaaaatgggctgaagatcgacatccatgtcatcatcccgtatgaaggtctgagcggcgaccaaatgggccagatcgaaaaaatttttaaggtggtgtaccctgtggatgatcatcactttaaggtgatcctgcactatggcacactggtaatcgacggggttacgccgaacatgatcgactatttcggacggccgtatgaaggcatcgccgtgttcgacggcaaaaagatcactgtaacagggaccctgtggaacggcaacaaaattatcgacgagcgcctgatcaaccccgacggctccctgctgttccgagtaaccatcaacggagtgaccggctggcggctgtgcgaacgcattctggcggctgctgctgcgcgccgggaggcagaggacctgcaggtggggcaggtggagctgggcgggggcccaggcgcaggcagcctgcagcccttggccctggaggggtccctgcagaagcgtggcattgtggaacaatgctgtaccagcatctgctccctctaccagctggagaactactgcaactag

SEQ ID NO: 66 - DNA, 840 bp, synthetic construct
  source 1..840: mol_type = other DNA; note = Proinsulin B NLuc Delta B25-30
atggccctgtggatgcgcctcctgcccctgctggcgctgctggccctctggggacctgacccagccgcagcctttgtgaaccaacacctgtgcggctcacacctggtggaagctctctacctagtgtgcggggaacgaggcttcatggtcttcacactcgaagatttcgttggggactggcgacagacagccggctacaacctggaccaagtccttgaacagggaggtgtgtccagtttgtttcagaatctcggggtgtccgtaactccgatccaaaggattgtcctgagcggtgaaaatgggctgaagatcgacatccatgtcatcatcccgtatgaaggtctgagcggcgaccaaatgggccagatcgaaaaaatttttaaggtggtgtaccctgtggatgatcatcactttaaggtgatcctgcactatggcacactggtaatcgacggggttacgccgaacatgatcgactatttcggacggccgtatgaaggcatcgccgtgttcgacggcaaaaagatcactgtaacagggaccctgtggaacggcaacaaaattatcgacgagcgcctgatcaaccccgacggctccctgctgttccgagtaaccatcaacggagtgaccggctggcggctgtgcgaacgcattctggcggctgctgctgcgcgccgggaggcagaggacctgcaggtggggcaggtggagctgggcgggggcccaggcgcaggcagcctgcagcccttggccctggaggggtccctgcagaagcgtggcattgtggaacaatgctgtaccagcatctgctccctctaccagctggagaactactgcaactag

SEQ ID NO: 67 - DNA, 843 bp, synthetic construct
  source 1..843: mol_type = other DNA; note = Proinsulin B NLuc Delta B26-30
atggccctgtggatgcgcctcctgcccctgctggcgctgctggccctctggggacctgacccagccgcagcctttgtgaaccaacacctgtgcggctcacacctggtggaagctctctacctagtgtgcggggaacgaggcttcttcatggtcttcacactcgaagatttcgttggggactggcgacagacagccggctacaacctggaccaagtccttgaacagggaggtgtgtccagtttgtttcagaatctcggggtgtccgtaactccgatccaaaggattgtcctgagcggtgaaaatgggctgaagatcgacatccatgtcatcatcccgtatgaaggtctgagcggcgaccaaatgggccagatcgaaaaaatttttaaggtggtgtaccctgtggatgatcatcactttaaggtgatcctgcactatggcacactggtaatcgacggggttacgccgaacatgatcgactatttcggacggccgtatgaaggcatcgccgtgttcgacggcaaaaagatcactgtaacagggaccctgtggaacggcaacaaaattatcgacgagcgcctgatcaaccccgacggctccctgctgttccgagtaaccatcaacggagtgaccggctggcggctgtgcgaacgcattctggcggctgctgctgcgcgccgggaggcagaggacctgcaggtggggcaggtggagctgggcgggggcccaggcgcaggcagcctgcagcccttggccctggaggggtccctgcagaagcgtggcattgtggaacaatgctgtaccagcatctgctccctctaccagctggagaactactgcaactag

SEQ ID NO: 68 - DNA, 846 bp, synthetic construct
  source 1..846: mol_type = other DNA; note = Proinsulin B NLuc Delta B27-30
atggccctgtggatgcgcctcctgcccctgctggcgctgctggccctctggggacctgacccagccgcagcctttgtgaaccaacacctgtgcggctcacacctggtggaagctctctacctagtgtgcggggaacgaggcttcttctacatggtcttcacactcgaagatttcgttggggactggcgacagacagccggctacaacctggaccaagtccttgaacagggaggtgtgtccagtttgtttcagaatctcggggtgtccgtaactccgatccaaaggattgtcctgagcggtgaaaatgggctgaagatcgacatccatgtcatcatcccgtatgaaggtctgagcggcgaccaaatgggccagatcgaaaaaatttttaaggtggtgtaccctgtggatgatcatcactttaaggtgatcctgcactatggcacactggtaatcgacggggttacgccgaacatgatcgactatttcggacggccgtatgaaggcatcgccgtgttcgacggcaaaaagatcactgtaacagggaccctgtggaacggcaacaaaattatcgacgagcgcctgatcaaccccgacggctccctgctgttccgagtaaccatcaacggagtgaccggctggcggctgtgcgaacgcattctggcggctgctgctgcgcgccgggaggcagaggacctgcaggtggggcaggtggagctgggcgggggcccaggcgcaggcagcctgcagcccttggccctggaggggtccctgcagaagcgtggcattgtggaacaatgctgtaccagcatctgctccctctaccagctggagaactactgcaactag

SEQ ID NO: 69 - DNA, 849 bp, synthetic construct
  source 1..849: mol_type = other DNA; note = Proinsulin B NLuc Delta B28-30
atggccctgtggatgcgcctcctgcccctgctggcgctgctggccctctggggacctgacccagccgcagcctttgtgaaccaacacctgtgcggctcacacctggtggaagctctctacctagtgtgcggggaacgaggcttcttctacacaatggtcttcacactcgaagatttcgttggggactggcgacagacagccggctacaacctggaccaagtccttgaacagggaggtgtgtccagtttgtttcagaatctcggggtgtccgtaactccgatccaaaggattgtcctgagcggtgaaaatgggctgaagatcgacatccatgtcatcatcccgtatgaaggtctgagcggcgaccaaatgggccagatcgaaaaaatttttaaggtggtgtaccctgtggatgatcatcactttaaggtgatcctgcactatggcacactggtaatcgacggggttacgccgaacatgatcgactatttcggacggccgtatgaaggcatcgccgtgttcgacggcaaaaagatcactgtaacagggaccctgtggaacggcaacaaaattatcgacgagcgcctgatcaaccccgacggctccctgctgttccgagtaaccatcaacggagtgaccggctggcggctgtgcgaacgcattctggcggctgctgctgcgcgccgggaggcagaggacctgcaggtggggcaggtggagctgggcgggggcccaggcgcaggcagcctgcagcccttggccctggaggggtccctgcagaagcgtggcattgtggaacaatgctgtaccagcatctgctccctctaccagctggagaactactgcaactag

SEQ ID NO: 70 - DNA, 858 bp, synthetic construct
  source 1..858: mol_type = other DNA; note = Proinsulin B NLuc mut A L13A
atggccctgtggatgcgcctcctgcccctgctggcgctgctggccctctggggacctgacccagccgcagcctttgtgaaccaacacctgtgcggctcacacctggtggaagctctctacctagtgtgcggggaacgaggcttcttctacacacccaagaccatggtcttcacactcgaagatttcgttggggactggcgacagacagccggctacaacctggaccaagtccttgaacagggaggtgtgtccagtttgtttcagaatctcggggtgtccgtaactccgatccaaaggattgtcctgagcggtgaaaatgggctgaagatcgacatccatgtcatcatcccgtatgaaggtctgagcggcgaccaaatgggccagatcgaaaaaatttttaaggtggtgtaccctgtggatgatcatcactttaaggtgatcctgcactatggcacactggtaatcgacggggttacgccgaacatgatcgactatttcggacggccgtatgaaggcatcgccgtgttcgacggcaaaaagatcactgtaacagggaccctgtggaacggcaacaaaattatcgacgagcgcctgatcaaccccgacggctccctgctgttccgagtaaccatcaacggagtgaccggctggcggctgtgcgaacgcattctggcggctgctgctgcgcgccgggaggcagaggacctgcaggtggggcaggtggagctgggcgggggcccaggcgcaggcagcctgcagcccttggccctggaggggtccctgcagaagcgtggcattgtggaacaatgctgtaccagcatctgctccgcctaccagctggagaactactgcaactag

SEQ ID NO: 71 - DNA, 858 bp, synthetic construct
  source 1..858: mol_type = other DNA; note = Proinsulin B NLuc mut A L13W
atggccctgtggatgcgcctcctgcccctgctggcgctgctggccctctggggacctgacccagccgcagcctttgtgaaccaacacctgtgcggctcacacctggtggaagctctctacctagtgtgcggggaacgaggcttcttctacacacccaagaccatggtcttcacactcgaagatttcgttggggactggcgacagacagccggctacaacctggaccaagtccttgaacagggaggtgtgtccagtttgtttcagaatctcggggtgtccgtaactccgatccaaaggattgtcctgagcggtgaaaatgggctgaagatcgacatccatgtcatcatcccgtatgaaggtctgagcggcgaccaaatgggccagatcgaaaaaatttttaaggtggtgtaccctgtggatgatcatcactttaaggtgatcctgcactatggcacactggtaatcgacggggttacgccgaacatgatcgactatttcggacggccgtatgaaggcatcgccgtgttcgacggcaaaaagatcactgtaacagggaccctgtggaacggcaacaaaattatcgacgagcgcctgatcaaccccgacggctccctgctgttccgagtaaccatcaacggagtgaccggctggcggctgtgcgaacgcattctggcggctgctgctgcgcgccgggaggcagaggacctgcaggtggggcaggtggagctgggcgggggcccaggcgcaggcagcctgcagcccttggccctggaggggtccctgcagaagcgtggcattgtggaacaatgctgtaccagcatctgctcctggtaccagctggagaactactgcaactag

SEQ ID NO: 72 - DNA, 858 bp, synthetic construct
  source 1..858: mol_type = other DNA; note = Proinsulin B NLuc mut A Y14A
atggccctgtggatgcgcctcctgcccctgctggcgctgctggccctctggggacctgacccagccgcagcctttgtgaaccaacacctgtgcggctcacacctggtggaagctctctacctagtgtgcggggaacgaggcttcttctacacacccaagaccatggtcttcacactcgaagatttcgttggggactggcgacagacagccggctacaacctggaccaagtccttgaacagggaggtgtgtccagtttgtttcagaatctcggggtgtccgtaactccgatccaaaggattgtcctgagcggtgaaaatgggctgaagatcgacatccatgtcatcatcccgtatgaaggtctgagcggcgaccaaatgggccagatcgaaaaaatttttaaggtggtgtaccctgtggatgatcatcactttaaggtgatcctgcactatggcacactggtaatcgacggggttacgccgaacatgatcgactatttcggacggccgtatgaaggcatcgccgtgttcgacggcaaaaagatcactgtaacagggaccctgtggaacggcaacaaaattatcgacgagcgcctgatcaaccccgacggctccctgctgttccgagtaaccatcaacggagtgaccggctggcggctgtgcgaacgcattctggcggctgctgctgcgcgccgggaggcagaggacctgcaggtggggcaggtggagctgggcgggggcccaggcgcaggcagcctgcagcccttggccctggaggggtccctgcagaagcgtggcattgtggaacaatgctgtaccagcatctgctccctcgcccagctggagaactactgcaactag

SEQ ID NO: 73 - DNA, 858 bp, synthetic construct
  source 1..858: mol_type = other DNA; note = Proinsulin B NLuc mut B F1A
atggccctgtggatgcgcctcctgcccctgctggcgctgctggccctctggggacctgacccagccgcagccgctgtgaaccaacacctgtgcggctcacacctggtggaagctctctacctagtgtgcggggaacgaggcttcttctacacacccaagaccatggtcttcacactcgaagatttcgttggggactggcgacagacagccggctacaacctggaccaagtccttgaacagggaggtgtgtccagtttgtttcagaatctcggggtgtccgtaactccgatccaaaggattgtcctgagcggtgaaaatgggctgaagatcgacatccatgtcatcatcccgtatgaaggtctgagcggcgaccaaatgggccagatcgaaaaaatttttaaggtggtgtaccctgtggatgatcatcactttaaggtgatcctgcactatggcacactggtaatcgacggggttacgccgaacatgatcgactatttcggacggccgtatgaaggcatcgccgtgttcgacggcaaaaagatcactgtaacagggaccctgtggaacggcaacaaaattatcgacgagcgcctgatcaaccccgacggctccctgctgttccgagtaaccatcaacggagtgaccggctggcggctgtgcgaacgcattctggcggctgctgctgcgcgccgggaggcagaggacctgcaggtggggcaggtggagctgggcgggggcccaggcgcaggcagcctgcagcccttggccctggaggggtccctgcagaagcgtggcattgtggaacaatgctgtaccagcatctgctccctctaccagctggagaactactgcaactag

SEQ ID NO: 74 - DNA, 858 bp, synthetic construct
  source 1..858: mol_type = other DNA; note = Proinsulin B NLuc mut B L17A
atggccctgtggatgcgcctcctgcccctgctggcgctgctggccctctggggacctgacccagccgcagcctttgtgaaccaacacctgtgcggctcacacctggtggaagctctctacgcagtgtgcggggaacgaggcttcttctacacacccaagaccatggtcttcacactcgaagatttcgttggggactggcgacagacagccggctacaacctggaccaagtccttgaacagggaggtgtgtccagtttgtttcagaatctcggggtgtccgtaactccgatccaaaggattgtcctgagcggtgaaaatgggctgaagatcgacatccatgtcatcatcccgtatgaaggtctgagcggcgaccaaatgggccagatcgaaaaaatttttaaggtggtgtaccctgtggatgatcatcactttaaggtgatcctgcactatggcacactggtaatcgacggggttacgccgaacatgatcgactatttcggacggccgtatgaaggcatcgccgtgttcgacggcaaaaagatcactgtaacagggaccctgtggaacggcaacaaaattatcgacgagcgcctgatcaaccccgacggctccctgctgttccgagtaaccatcaacggagtgaccggctggcggctgtgcgaacgcattctggcggctgctgctgcgcgccgggaggcagaggacctgcaggtggggcaggtggagctgggcgggggcccaggcgcaggcagcctgcagcccttggccctggaggggtccctgcagaagcgtggcattgtggaacaatgctgtaccagcatctgctccctctaccagctggagaactactgcaactag

SEQ ID NO: 75 - DNA, 861 bp, synthetic construct
  source 1..861: mol_type = other DNA; note = Proinsulin A NLuc
atggccctgtggatgcgcttgttgccccttctggcccttctcgcactgtggggacctgatccagctgcggcctttgtgaaccagcacctgtgtgggtcccatctggtggaagccctgtatctcgtctgtggagaacgcggcttcttctacacaccgaagacccgccgggaggcagaggacctgcaggtggggcaggtggagctgggcgggggcccaggcgcaggcagcctgcagcccttggccctggaggggtccctgcagaagcgtggcattgtggagcagtgctgcaccagcatctgctccctctaccagctggagaactactgcaacgaattcggtggaggcatggtcttcacactcgaagatttcgttggggactggcgacagacagccggctacaacctggaccaagtccttgaacagggaggtgtgtccagtttgtttcagaatctcggggtgtccgtaactccgatccaaaggattgtcctgagcggtgaaaatgggctgaagatcgacatccatgtcatcatcccgtatgaaggtctgagcggcgaccaaatgggccagatcgaaaaaatttttaaggtggtgtaccctgtggatgatcatcactttaaggtgatcctgcactatggcacactggtaatcgacggggttacgccgaacatgatcgactatttcggacggccgtatgaaggcatcgccgtgttcgacggcaaaaagatcactgtaacagggaccctgtggaacggcaacaaaattatcgacgagcgcctgatcaaccccgacggctccctgctgttccgagtaaccatcaacggagtgaccggctggcggctgtgcgaacgcattctggcgtaa

SEQ ID NO: 76 - DNA, 858 bp, synthetic construct
  source 1..858: mol_type = other DNA; note = Proinsulin B NLuc no PG duplication
atggccctgtggatgcgcctcctgcccctgctggcgctgctggccctctggggacctgacccagccgcagcctttgtgaaccaacacctgtgcggctcacacctggtggaagctctctacctagtgtgcggggaacgaggcttcttctacacacccaagaccatggtcttcacactcgaagatttcgttggggactggcgacagacagccggctacaacctggaccaagtccttgaacagggaggtgtgtccagtttgtttcagaatctcggggtgtccgtaactccgatccaaaggattgtcctgagcggtgaaaatgggctgaagatcgacatccatgtcatcatcccgtatgaaggtctgagcggcgaccaaatgggccagatcgaaaaaatttttaaggtggtgtaccctgtggatgatcatcactttaaggtgatcctgcactatggcacactggtaatcgacggggttacgccgaacatgatcgactatttcggacggccgtatgaaggcatcgccgtgttcgacggcaaaaagatcactgtaacagggaccctgtggaacggcaacaaaattatcgacgagcgcctgatcaaccccgacggctccctgctgttccgagtaaccatcaacggagtgaccggctggcggctgtgcgaacgcattctggcggctgctgctgcgcgccgggaggcagaggacctgcaggtggggcaggtggagctgggcgggggcccaggcgcaggcagcctgcagcccttggccctggaggggtccctgcagaagcgtggcattgtggaacaatgctgtaccagcatctgctccctctaccagctggagaactactgcaactag

SEQ ID NO: 77 - DNA, 864 bp, synthetic construct
  source 1..864: mol_type = other DNA; note = Proinsulin B NLuc
atggccctgtggatgcgcctcctgcccctgctggcgctgctggccctctggggacctgacccagccgcagcctttgtgaaccaacacctgtgcggctcacacctggtggaagctctctacctagtgtgcggggaacgaggcttcttctacacacccaagaccatggtcttcacactcgaagatttcgttggggactggcgacagacagccggctacaacctggaccaagtccttgaacagggaggtgtgtccagtttgtttcagaatctcggggtgtccgtaactccgatccaaaggattgtcctgagcggtgaaaatgggctgaagatcgacatccatgtcatcatcccgtatgaaggtctgagcggcgaccaaatgggccagatcgaaaaaatttttaaggtggtgtaccctgtggatgatcatcactttaaggtgatcctgcactatggcacactggtaatcgacggggttacgccgaacatgatcgactatttcggacggccgtatgaaggcatcgccgtgttcgacggcaaaaagatcactgtaacagggaccctgtggaacggcaacaaaattatcgacgagcgcctgatcaaccccgacggctccctgctgttccgagtaaccatcaacggagtgaccggctggcggctgtgcgaacgcattctggcggctgctgctgcgcgccgggaggcagaggacctgcaggtggggcaggtggagctgggcgggggcccaggccctggtgcaggcagcctgcagcccttggccctggaggggtccctgcagaagcgtggcattgtggaacaatgctgtaccagcatctgctccctctaccagctggagaactactgcaactag

SEQ ID NO: 78 - DNA, 864 bp, synthetic construct
  source 1..864: mol_type = other DNA; note = Proinsulin C pep NLuc C pep
atggccctgtggatgcgcctcctgcccctgctggcgctgctggccctctggggacctgacccagccgcagcctttgtgaaccaacacctgtgcggctcacacctggtggaagctctctacctagtgtgcggggaacgaggcttcttctacacacccaagacccgccgggaggcagaggacctgcaggtggggcaggtggagctgggcgggggcccaatggtcttcacactcgaagatttcgttggggactggcgacagacagccggctacaacctggaccaagtccttgaacagggaggtgtgtccagtttgtttcagaatctcggggtgtccgtaactccgatccaaaggattgtcctgagcggtgaaaatgggctgaagatcgacatccatgtcatcatcccgtatgaaggtctgagcggcgaccaaatgggccagatcgaaaaaatttttaaggtggtgtaccctgtggatgatcatcactttaaggtgatcctgcactatggcacactggtaatcgacggggttacgccgaacatgatcgactatttcggacggccgtatgaaggcatcgccgtgttcgacggcaaaaagatcactgtaacagggaccctgtggaacggcaacaaaattatcgacgagcgcctgatcaaccccgacggctccctgctgttccgagtaaccatcaacggagtgaccggctggcggctgtgcgaacgcattctggcggctgctgctgcgggccctggtgcaggcagcctgcagcccttggccctggaggggtccctgcagaagcgtggcattgtggaacaatgctgtaccagcatctgctccctctaccagctggagaactactgcaactag

SEQ ID NO: 79 - DNA, 864 bp, synthetic construct
  source 1..864: mol_type = other DNA; note = Proinsulin NLuc A c peptide PG duplication
atggccctgtggatgcgcctcctgcccctgctggcgctgctggccctctggggacctgacccagccgcagcctttgtgaaccaacacctgtgcggctcacacctggtggaagctctctacctagtgtgcggggaacgaggcttcttctacacacccaagacccgccgggaggcagaggacctgcaggtggggcaggtggagctgggcgggggcccaggccctggtgcaggcagcctgcagcccttggccctggaggggtccctgcagaagcgtatggtcttcacactcgaagatttcgttggggactggcgacagacagccggctacaacctggaccaagtccttgaacagggaggtgtgtccagtttgtttcagaatctcggggtgtccgtaactccgatccaaaggattgtcctgagcggtgaaaatgggctgaagatcgacatccatgtcatcatcccgtatgaaggtctgagcggcgaccaaatgggccagatcgaaaaaatttttaaggtggtgtaccctgtggatgatcatcactttaaggtgatcctgcactatggcacactggtaatcgacggggttacgccgaacatgatcgactatttcggacggccgtatgaaggcatcgccgtgttcgacggcaaaaagatcactgtaacagggaccctgtggaacggcaacaaaattatcgacgagcgcctgatcaaccccgacggctccctgctgttccgagtaaccatcaacggagtgaccggctggcggctgtgcgaacgcattctggcggctgctgctgcgggcattgtggaacaatgctgtaccagcatctgctccctctaccagctggagaactactgcaactag

SEQ ID NO: 80 - DNA, 858 bp, synthetic construct
  source 1..858: mol_type = other DNA; note = Proinsulin NLuc A
atggccctgtggatgcgcctcctgcccctgctggcgctgctggccctctggggacctgacccagccgcagcctttgtgaaccaacacctgtgcggctcacacctggtggaagctctctacctagtgtgcggggaacgaggcttcttctacacacccaagacccgccgggaggcagaggacctgcaggtggggcaggtggagctgggcgggggcccaggcgcaggcagcctgcagcccttggccctggaggggtccctgcagaagcgtatggtcttcacactcgaagatttcgttggggactggcgacagacagccggctacaacctggaccaagtccttgaacagggaggtgtgtccagtttgtttcagaatctcggggtgtccgtaactccgatccaaaggattgtcctgagcggtgaaaatgggctgaagatcgacatccatgtcatcatcccgtatgaaggtctgagcggcgaccaaatgggccagatcgaaaaaatttttaaggtggtgtaccctgtggatgatcatcactttaaggtgatcctgcactatggcacactggtaatcgacggggttacgccgaacatgatcgactatttcggacggccgtatgaaggcatcgccgtgttcgacggcaaaaagatcactgtaacagggaccctgtggaacggcaacaaaattatcgacgagcgcctgatcaaccccgacggctccctgctgttccgagtaaccatcaacggagtgaccggctggcggctgtgcgaacgcattctggcggctgctgctgcgggcattgtggaacaatgctgtaccagcatctgctccctctaccagctggagaactactgcaactag

SEQ ID NO: 81 - DNA, 873 bp, synthetic construct
  source 1..873: mol_type = other DNA; note = secNLuc Proinsulin
atgaactccttctccacaagcgccttcggtccagttgccttctccctgggcctgctcctggtgttgcctgctgccttccctgccccagtcttcacactcgaagatttcgttggggactggcgacagacagccggctacaacctggaccaagtccttgaacagggaggtgtgtccagtttgtttcagaatctcggggtgtccgtaactccgatccaaaggattgtcctgagcggtgaaaatgggctgaagatcgacatccatgtcatcatcccgtatgaaggtctgagcggcgaccaaatgggccagatcgaaaaaatttttaaggtggtgtaccctgtggatgatcatcactttaaggtgatcctgcactatggcacactggtaatcgacggggttacgccgaacatgatcgactatttcggacggccgtatgaaggcatcgccgtgttcgacggcaaaaagatcactgtaacagggaccctgtggaacggcaacaaaattatcgacgagcgcctgatcaaccccgacggctccctgctgttccgagtaaccatcaacggagtgaccggctggcggctgtgcgaacgcattctggcgggtggaggctttgtgaaccaacacctgtgcggctcacacctggtggaagctctctacctagtgtgcggggaacgaggcttcttctacacacccaagacccgccgggaggcagaggacctgcaggtggggcaggtggagctgggcgggggcccaggccctggtgcaggcagcctgcagcccttggccctggaggggtccctgcagaagcgtggcattgtggaacaatgctgtaccagcatctgctccctctaccagctggagaactactgcaactag

SEQ ID NO: 82 - DNA, 858 bp, synthetic construct
  source 1..858: mol_type = other DNA; note = Proinsulin NLuc A mut A L13A
atggccctgtggatgcgcctcctgcccctgctggcgctgctggccctctggggacctgacccagccgcagcctttgtgaaccaacacctgtgcggctcacacctggtggaagctctctacctagtgtgcggggaacgaggcttcttctacacacccaagacccgccgggaggcagaggacctgcaggtggggcaggtggagctgggcgggggcccaggcgcaggcagcctgcagcccttggccctggaggggtccctgcagaagcgtatggtcttcacactcgaagatttcgttggggactggcgacagacagccggctacaacctggaccaagtccttgaacagggaggtgtgtccagtttgtttcagaatctcggggtgtccgtaactccgatccaaaggattgtcctgagcggtgaaaatgggctgaagatcgacatccatgtcatcatcccgtatgaaggtctgagcggcgaccaaatgggccagatcgaaaaaatttttaaggtggtgtaccctgtggatgatcatcactttaaggtgatcctgcactatggcacactggtaatcgacggggttacgccgaacatgatcgactatttcggacggccgtatgaaggcatcgccgtgttcgacggcaaaaagatcactgtaacagggaccctgtggaacggcaacaaaattatcgacgagcgcctgatcaaccccgacggctccctgctgttccgagtaaccatcaacggagtgaccggctggcggctgtgcgaacgcattctggcggctgctgctgcgggcattgtggaacaatgctgtaccagcatctgctccgcctaccagctggagaactactgcaactag

SEQ ID NO: 83 - DNA, 858 bp, synthetic construct
  source 1..858: mol_type = other DNA; note = Proinsulin NLuc A mut A L13W
atggccctgtggatgcgcctcctgcccctgctggcgctgctggccctctggggacctgacccagccgcagcctttgtgaaccaacacctgtgcggctcacacctggtggaagctctctacctagtgtgcggggaacgaggcttcttctacacacccaagacccgccgggaggcagaggacctgcaggtggggcaggtggagctgggcgggggcccaggcgcaggcagcctgcagcccttggccctggaggggtccctgcagaagcgtatggtcttcacactcgaagatttcgttggggactggcgacagacagccggctacaacctggaccaagtccttgaacagggaggtgtgtccagtttgtttcagaatctcggggtgtccgtaactccgatccaaaggattgtcctgagcggtgaaaatgggctgaagatcgacatccatgtcatcatcccgtatgaaggtctgagcggcgaccaaatgggccagatcgaaaaaatttttaaggtggtgtaccctgtggatgatcatcactttaaggtgatcctgcactatggcacactggtaatcgacggggttacgccgaacatgatcgactatttcggacggccgtatgaaggcatcgccgtgttcgacggcaaaaagatcactgtaacagggaccctgtggaacggcaacaaaattatcgacgagcgcctgatcaaccccgacggctccctgctgttccgagtaaccatcaacggagtgaccggctggcggctgtgcgaacgcattctggcggctgctgctgcgggcattgtggaacaatgctgtaccagcatctgctcctggtaccagctggagaactactgcaactag

SEQ ID NO: 84 - DNA, 858 bp, synthetic construct
  source 1..858: mol_type = other DNA; note = Proinsulin NLuc A mut A Y14A
atggccctgtggatgcgcctcctgcccctgctggcgctgctggccctctggggacctgacccagccgcagcctttgtgaaccaacacctgtgcggctcacacctggtggaagctctctacctagtgtgcggggaacgaggcttcttctacacacccaagacccgccgggaggcagaggacctgcaggtggggcaggtggagctgggcgggggcccaggcgcaggcagcctgcagcccttggccctggaggggtccctgcagaagcgtatggtcttcacactcgaagatttcgttggggactggcgacagacagccggctacaacctggaccaagtccttgaacagggaggtgtgtccagtttgtttcagaatctcggggtgtccgtaactccgatccaaaggattgtcctgagcggtgaaaatgggctgaagatcgacatccatgtcatcatcccgtatgaaggtctgagcggcgaccaaatgggccagatcgaaaaaatttttaaggtggtgtaccctgtggatgatcatcactttaaggtgatcctgcactatggcacactggtaatcgacggggttacgccgaacatgatcgactatttcggacggccgtatgaaggcatcgccgtgttcgacggcaaaaagatcactgtaacagggaccctgtggaacggcaacaaaattatcgacgagcgcctgatcaaccccgacggctccctgctgttccgagtaaccatcaacggagtgaccggctggcggctgtgcgaacgcattctggcggctgctgctgcgggcattgtggaacaatgctgtaccagcatctgctccctcgcccagctggagaactactgcaactag

SEQ ID NO: 85 - DNA, 858 bp, synthetic construct
  source 1..858: mol_type = other DNA; note = Proinsulin NLuc A mut B F1A
atggccctgtggatgcgcctcctgcccctgctggcgctgctggccctctggggacctgacccagccgcagccgctgtgaaccaacacctgtgcggctcacacctggtggaagctctctacctagtgtgcggggaacgaggcttcttctacacacccaagacccgccgggaggcagaggacctgcaggtggggcaggtggagctgggcgggggcccaggcgcaggcagcctgcagcccttggccctggaggggtccctgcagaagcgtatggtcttcacactcgaagatttcgttggggactggcgacagacagccggctacaacctggaccaagtccttgaacagggaggtgtgtccagtttgtttcagaatctcggggtgtccgtaactccgatccaaaggattgtcctgagcggtgaaaatgggctgaagatcgacatccatgtcatcatcccgtatgaaggtctgagcggcgaccaaatgggccagatcgaaaaaatttttaaggtggtgtaccctgtggatgatcatcactttaaggtgatcctgcactatggcacactggtaatcgacggggttacgccgaacatgatcgactatttcggacggccgtatgaaggcatcgccgtgttcgacggcaaaaagatcactgtaacagggaccctgtggaacggcaacaaaattatcgacgagcgcctgatcaaccccgacggctccctgctgttccgagtaaccatcaacggagtgaccggctggcggctgtgcgaacgcattctggcggctgctgctgcgggcattgtggaacaatgctgtaccagcatctgctccctctaccagctggagaactactgcaactag

SEQ ID NO: 86 - DNA, 858 bp, synthetic construct
  source 1..858: mol_type = other DNA; note = Proinsulin NLuc A mut B L17A V18A
atggccctgtggatgcgcctcctgcccctgctggcgctgctggccctctggggacctgacccagccgcagcctttgtgaaccaacacctgtgcggctcacacctggtggaagctctctacgcagcgtgcggggaacgaggcttcttctacacacccaagacccgccgggaggcagaggacctgcaggtggggcaggtggagctgggcgggggcccaggcgcaggcagcctgcagcccttggccctggaggggtccctgcagaagcgtatggtcttcacactcgaagatttcgttggggactggcgacagacagccggctacaacctggaccaagtccttgaacagggaggtgtgtccagtttgtttcagaatctcggggtgtccgtaactccgatccaaaggattgtcctgagcggtgaaaatgggctgaagatcgacatccatgtcatcatcccgtatgaaggtctgagcggcgaccaaatgggccagatcgaaaaaatttttaaggtggtgtaccctgtggatgatcatcactttaaggtgatcctgcactatggcacactggtaatcgacggggttacgccgaacatgatcgactatttcggacggccgtatgaaggcatcgccgtgttcgacggcaaaaagatcactgtaacagggaccctgtggaacggcaacaaaattatcgacgagcgcctgatcaaccccgacggctccctgctgttccgagtaaccatcaacggagtgaccggctggcggctgtgcgaacgcattctggcggctgctgctgcgggcattgtggaacaatgctgtaccagcatctgctccctctaccagctggagaactactgcaactag

SEQ ID NO: 87 - DNA, 858 bp, synthetic construct
  source 1..858: mol_type = other DNA; note = Proinsulin NLuc A mut B L17A
atggccctgtggatgcgcctcctgcccctgctggcgctgctggccctctggggacctgacccagccgcagcctttgtgaaccaacacctgtgcggctcacacctggtggaagctctctacgcagtgtgcggggaacgaggcttcttctacacacccaagacccgccgggaggcagaggacctgcaggtggggcaggtggagctgggcgggggcccaggcgcaggcagcctgcagcccttggccctggaggggtccctgcagaagcgtatggtcttcacactcgaagatttcgttggggactggcgacagacagccggctacaacctggaccaagtccttgaacagggaggtgtgtccagtttgtttcagaatctcggggtgtccgtaactccgatccaaaggattgtcctgagcggtgaaaatgggctgaagatcgacatccatgtcatcatcccgtatgaaggtctgagcggcgaccaaatgggccagatcgaaaaaatttttaaggtggtgtaccctgtggatgatcatcactttaaggtgatcctgcactatggcacactggtaatcgacggggttacgccgaacatgatcgactatttcggacggccgtatgaaggcatcgccgtgttcgacggcaaaaagatcactgtaacagggaccctgtggaacggcaacaaaattatcgacgagcgcctgatcaaccccgacggctccctgctgttccgagtaaccatcaacggagtgaccggctggcggctgtgcgaacgcattctggcggctgctgctgcgggcattgtggaacaatgctgtaccagcatctgctccctctaccagctggagaactactgcaactag

SEQ ID NO: 88 - DNA, 4914 bp, synthetic construct
  source 1..4914: mol_type = other DNA; note = pCMVTnT ProIns B Nluc A chain L13A
tcaatattggccattagccatattattcattggttatatagcataaatcaatattggctattggccattgcatacgttgtatctatatcataatatgtacatttatattggctcatgtccaatatgaccgccatgttggcattgattattgactagttattaatagtaatcaattacggggtcattagttcatagcccatatatggagttccgcgttacataacttacggtaaatggcccgcctggctgaccgcccaacgacccccgcccattgacgtcaataatgacgtatgttcccatagtaacgccaatagggactttccattgacgtcaatgggtggagtatttacggtaaactgcccacttggcagtacatcaagtgtatcatatgccaagtccgccccctattgacgtcaatgacggtaaatggcccgcctggcattatgcccagtacatgaccttacgggactttcctacttggcagtacatctacgtattagtcatcgctattaccatggtgatgcggttttggcagtacaccaatgggcgtggatagcggtttgactcacggggatttccaagtctccaccccattgacgtcaatgggagtttgttttggcaccaaaatcaacgggactttccaaaatgtcgtaataaccccgccccgttgacgcaaatgggcggtaggcgtgtacggtgggaggtctatataagcagagctcgtttagtgaaccgtcagatcactagaagctttattgcggtagtttatcacagttaaattgctaacgcagtcagtgcttctgacacaacagtctcgaacttaagctgcagaagttggtcgtgaggcactgggcaggtaagtatcaaggttacaagacaggtttaaggagaccaatagaaactgggcttgtcgagacagagaagactcttgcgtttctgataggcacctattggtcttactgacatccactttgcctttctctccacaggtgtccactcccagttcaattacagctcttaaggctagagtacttaatacgactcactataggctagcatttaggtgacactatagaatacaagctacttgttctttttgcactcgagaattcatggccctgtggatgcgcctcctgcccctgctggcgctgctggccctctggggacctgacccagccgcagcctttgtgaaccaacacctgtgcggctcacacctggtggaagctctctacctagtgtgcggggaacgaggcttcttctacacacccaagaccatggtcttcacactcgaagatttcgttggggactggcgacagacagccggctacaacctggaccaagtccttgaacagggaggtgtgtccagtttgtttcagaatctcggggtgtccgtaactccgatccaaaggattgtcctgagcggtgaaaatgggctgaagatcgacatccatgtcatcatcccgtatgaaggtctgagcggcgaccaaatgggccagatcgaaaaaatttttaaggtggtgtaccctgtggatgatcatcactttaaggtgatcctgcactatggcacactggtaatcgacggggttacgccgaacatgatcgactatttcggacggccgtatgaaggcatcgccgtgttcgacggcaaaaagatcactgtaacagggaccctgtggaacggcaacaaaattatcgacgagcgcctgatcaaccccgacggctccctgctgttccgagtaaccatcaacggagtgaccggctggcggctgtgcgaacgcattctggcggctgctgctgcgcgccgggaggcagaggacctgcaggtggggcaggtggagctgggcgggggcccaggcgcaggcagcctgcagcccttggccctggaggggtccctgcagaagcgtggcattgtggaacaatgctgtaccagcatctgctccgcctaccagctggagaactactgcaactaggaattcacgcgtggtacctctagagtcgacccgggcggccgcttcgagcagacatgataagatacattgatgagtttggacaaaccacaactagaatgcagtgaaaaaaatgctttatttgtgaaatttgtgatgctattgctttatttgtaaccattataagctgcaataaacaagttaacaacaacaattgcattcattttatgtttcaggttcagggggagatgtgggaggttttttaaagcaagtaaaacctctacaaatgtggtaaaatcgataaggatccgggctggcgtaatagcgaagaggcccgcaccgatcgcccttcccaacagttgcgcagcctgaatggcgaatggacgcgccctgtagcggcgcattaagcgcggcgggtgtggtggttacgcgcagcgtgaccgctacacttgccagcgccctagcgcccgctcctttcgctttcttcccttcctttctcgccacgttcgccggctttccccgtcaagctctaaatcgggggctccctttagggttccgatttagtgctttacggcacctcgaccccaaaaaacttgattagggtgatggttcacgtagtgggccatcgccctgatagacggtttttcgccctttgacgttggagtccacgttctttaatagtggactcttgttccaaactggaacaacactcaaccctatctcggtctattcttttgatttataagggattttgccgatttcggcctattggttaaaaaatgagctgatttaacaaaaatttaacgcgaattttaacaaaatattaacgcttacaatttcctgatgcggtattttctccttacgcatctgtgcggtatttcacaccgcatatggtgcactctcagtacaatctgctctgatgccgcatagttaagccagccccgacacccgccaacacccgctgacgcgccctgacgggcttgtctgctcccggcatccgcttacagacaagctgtgaccgtctccgggagctgcatgtgtcagaggttttcaccgtcatcaccgaaacgcgcgagacgaaagggcctcgtgatacgcctatttttataggttaatgtcatgataataatggtttcttagacgtcaggtggcacttttcggggaaatgtgcgcggaacccctatttgtttatttttctaaatacattcaaatatgtatccgctcatgagacaataaccctgataaatgcttcaataatattgaaaaaggaagagtatgagtattcaacatttccgtgtcgcccttattcccttttttgcggcattttgccttcctgtttttgctcacccagaaacgctggtgaaagtaaaagatgctgaagatcagttgggtgcacgagtgggttacatcgaactggatctcaacagcggtaagatccttgagagttttcgccccgaagaacgttttccaatgatgagcacttttaaagttctgctatgtggcgcggtattatcccgtattgacgccgggcaagagcaactcggtcgccgcatacactattctcagaatgacttggttgagtactcaccagtcacagaaaagcatcttacggatggcatgacagtaagagaattatgcagtgctgccataaccatgagtgataacactgcggccaacttacttctgacaacgatcggaggaccgaaggagctaaccgcttttttgcacaacatgggggatcatgtaactcgccttgatcgttgggaaccggagctgaatgaagccataccaaacgacgagcgtgacaccacgatgcctgtagcaatggcaacaacgttgcgcaaactattaactggcgaactacttactctagcttcccggcaacaattaatagactggatggaggcggataaagttgcaggaccacttctgcgctcggcccttccggctggctggtttattgctgataaatctggagccggtgagcgtgggtctcgcggtatcattgcagcactggggccagatggtaagccctcccgtatcgtagttatctacacgacggggagtcaggcaactatggatgaacgaaatagacagatcgctgagataggtgcctcactgattaagcattggtaactgtcagaccaagtttactcatatatactttagattgatttaaaacttcatttttaatttaaaaggatctaggtgaagatcctttttgataatctcatgaccaaaatcccttaacgtgagttttcgttccactgagcgtcagaccccgtagaaaagatcaaaggatcttcttgagatcctttttttctgcgcgtaatctgctgcttgcaaacaaaaaaaccaccgctaccagcggtggtttgtttgccggatcaagagctaccaactctttttccgaaggtaactggcttcagcagagcgcagataccaaatactgttcttctagtgtagccgtagttaggccaccacttcaagaactctgtagcaccgcctacatacctcgctctgctaatcctgttaccagtggctgctgccagtggcgataagtcgtgtcttaccgggttggactcaagacgatagttaccggataaggcgcagcggtcgggctgaacggggggttcgtgcacacagcccagcttggagcgaacgacctacaccgaactgagatacctacagcgtgagctatgagaaagcgccacgcttcccgaagggagaaaggcggacaggtatccggtaagcggcagggtcggaacaggagagcgcacgagggagcttccagggggaaacgcctggtatctttatagtcctgtcgggtttcgccacctctgacttgagcgtcgatttttgtgatgctcgtcaggggggcggagcctatggaaaaacgccagcaacgcggcctttttacggttcctggccttttgctggccttttgctcacatggctcgacagatct

SEQ ID NO: 89 - DNA, 4914 bp, synthetic construct
  source 1..4914: mol_type = other DNA; note = pCMVTnT ProIns B Nluc A chain L13W
tcaatattggccattagccatattattcattggttatatagcataaatcaatattggctattggccattgcatacgttgtatctatatcataatatgtacatttatattggctcatgtccaatatgaccgccatgttggcattgattattgactagttattaatagtaatcaattacggggtcattagttcatagcccatatatggagttccgcgttacataacttacggtaaatggcccgcctggctgaccgcccaacgacccccgcccattgacgtcaataatgacgtatgttcccatagtaacgccaatagggactttccattgacgtcaatgggtggagtatttacggtaaactgcccacttggcagtacatcaagtgtatcatatgccaagtccgccccctattgacgtcaatgacggtaaatggcccgcctggcattatgcccagtacatgaccttacgggactttcctacttggcagtacatctacgtattagtcatcgctattaccatggtgatgcggttttggcagtacaccaatgggcgtggatagcggtttgactcacggggatttccaagtctccaccccattgacgtcaatgggagtttgttttggcaccaaaatcaacgggactttccaaaatgtcgtaataaccccgccccgttgacgcaaatgggcggtaggcgtgtacggtgggaggtctatataagcagagctcgtttagtgaaccgtcagatcactagaagctttattgcggtagtttatcacagttaaattgctaacgcagtcagtgcttctgacacaacagtctcgaacttaagctgcagaagttggtcgtgaggcactgggcaggtaagtatcaaggttacaagacaggtttaaggagaccaatagaaactgggcttgtcgagacagagaagactcttgcgtttctgataggcacctattggtcttactgacatccactttgcctttctctccacaggtgtccactcccagttcaattacagctcttaaggctagagtacttaatacgactcactataggctagcatttaggtgacactatagaatacaagctacttgttctttttgcactcgagaattcatggccctgtggatgcgcctcctgcccctgctggcgctgctggccctctggggacctgacccagccgcagcctttgtgaaccaacacctgtgcggctcacacctggtggaagctctctacctagtgtgcggggaacgaggcttcttctacacacccaagaccatggtcttcacactcgaagatttcgttggggactggcgacagacagccggctacaacctggaccaagtccttgaacagggaggtgtgtccagtttgtttcagaatctcggggtgtccgtaactccgatccaaaggattgtcctgagcggtgaaaatgggctgaagatcgacatccatgtcatcatcccgtatgaaggtctgagcggcgaccaaatgggccagatcgaaaaaatttttaaggtggtgtaccctgtggatgatcatcactttaaggtgatcctgcactatggcacactggtaatcgacggggttacgccgaacatgatcgactatttcggacggccgtatgaaggcatcgccgtgttcgacggcaaaaagatcactgtaacagggaccctgtggaacggcaacaaaattatcgacgagcgcctgatcaaccccgacggctccctgctgttccgagtaaccatcaacggagtgaccggctggcggctgtgcgaacgcattctggcggctgctgctgcgcgccgggaggcagaggacctgcaggtggggcaggtggagctgggcgggggcccaggcgcaggcagcctgcagcccttggccctggaggggtccctgcagaagcgtggcattgtggaacaatgctgtaccagcatctgctcctggtaccagctggagaactactgcaactaggaattcacgcgtggtacctctagagtcgacccgggcggccgcttcgagcagacatgataagatacattgatgagtttggacaaaccacaactagaatgcagtgaaaaaaatgctttatttgtgaaatttgtgatgctattgctttatttgtaaccattataagctgcaataaacaagttaacaacaacaattgcattcattttatgtttcaggttcagggggagatgtgggaggttttttaaagcaagtaaaacctctacaaatgtggtaaaatcgataaggatccgggctggcgtaatagcgaagaggcccgcaccgatcgcccttcccaacagttgcgcagcctgaatggcgaatggacgcgccctgtagcggcgcattaagcgcggcgggtgtggtggttacgcgcagcgtgaccgctacacttgccagcgccctagcgcccgctcctttcgctttcttcccttcctttctcgccacgttcgccggctttccccgtcaagctctaaatcgggggctccctttagggttccgatttagtgctttacggcacctcgaccccaaaaaacttgattagggtgatggttcacgtagtgggccatcgccctgatagacggtttttcgccctttgacgttggagtccacgttctttaatagtggactcttgttccaaactggaacaacactcaaccctatctcggtctattcttttgatttataagggattttgccgatttcggcctattggttaaaaaatgagctgatttaacaaaaatttaacgcgaattttaacaaaatattaacgcttacaatttcctgatgcggtattttctccttacgcatctgtgcggtatttcacaccgcatatggtgcactctcagtacaatctgctctgatgccgcatagttaagccagccccgacacccgccaacacccgctgacgcgccctgacgggcttgtctgctcccggcatccgcttacagacaagctgtgaccgtctccgggagctgcatgtgtcagaggttttcaccgtcatcaccgaaacgcgcgagacgaaagggcctcgtgatacgcctatttttataggttaatgtcatgataataatggtttcttagacgtcaggtggcacttttcggggaaatgtgcgcggaacccctatttgtttatttttctaaatacattcaaatatgtatccgctcatgagacaataaccctgataaatgcttcaataatattgaaaaaggaagagtatgagtattcaacatttccgtgtcgcccttattcccttttttgcggcattttgccttcctgtttttgctcacccagaaacgctggtgaaagtaaaagatgctgaagatcagttgggtgcacgagtgggttacatcgaactggatctcaacagcggtaagatccttgagagttttcgccccgaagaacgttttccaatgatgagcacttttaaagttctgctatgtggcgcggtattatcccgtattgacgccgggcaagagcaactcggtcgccgcatacactattctcagaatgacttggttgagtactcaccagtcacagaaaagcatcttacggatggcatgacagtaagagaattatgcagtgctgccataaccatgagtgataacactgcggccaacttacttctgacaacgatcggaggaccgaaggagctaaccgcttttttgcacaacatgggggatcatgtaactcgccttgatcgttgggaaccggagctgaatgaagccataccaaacgacgagcgtgacaccacgatgcctgtagcaatggcaacaacgttgcgcaaactattaactggcgaactacttactctagcttcccggcaacaattaatagactggatggaggcggataaagttgcaggaccacttctgcgctcggcccttccggctggctggtttattgctgataaatctggagccggtgagcgtgggtctcgcggtatcattgcagcactggggccagatggtaagccctcccgtatcgtagttatctacacgacggggagtcaggcaactatggatgaacgaaatagacagatcgctgagataggtgcctcactgattaagcattggtaactgtcagaccaagtttactcatatatactttagattgatttaaaacttcatttttaatttaaaaggatctaggtgaagatcctttttgataatctcatgaccaaaatcccttaacgtgagttttcgttccactgagcgtcagaccccgtagaaaagatcaaaggatcttcttgagatcctttttttctgcgcgtaatctgctgcttgcaaacaaaaaaaccaccgctaccagcggtggtttgtttgccggatcaagagctaccaactctttttccgaaggtaactggcttcagcagagcgcagataccaaatactgttcttctagtgtagccgtagttaggccaccacttcaagaactctgtagcaccgcctacatacctcgctctgctaatcctgttaccagtggctgctgccagtggcgataagtcgtgtcttaccgggttggactcaagacgatagttaccggataaggcgcagcggtcgggctgaacggggggttcgtgcacacagcccagcttggagcgaacgacctacaccgaactgagatacctacagcgtgagctatgagaaagcgccacgcttcccgaagggagaaaggcggacaggtatccggtaagcggcagggtcggaacaggagagcgcacgagggagcttccagggggaaacgcctggtatctttatagtcctgtcgggtttcgccacctctgacttgagcgtcgatttttgtgatgctcgtcaggggggcggagcctatggaaaaacgccagcaacgcggcctttttacggttcctggccttttgctggccttttgctcacatggctcgacagatct

SEQ ID NO: 90 - DNA, 4914 bp, synthetic construct
  source 1..4914: mol_type = other DNA; note = pCMVTnT Proinsulin B Nluc A chain E17A
tcaatattggccattagccatattattcattggttatatagcataaatcaatattggctattggccattgcatacgttgtatctatatcataatatgtacatttatattggctcatgtccaatatgaccgccatgttggcattgattattgactagttattaatagtaatcaattacggggtcattagttcatagcccatatatggagttccgcgttacataacttacggtaaatggcccgcctggctgaccgcccaacgacccccgcccattgacgtcaataatgacgtatgttcccatagtaacgccaatagggactttccattgacgtcaatgggtggagtatttacggtaaactgcccacttggcagtacatcaagtgtatcatatgccaagtccgccccctattgacgtcaatgacggtaaatggcccgcctggcattatgcccagtacatgaccttacgggactttcctacttggcagtacatctacgtattagtcatcgctattaccatggtgatgcggttttggcagtacaccaatgggcgtggatagcggtttgactcacggggatttccaagtctccaccccattgacgtcaatgggagtttgttttggcaccaaaatcaacgggactttccaaaatgtcgtaataaccccgccccgttgacgcaaatgggcggtaggcgtgtacggtgggaggtctatataagcagagctcgtttagtgaaccgtcagatcactagaagctttattgcggtagtttatcacagttaaattgctaacgcagtcagtgcttctgacacaacagtctcgaacttaagctgcagaagttggtcgtgaggcactgggcaggtaagtatcaaggttacaagacaggtttaaggagaccaatagaaactgggcttgtcgagacagagaagactcttgcgtttctgataggcacctattggtcttactgacatccactttgcctttctctccacaggtgtccactcccagttcaattacagctcttaaggctagagtacttaatacgactcactataggctagcatttaggtgacactatagaatacaagctacttgttctttttgcactcgagaattcatggccctgtggatgcgcctcctgcccctgctggcgctgctggccctctggggacctgacccagccgcagcctttgtgaaccaacacctgtgcggctcacacctggtggaagctctctacctagtgtgcggggaacgaggcttcttctacacacccaagaccatggtcttcacactcgaagatttcgttggggactggcgacagacagccggctacaacctggaccaagtccttgaacagggaggtgtgtccagtttgtttcagaatctcggggtgtccgtaactccgatccaaaggattgtcctgagcggtgaaaatgggctgaagatcgacatccatgtcatcatcccgtatgaaggtctgagcggcgaccaaatgggccagatcgaaaaaatttttaaggtggtgtaccctgtggatgatcatcactttaaggtgatcctgcactatggcacactggtaatcgacggggttacgccgaacatgatcgactatttcggacggccgtatgaaggcatcgccgtgttcgacggcaaaaagatcactgtaacagggaccctgtggaacggcaacaaaattatcgacgagcgcctgatcaaccccgacggctccctgctgttccgagtaaccatcaacggagtgaccggctggcggctgtgcgaacgcattctggcggctgctgctgcgcgccgggaggcagaggacctgcaggtggggcaggtggagctgggcgggggcccaggcgcaggcagcctgcagcccttggccctggaggggtccctgcagaagcgtggcattgtggaacaatgctgtaccagcatctgctccctctaccagctggcgaactactgcaactaggaattcacgcgtggtacctctagagtcgacccgggcggccgcttcgagcagacatgataagatacattgatgagtttggacaaaccacaactagaatgcagtgaaaaaaatgctttatttgtgaaatttgtgatgctattgctttatttgtaaccattataagctgcaataaacaagttaacaacaacaattgcattcattttatgtttcaggttcagggggagatgtgggaggttttttaaagcaagtaaaacctctacaaatgtggtaaaatcgataaggatccgggctggcgtaatagcgaagaggcccgcaccgatcgcccttcccaacagttgcgcagcctgaatggcgaatggacgcgccctgtagcggcgcattaagcgcggcgggtgtggtggttacgcgcagcgtgaccgctacacttgccagcgccctagcgcccgctcctttcgctttcttcccttcctttctcgccacgttcgccggctttccccgtcaagctctaaatcgggggctccctttagggttccgatttagtgctttacggcacctcgaccccaaaaaacttgattagggtgatggttcacgtagtgggccatcgccctgatagacggtttttcgccctttgacgttggagtccacgttctttaatagtggactcttgttccaaactggaacaacactcaaccctatctcggtctattcttttgatttataagggattttgccgatttcggcctattggttaaaaaatgagctgatttaacaaaaatttaacgcgaattttaacaaaatattaacgcttacaatttcctgatgcggtattttctccttacgcatctgtgcggtatttcacaccgcatatggtgcactctcagtacaatctgctctgatgccgcatagttaagccagccccgacacccgccaacacccgctgacgcgccctgacgggcttgtctgctcccggcatccgcttacagacaagctgtgaccgtctccgggagctgcatgtgtcagaggttttcaccgtcatcaccgaaacgcgcgagacgaaagggcctcgtgatacgcctatttttataggttaatgtcatgataataatggtttcttagacgtcaggtggcacttttcggggaaatgtgcgcggaacccctatttgtttatttttctaaatacattcaaatatgtatccgctcatgagacaataaccctgataaatgcttcaataatattgaaaaaggaagagtatgagtattcaacatttccgtgtcgcccttattcccttttttgcggcattttgccttcctgtttttgctcacccagaaacgctggtgaaagtaaaagatgctgaagatcagttgggtgcacgagtgggttacatcgaactggatctcaacagcggtaagatccttgagagttttcgccccgaagaacgttttccaatgatgagcacttttaaagttctgctatgtggcgcggtattatcccgtattgacgccgggcaagagcaactcggtcgccgcatacactattctcagaatgacttggttgagtactcaccagtcacagaaaagcatcttacggatggcatgacagtaagagaattatgcagtgctgccataaccatgagtgataacactgcggccaacttacttctgacaacgatcggaggaccgaaggagctaaccgcttttttgcacaacatgggggatcatgtaactcgccttgatcgttgggaaccggagctgaatgaagccataccaaacgacgagcgtgacaccacgatgcctgtagcaatggcaacaacgttgcgcaaactattaactggcgaactacttactctagcttcccggcaacaattaatagactggatggaggcggataaagttgcaggaccacttctgcgctcggcccttccggctggctggtttattgctgataaatctggagccggtgagcgtgggtctcgcggtatcattgcagcactggggccagatggtaagccctcccgtatcgtagttatctacacgacggggagtcaggcaactatggatgaacgaaatagacagatcgctgagataggtgcctcactgattaagcattggtaactgtcagaccaagtttactcatatatactttagattgatttaaaacttcatttttaatttaaaaggatctaggtgaagatcctttttgataatctcatgaccaaaatcccttaacgtgagttttcgttccactgagcgtcagaccccgtagaaaagatcaaaggatcttcttgagatcctttttttctgcgcgtaatctgctgcttgcaaacaaaaaaaccaccgctaccagcggtggtttgtttgccggatcaagagctaccaactctttttccgaaggtaactggcttcagcagagcgcagataccaaatactgttcttctagtgtagccgtagttaggccaccacttcaagaactctgtagcaccgcctacatacctcgctctgctaatcctgttaccagtggctgctgccagtggcgataagtcgtgtcttaccgggttggactcaagacgatagttaccggataaggcgcagcggtcgggctgaacggggggttcgtgcacacagcccagcttggagcgaacgacctacaccgaactgagatacctacagcgtgagctatgagaaagcgccacgcttcccgaagggagaaaggcggacaggtatccggtaagcggcagggtcggaacaggagagcgcacgagggagcttccagggggaaacgcctggtatctttatagtcctgtcgggtttcgccacctctgacttgagcgtcgatttttgtgatgctcgtcaggggggcggagcctatggaaaaacgccagcaacgcggcctttttacggttcctggccttttgctggccttttgctcacatggctcgacagatct

SEQ ID NO: 91 - DNA, 4914 bp, synthetic construct
  source 1..4914: mol_type = other DNA; note = pCMVTnT Proinsulin B Nluc A chain Y14A
tcaatattggccattagccatattattcattggttatatagcataaatcaatattggctattggccattgcatacgttgtatctatatcataatatgtacatttatattggctcatgtccaatatgaccgccatgttggcattgattattgactagttattaatagtaatcaattacggggtcattagttcatagcccatatatggagttccgcgttacataacttacggtaaatggcccgcctggctgaccgcccaacgacccccgcccattgacgtcaataatgacgtatgttcccatagtaacgccaatagggactttccattgacgtcaatgggtggagtatttacggtaaactgcccacttggcagtacatcaagtgtatcatatgccaagtccgccccctattgacgtcaatgacggtaaatggcccgcctggcattatgcccagtacatgaccttacgggactttcctacttggcagtacatctacgtattagtcatcgctattaccatggtgatgcggttttggcagtacaccaatgggcgtggatagcggtttgactcacggggatttccaagtctccaccccattgacgtcaatgggagtttgttttggcaccaaaatcaacgggactttccaaaatgtcgtaataaccccgccccgttgacgcaaatgggcggtaggcgtgtacggtgggaggtctatataagcagagctcgtttagtgaaccgtcagatcactagaagctttattgcggtagtttatcacagttaaattgctaacgcagtcagtgcttctgacacaacagtctcgaacttaagctgcagaagttggtcgtgaggcactgggcaggtaagtatcaaggttacaagacaggtttaaggagaccaatagaaactgggcttgtcgagacagagaagactcttgcgtttctgataggcacctattggtcttactgacatccactttgcctttctctccacaggtgtccactcccagttcaattacagctcttaaggctagagtacttaatacgactcactataggctagcatttaggtgacactatagaatacaagctacttgttctttttgcactcgagaattcatggccctgtggatgcgcctcctgcccctgctggcgctgctggccctctggggacctgacccagccgcagcctttgtgaaccaacacctgtgcggctcacacctggtggaagctctctacctagtgtgcggggaacgaggcttcttctacacacccaagaccatggtcttcacactcgaagatttcgttggggactggcgacagacagccggctacaacctggaccaagtccttgaacagggaggtgtgtccagtttgtttcagaatctcggggtgtccgtaactccgatccaaaggattgtcctgagcggtgaaaatgggctgaagatcgacatccatgtcatcatcccgtatgaaggtctgagcggcgaccaaatgggccagatcgaaaaaatttttaaggtggtgtaccctgtggatgatcatcactttaaggtgatcctgcactatggcacactggtaatcgacggggttacgccgaacatgatcgactatttcggacggccgtatgaaggcatcgccgtgttcgacggcaaaaagatcactgtaacagggaccctgtggaacggcaacaaaattatcgacgagcgcctgatcaaccccgacggctccctgctgttccgagtaaccatcaacggagtgaccggctggcggctgtgcgaacgcattctggcggctgctgctgcgcgccgggaggcagaggacctgcaggtggggcaggtggagctgggcgggggcccaggcgcaggcagcctgcagcccttggccctggaggggtccctgcagaagcgtggcattgtggaacaatgctgtaccagcatctgctccctcgcccagctggagaactactgcaactaggaattcacgcgtggtacctctagagtcgacccgggcggccgcttcgagcagacatgataagatacattgatgagtttggacaaaccacaactagaatgcagtgaaaaaaatgctttatttgtgaaatttgtgatgctattgctttatttgtaaccattataagctgcaataaacaagttaacaacaacaattgcattcattttatgtttcaggttcagggggagatgtgggaggttttttaaagcaagtaaaacctctacaaatgtggtaaaatcgataaggatccgggctggcgtaatagcgaagaggcccgcaccgatcgcccttcccaacagttgcgcagcctgaatggcgaatggacgcgccctgtagcggcgcattaagcgcggcgggtgtggtggttacgcgcagcgtgaccgctacacttgccagcgccctagcgcccgctcctttcgctttcttcccttcctttctcgccacgttcgccggctttccccgtcaagctctaaatcgggggctccctttagggttccgatttagtgctttacggcacctcgaccccaaaaaacttgattagggtgatggttcacgtagtgggccatcgccctgatagacggtttttcgccctttgacgttggagtccacgttctttaatagtggactcttgttccaaactggaacaacactcaaccctatctcggtctattcttttgatttataagggattttgccgatttcggcctattggttaaaaaatgagctgatttaacaaaaatttaacgcgaattttaacaaaatattaacgcttacaatttcctgatgcggtattttctccttacgcatctgtgcggtatttcacaccgcatatggtgcactctcagtacaatctgctctgatgccgcatagttaagccagccccgacacccgccaacacccgctgacgcgccctgacgggcttgtctgctcccggcatccgcttacagacaagctgtgaccgtctccgggagctgcatgtgtcagaggttttcaccgtcatcaccgaaacgcgcgagacgaaagggcctcgtgatacgcctatttttataggttaatgtcatgataataatggtttcttagacgtcaggtggcacttttcggggaaatgtgcgcggaacccctatttgtttatttttctaaatacattcaaatatgtatccgctcatgagacaataaccctgataaatgcttcaataatattgaaaaaggaagagtatgagtattcaacatttccgtgtcgcccttattcccttttttgcggcattttgccttcctgtttttgctcacccagaaacgctggtgaaagtaaaagatgctgaagatcagttgggtgcacgagtgggttacatcgaactggatctcaacagcggtaagatccttgagagttttcgccccgaagaacgttttccaatgatgagcacttttaaagttctgctatgtggcgcggtattatcccgtattgacgccgggcaagagcaactcggtcgccgcatacactattctcagaatgacttggttgagtactcaccagtcacagaaaagcatcttacggatggcatgacagtaagagaattatgcagtgctgccataaccatgagtgataacactgcggccaacttacttctgacaacgatcggaggaccgaaggagctaaccgcttttttgcacaacatgggggatcatgtaactcgccttgatcgttgggaaccggagctgaatgaagccataccaaacgacgagcgtgacaccacgatgcctgtagcaatggcaacaacgttgcgcaaactattaactggcgaactacttactctagcttcccggcaacaattaatagactggatggaggcggataaagttgcaggaccacttctgcgctcggcccttccggctggctggtttattgctgataaatctggagccggtgagcgtgggtctcgcggtatcattgcagcactggggccagatggtaagccctcccgtatcgtagttatctacacgacggggagtcaggcaactatggatgaacgaaatagacagatcgctgagataggtgcctcactgattaagcattggtaactgtcagaccaagtttactcatatatactttagattgatttaaaacttcatttttaatttaaaaggatctaggtgaagatcctttttgataatctcatgaccaaaatcccttaacgtgagttttcgttccactgagcgtcagaccccgtagaaaagatcaaaggatcttcttgagatcctttttttctgcgcgtaatctgctgcttgcaaacaaaaaaaccaccgctaccagcggtggtttgtttgccggatcaagagctaccaactctttttccgaaggtaactggcttcagcagagcgcagataccaaatactgttcttctagtgtagccgtagttaggccaccacttcaagaactctgtagcaccgcctacatacctcgctctgctaatcctgttaccagtggctgctgccagtggcgataagtcgtgtcttaccgggttggactcaagacgatagttaccggataaggcgcagcggtcgggctgaacggggggttcgtgcacacagcccagcttggagcgaacgacctacaccgaactgagatacctacagcgtgagctatgagaaagcgccacgcttcccgaagggagaaaggcggacaggtatccggtaagcggcagggtcggaacaggagagcgcacgagggagcttccagggggaaacgcctggtatctttatagtcctgtcgggtttcgccacctctgacttgagcgtcgatttttgtgatgctcgtcaggggggcggagcctatggaaaaacgccagcaacgcggcctttttacggttcctggccttttgctggccttttgctcacatggctcgacagatct

SEQ ID NO: 92 - DNA, 4914 bp, synthetic construct
  source 1..4914: mol_type = other DNA; note = pCMVTnT Proinsulin B Nluc B chain F1A
tcaatattggccattagccatattattcattggttatatagcataaatcaatattggctattggccattgcatacgttgtatctatatcataatatgtacatttatattggctcatgtccaatatgaccgccatgttggcattgattattgactagttattaatagtaatcaattacggggtcattagttcatagcccatatatggagttccgcgttacataacttacggtaaatggcccgcctggctgaccgcccaacgacccccgcccattgacgtcaataatgacgtatgttcccatagtaacgccaatagggactttccattgacgtcaatgggtggagtatttacggtaaactgcccacttggcagtacatcaagtgtatcatatgccaagtccgccccctattgacgtcaatgacggtaaatggcccgcctggcattatgcccagtacatgaccttacgggactttcctacttggcagtacatctacgtattagtcatcgctattaccatggtgatgcggttttggcagtacaccaatgggcgtggatagcggtttgactcacggggatttccaagtctccaccccattgacgtcaatgggagtttgttttggcaccaaaatcaacgggactttccaaaatgtcgtaataaccccgccccgttgacgcaaatgggcggtaggcgtgtacggtgggaggtctatataagcagagctcgtttagtgaaccgtcagatcactagaagctttattgcggtagtttatcacagttaaattgctaacgcagtcagtgcttctgacacaacagtctcgaacttaagctgcagaagttggtcgtgaggcactgggcaggtaagtatcaaggttacaagacaggtttaaggagaccaatagaaactgggcttgtcgagacagagaagactcttgcgtttctgataggcacctattggtcttactgacatccactttgcctttctctccacaggtgtccactcccagttcaattacagctcttaaggctagagtacttaatacgactcactataggctagcatttaggtgacactatagaatacaagctacttgttctttttgcactcgagaattcatggccctgtggatgcgcctcctgcccctgctggcgctgctggccctctggggacctgacccagccgcagccgctgtgaaccaacacctgtgcggctcacacctggtggaagctctctacctagtgtgcggggaacgaggcttcttctacacacccaagaccatggtcttcacactcgaagatttcgttggggactggcgacagacagccggctacaacctggaccaagtccttgaacagggaggtgtgtccagtttgtttcagaatctcggggtgtccgtaactccgatccaaaggattgtcctgagcggtgaaaatgggctgaagatcgacatccatgtcatcatcccgtatgaaggtctgagcggcgaccaaatgggccagatcgaaaaaatttttaaggtggtgtaccctgtggatgatcatcactttaaggtgatcctgcactatggcacactggtaatcgacggggttacgccgaacatgatcgactatttcggacggccgtatgaaggcatcgccgtgttcgacggcaaaaagatcactgtaacagggaccctgtggaacggcaacaaaattatcgacgagcgcctgatcaaccccgacggctccctgctgttccgagtaaccatcaacggagtgaccggctggcggctgtgcgaacgcattctggcggctgctgctgcgcgccgggaggcagaggacctgcaggtggggcaggtggagctgggcgggggcccaggcgcaggcagcctgcagcccttggccctggaggggtccctgcagaagcgtggcattgtggaacaatgctgtaccagcatctgctccctctaccagctggagaactactgcaactaggaattcacgcgtggtacctctagagtcgacccgggcggccgcttcgagcagacatgataagatacattgatgagtttggacaaaccacaactagaatgcagtgaaaaaaatgctttatttgtgaaatttgtgatgctattgctttatttgtaaccattataagctgcaataaacaagttaacaacaacaattgcattcattttatgtttcaggttcagggggagatgtgggaggttttttaaagcaagtaaaacctctacaaatgtggtaaaatcgataaggatccgggctggcgtaatagcgaagaggcccgcaccgatcgcccttcccaacagttgcgcagcctgaatggcgaatggacgcgccctgtagcggcgcattaagcgcggcgggtgtggtggttacgcgcagcgtgaccgctacacttgccagcgccctagcgcccgctcctttcgctttcttcccttcctttctcgccacgttcgccggctttccccgtcaagctctaaatcgggggctccctttagggttccgatttagtgctttacggcacctcgaccccaaaaaacttgattagggtgatggttcacgtagtgggccatcgccctgatagacggtttttcgccctttgacgttggagtccacgttctttaatagtggactcttgttccaaactggaacaacactcaaccctatctcggtctattcttttgatttataagggattttgccgatttcggcctattggttaaaaaatgagctgatttaacaaaaatttaacgcgaattttaacaaaatattaacgcttacaatttcctgatgcggtattttctccttacgcatctgtgcggtatttcacaccgcatatggtgcactctcagtacaatctgctctgatgccgcatagttaagccagccccgacacccgccaacacccgctgacgcgccctgacgggcttgtctgctcccggcatccgcttacagacaagctgtgaccgtctccgggagctgcatgtgtcagaggttttcaccgtcatcaccgaaacgcgcgagacgaaagggcctcgtgatacgcctatttttataggttaatgtcatgataataatggtttcttagacgtcaggtggcacttttcggggaaatgtgcgcggaacccctatttgtttatttttctaaatacattcaaatatgtatccgctcatgagacaataaccctgataaatgcttcaataatattgaaaaaggaagagtatgagtattcaacatttccgtgtcgcccttattcccttttttgcggcattttgccttcctgtttttgctcacccagaaacgctggtgaaagtaaaagatgctgaagatcagttgggtgcacgagtgggttacatcgaactggatctcaacagcggtaagatccttgagagttttcgccccgaagaacgttttccaatgatgagcacttttaaagttctgctatgtggcgcggtattatcccgtattgacgccgggcaagagcaactcggtcgccgcatacactattctcagaatgacttggttgagtactcaccagtcacagaaaagcatcttacggatggcatgacagtaagagaattatgcagtgctgccataaccatgagtgataacactgcggccaacttacttctgacaacgatcggaggaccgaaggagctaaccgcttttttgcacaacatgggggatcatgtaactcgccttgatcgttgggaaccggagctgaatgaagccataccaaacgacgagcgtgacaccacgatgcctgtagcaatggcaacaacgttgcgcaaactattaactggcgaactacttactctagcttcccggcaacaattaatagactggatggaggcggataaagttgcaggaccacttctgcgctcggcccttccggctggctggtttattgctgataaatctggagccggtgagcgtgggtctcgcggtatcattgcagcactggggccagatggtaagccctcccgtatcgtagttatctacacgacggggagtcaggcaactatggatgaacgaaatagacagatcgctgagataggtgcctcactgattaagcattggtaactgtcagaccaagtttactcatatatactttagattgatttaaaacttcatttttaatttaaaaggatctaggtgaagatcctttttgataatctcatgaccaaaatcccttaacgtgagttttcgttccactgagcgtcagaccccgtagaaaagatcaaaggatcttcttgagatcctttttttctgcgcgtaatctgctgcttgcaaacaaaaaaaccaccgctaccagcggtggtttgtttgccggatcaagagctaccaactctttttccgaaggtaactggcttcagcagagcgcagataccaaatactgttcttctagtgtagccgtagttaggccaccacttcaagaactctgtagcaccgcctacatacctcgctctgctaatcctgttaccagtggctgctgccagtggcgataagtcgtgtcttaccgggttggactcaagacgatagttaccggataaggcgcagcggtcgggctgaacggggggttcgtgcacacagcccagcttggagcgaacgacctacaccgaactgagatacctacagcgtgagctatgagaaagcgccacgcttcccgaagggagaaaggcggacaggtatccggtaagcggcagggtcggaacaggagagcgcacgagggagcttccagggggaaacgcctggtatctttatagtcctgtcgggtttcgccacctctgacttgagcgtcgatttttgtgatgctcgtcaggggggcggagcctatggaaaaacgccagcaacgcggcctttttacggttcctggccttttgctggccttttgctcacatggctcgacagatct

SEQ ID NO: 93 - DNA, 4914 bp, synthetic construct
  source 1..4914: mol_type = other DNA; note = pCMVTnT Proinsulin B Nluc B chain L17A
tcaatattggccattagccatattattcattggttatatagcataaatcaatattggctattggccattgcatacgttgtatctatatcataatatgtacatttatattggctcatgtccaatatgaccgccatgttggcattgattattgactagttattaatagtaatcaattacggggtcattagttcatagcccatatatggagttccgcgttacataacttacggtaaatggcccgcctggctgaccgcccaacgacccccgcccattgacgtcaataatgacgtatgttcccatagtaacgccaatagggactttccattgacgtcaatgggtggagtatttacggtaaactgcccacttggcagtacatcaagtgtatcatatgccaagtccgccccctattgacgtcaatgacggtaaatggcccgcctggcattatgcccagtacatgaccttacgggactttcctacttggcagtacatctacgtattagtcatcgctattaccatggtgatgcggttttggcagtacaccaatgggcgtggatagcggtttgactcacggggatttccaagtctccaccccattgacgtcaatgggagtttgttttggcaccaaaatcaacgggactttccaaaatgtcgtaataaccccgccccgttgacgcaaatgggcggtaggcgtgtacggtgggaggtctatataagcagagctcgtttagtgaaccgtcagatcactagaagctttattgcggtagtttatcacagttaaattgctaacgcagtcagtgcttctgacacaacagtctcgaacttaagctgcagaagttggtcgtgaggcactgggcaggtaagtatcaaggttacaagacaggtttaaggagaccaatagaaactgggcttgtcgagacagagaagactcttgcgtttctgataggcacctattggtcttactgacatccactttgcctttctctccacaggtgtccactcccagttcaattacagctcttaaggctagagtacttaatacgactcactataggctagcatttaggtgacactatagaatacaagctacttgttctttttgcactcgagaattcatggccctgtggatgcgcctcctgcccctgctggcgctgctggccctctggggacctgacccagccgcagcctttgtgaaccaacacctgtgcggctcacacctggtggaagctctctacgcagtgtgcggggaacgaggcttcttctacacacccaagaccatggtcttcacactcgaagatttcgttggggactggcgacagacagccggctacaacctggaccaagtccttgaacagggaggtgtgtccagtttgtttcagaatctcggggtgtccgtaactccgatccaaaggattgtcctgagcggtgaaaatgggctgaagatcgacatccatgtcatcatcccgtatgaaggtctgagcggcgaccaaatgggccagatcgaaaaaatttttaaggtggtgtaccctgtggatgatcatcactttaaggtgatcctgcactatggcacactggtaatcgacggggttacgccgaacatgatcgactatttcggacggccgtatgaaggcatcgccgtgttcgacggcaaaaagatcactgtaacagggaccctgtggaacggcaacaaaattatcgacgagcgcctgatcaaccccgacggctccctgctgttccgagtaaccatcaacggagtgaccggctggcggctgtgcgaacgcattctggcggctgctgctgcgcgccgggaggcagaggacctgcaggtggggcaggtggagctgggcgggggcccaggcgcaggcagcctgcagcccttggccctggaggggtccctgcagaagcgtggcattgtggaacaatgctgtaccagcatctgctccctctaccagctggagaactactgcaactaggaattcacgcgtggtacctctagagtcgacccgggcggccgcttcgagcagacatgataagatacattgatgagtttggacaaaccacaactagaatgcagtgaaaaaaatgctttatttgtgaaatttgtgatgctattgctttatttgtaaccattataagctgcaataaacaagttaacaacaacaattgcattcattttatgtttcaggttcagggggagatgtgggaggttttttaaagcaagtaaaacctctacaaatgtggtaaaatcgataaggatccgggctggcgtaatagcgaagaggcccgcaccgatcgcccttcccaacagttgcgcagcctgaatggcgaatggacgcgccctgtagcggcgcattaagcgcggcgggtgtggtggttacgcgcagcgtgaccgctacacttgccagcgccctagcgcccgctcctttcgctttcttcccttcctttctcgccacgttcgccggctttccccgtcaagctctaaatcgggggctccctttagggttccgatttagtgctttacggcacctcgaccccaaaaaacttgattagggtgatggttcacgtagtgggccatcgccctgatagacggtttttcgccctttgacgttggagtccacgttctttaatagtggactcttgttccaaactggaacaacactcaaccctatctcggtctattcttttgatttataagggattttgccgatttcggcctattggttaaaaaatgagctgatttaacaaaaatttaacgcgaattttaacaaaatattaacgcttacaatttcctgatgcggtattttctccttacgcatctgtgcggtatttcacaccgcatatggtgcactctcagtacaatctgctctgatgccgcatagttaagccagccccgacacccgccaacacccgctgacgcgccctgacgggcttgtctgctcccggcatccgcttacagacaagctgtgaccgtctccgggagctgcatgtgtcagaggttttcaccgtcatcaccgaaacgcgcgagacgaaagggcctcgtgatacgcctatttttataggttaatgtcatgataataatggtttcttagacgtcaggtggcacttttcggggaaatgtgcgcggaacccctatttgtttatttttctaaatacattcaaatatgtatccgctcatgagacaataaccctgataaatgcttcaataatattgaaaaaggaagagtatgagtattcaacatttccgtgtcgcccttattcccttttttgcggcattttgccttcctgtttttgctcacccagaaacgctggtgaaagtaaaagatgctgaagatcagttgggtgcacgagtgggttacatcgaactggatctcaacagcggtaagatccttgagagttttcgccccgaagaacgttttccaatgatgagcacttttaaagttctgctatgtggcgcggtattatcccgtattgacgccgggcaagagcaactcggtcgccgcatacactattctcagaatgacttggttgagtactcaccagtcacagaaaagcatcttacggatggcatgacagtaagagaattatgcagtgctgccataaccatgagtgataacactgcggccaacttacttctgacaacgatcggaggaccgaaggagctaaccgcttttttgcacaacatgggggatcatgtaactcgccttgatcgttgggaaccggagctgaatgaagccataccaaacgacgagcgtgacaccacgatgcctgtagcaatggcaacaacgttgcgcaaactattaactggcgaactacttactctagcttcccggcaacaattaatagactggatggaggcggataaagttgcaggaccacttctgcgctcggcccttccggctggctggtttattgctgataaatctggagccggtgagcgtgggtctcgcggtatcattgcagcactggggccagatggtaagccctcccgtatcgtagttatctacacgacggggagtcaggcaactatggatgaacgaaatagacagatcgctgagataggtgcctcactgattaagcattggtaactgtcagaccaagtttactcatatatactttagattgatttaaaacttcatttttaatttaaaaggatctaggtgaagatcctttttgataatctcatgaccaaaatcccttaacgtgagttttcgttccactgagcgtcagaccccgtagaaaagatcaaaggatcttcttgagatcctttttttctgcgcgtaatctgctgcttgcaaacaaaaaaaccaccgctaccagcggtggtttgtttgccggatcaagagctaccaactctttttccgaaggtaactggcttcagcagagcgcagataccaaatactgttcttctagtgtagccgtagttaggccaccacttcaagaactctgtagcaccgcctacatacctcgctctgctaatcctgttaccagtggctgctgccagtggcgataagtcgtgtcttaccgggttggactcaagacgatagttaccggataaggcgcagcggtcgggctgaacggggggttcgtgcacacagcccagcttggagcgaacgacctacaccgaactgagatacctacagcgtgagctatgagaaagcgccacgcttcccgaagggagaaaggcggacaggtatccggtaagcggcagggtcggaacaggagagcgcacgagggagcttccagggggaaacgcctggtatctttatagtcctgtcgggtttcgccacctctgacttgagcgtcgatttttgtgatgctcgtcaggggggcggagcctatggaaaaacgccagcaacgcggcctttttacggttcctggccttttgctggccttttgctcacatggctcgacagatct

SEQ ID NO: 94 - DNA, 4914 bp, synthetic construct
  source 1..4914: mol_type = other DNA; note = pCMVTnT Proinsulin B Nluc no cpeptide PG duplication
tcaatattggccattagccatattattcattggttatatagcataaatcaatattggctattggccattgcatacgttgtatctatatcataatatgtacatttatattggctcatgtccaatatgaccgccatgttggcattgattattgactagttattaatagtaatcaattacggggtcattagttcatagcccatatatggagttccgcgttacataacttacggtaaatggcccgcctggctgaccgcccaacgacccccgcccattgacgtcaataatgacgtatgttcccatagtaacgccaatagggactttccattgacgtcaatgggtggagtatttacggtaaactgcccacttggcagtacatcaagtgtatcatatgccaagtccgccccctattgacgtcaatgacggtaaatggcccgcctggcattatgcccagtacatgaccttacgggactttcctacttggcagtacatctacgtattagtcatcgctattaccatggtgatgcggttttggcagtacaccaatgggcgtggatagcggtttgactcacggggatttccaagtctccaccccattgacgtcaatgggagtttgttttggcaccaaaatcaacgggactttccaaaatgtcgtaataaccccgccccgttgacgcaaatgggcggtaggcgtgtacggtgggaggtctatataagcagagctcgtttagtgaaccgtcagatcactagaagctttattgcggtagtttatcacagttaaattgctaacgcagtcagtgcttctgacacaacagtctcgaacttaagctgcagaagttggtcgtgaggcactgggcaggtaagtatcaaggttacaagacaggtttaaggagaccaatagaaactgggcttgtcgagacagagaagactcttgcgtttctgataggcacctattggtcttactgacatccactttgcctttctctccacaggtgtccactcccagttcaattacagctcttaaggctagagtacttaatacgactcactataggctagcatttaggtgacactatagaatacaagctacttgttctttttgcactcgagaattcatggccctgtggatgcgcctcctgcccctgctggcgctgctggccctctggggacctgacccagccgcagcctttgtgaaccaacacctgtgcggctcacacctggtggaagctctctacctagtgtgcggggaacgaggcttcttctacacacccaagaccatggtcttcacactcgaagatttcgttggggactggcgacagacagccggctacaacctggaccaagtccttgaacagggaggtgtgtccagtttgtttcagaatctcggggtgtccgtaactccgatccaaaggattgtcctgagcggtgaaaatgggctgaagatcgacatccatgtcatcatcccgtatgaaggtctgagcggcgaccaaatgggccagatcgaaaaaatttttaaggtggtgtaccctgtggatgatcatcactttaaggtgatcctgcactatggcacactggtaatcgacggggttacgccgaacatgatcgactatttcggacggccgtatgaaggcatcgccgtgttcgacggcaaaaagatcactgtaacagggaccctgtggaacggcaacaaaattatcgacgagcgcctgatcaaccccgacggctccctgctgttccgagtaaccatcaacggagtgaccggctggcggctgtgcgaacgcattctggcggctgctgctgcgcgccgggaggcagaggacctgcaggtggggcaggtggagctgggcgggggcccaggcgcaggcagcctgcagcccttggccctggaggggtccctgcagaagcgtggcattgtggaacaatgctgtaccagcatctgctccctctaccagctggagaactactgcaactaggaattcacgcgtggtacctctagagtcgacccgggcggccgcttcgagcagacatgataagatacattgatgagtttggacaaaccacaactagaatgcagtgaaaaaaatgctttatttgtgaaatttgtgatgctattgctttatttgtaaccattataagctgcaataaacaagttaacaacaacaattgcattcattttatgtttcaggttcagggggagatgtgggaggttttttaaagcaagtaaaacctctacaaatgtggtaaaatcgataaggatccgggctggcgtaatagcgaagaggcccgcaccgatcgcccttcccaacagttgcgcagcctgaatggcgaatggacgcgccctgtagcggcgcattaagcgcggcgggtgtggtggttacgcgcagcgtgaccgctacacttgccagcgccctagcgcccgctcctttcgctttcttcccttcctttctcgccacgttcgccggctttccccgtcaagctctaaatcgggggctccctttagggttccgatttagtgctttacggcacctcgaccccaaaaaacttgattagggtgatggttcacgtagtgggccatcgccctgatagacggtttttcgccctttgacgttggagtccacgttctttaatagtggactcttgttccaaactggaacaacactcaaccctatctcggtctattcttttgatttataagggattttgccgatttcggcctattggttaaaaaatgagctgatttaacaaaaatttaacgcgaattttaacaaaatattaacgcttacaatttcctgatgcggtattttctccttacgcatctgtgcggtatttcacaccgcatatggtgcactctcagtacaatctgctctgatgccgcatagttaagccagccccgacacccgccaacacccgctgacgcgccctgacgggcttgtctgctcccggcatccgcttacagacaagctgtgaccgtctccgggagctgcatgtgtcagaggttttcaccgtcatcaccgaaacgcgcgagacgaaagggcctcgtgatacgcctatttttataggttaatgtcatgataataatggtttcttagacgtcaggtggcacttttcggggaaatgtgcgcggaacccctatttgtttatttttctaaatacattcaaatatgtatccgctcatgagacaataaccctgataaatgcttcaataatattgaaaaaggaagagtatgagtattcaacatttccgtgtcgcccttattcccttttttgcggcattttgccttcctgtttttgctcacccagaaacgctggtgaaagtaaaagatgctgaagatcagttgggtgcacgagtgggttacatcgaactggatctcaacagcggtaagatccttgagagttttcgccccgaagaacgttttccaatgatgagcacttttaaagttctgctatgtggcgcggtattatcccgtattgacgccgggcaagagcaactcggtcgccgcatacactattctcagaatgacttggttgagtactcaccagtcacagaaaagcatcttacggatggcatgacagtaagagaattatgcagtgctgccataaccatgagtgataacactgcggccaacttacttctgacaacgatcggaggaccgaaggagctaaccgcttttttgcacaacatgggggatcatgtaactcgccttgatcgttgggaaccggagctgaatgaagccataccaaacgacgagcgtgacaccacgatgcctgtagcaatggcaacaacgttgcgcaaactattaactggcgaactacttactctagcttcccggcaacaattaatagactggatggaggcggataaagttgcaggaccacttctgcgctcggcccttccggctggctggtttattgctgataaatctggagccggtgagcgtgggtctcgcggtatcattgcagcactggggccagatggtaagccctcccgtatcgtagttatctacacgacggggagtcaggcaactatggatgaacgaaatagacagatcgctgagataggtgcctcactgattaagcattggtaactgtcagaccaagtttactcatatatactttagattgatttaaaacttcatttttaatttaaaaggatctaggtgaagatcctttttgataatctcatgaccaaaatcccttaacgtgagttttcgttccactgagcgtcagaccccgtagaaaagatcaaaggatcttcttgagatcctttttttctgcgcgtaatctgctgcttgcaaacaaaaaaaccaccgctaccagcggtggtttgtttgccggatcaagagctaccaactctttttccgaaggtaactggcttcagcagagcgcagataccaaatactgttcttctagtgtagccgtagttaggccaccacttcaagaactctgtagcaccgcctacatacctcgctctgctaatcctgttaccagtggctgctgccagtggcgataagtcgtgtcttaccgggttggactcaagacgatagttaccggataaggcgcagcggtcgggctgaacggggggttcgtgcacacagcccagcttggagcgaacgacctacaccgaactgagatacctacagcgtgagctatgagaaagcgccacgcttcccgaagggagaaaggcggacaggtatccggtaagcggcagggtcggaacaggagagcgcacgagggagcttccagggggaaacgcctggtatctttatagtcctgtcgggtttcgccacctctgacttgagcgtcgatttttgtgatgctcgtcaggggggcggagcctatggaaaaacgccagcaacgcggcctttttacggttcctggccttttgctggccttttgctcacatggctcgacagatct

SEQ ID NO: 95 - DNA, 4920 bp, synthetic construct
  source 1..4920: mol_type = other DNA; note = pCMVTnT_hPreProIns B chain Nluc cpeptide
tcaatattggccattagccatattattcattggttatatagcataaatcaatattggctattggccattgcatacgttgtatctatatcataatatgtacatttatattggctcatgtccaatatgaccgccatgttggcattgattattgactagttattaatagtaatcaattacggggtcattagttcatagcccatatatggagttccgcgttacataacttacggtaaatggcccgcctggctgaccgcccaacgacccccgcccattgacgtcaataatgacgtatgttcccatagtaacgccaatagggactttccattgacgtcaatgggtggagtatttacggtaaactgcccacttggcagtacatcaagtgtatcatatgccaagtccgccccctattgacgtcaatgacggtaaatggcccgcctggcattatgcccagtacatgaccttacgggactttcctacttggcagtacatctacgtattagtcatcgctattaccatggtgatgcggttttggcagtacaccaatgggcgtggatagcggtttgactcacggggatttccaagtctccaccccattgacgtcaatgggagtttgttttggcaccaaaatcaacgggactttccaaaatgtcgtaataaccccgccccgttgacgcaaatgggcggtaggcgtgtacggtgggaggtctatataagcagagctcgtttagtgaaccgtcagatcactagaagctttattgcggtagtttatcacagttaaattgctaacgcagtcagtgcttctgacacaacagtctcgaacttaagctgcagaagttggtcgtgaggcactgggcaggtaagtatcaaggttacaagacaggtttaaggagaccaatagaaactgggcttgtcgagacagagaagactcttgcgtttctgataggcacctattggtcttactgacatccactttgcctttctctccacaggtgtccactcccagttcaattacagctcttaaggctagagtacttaatacgactcactataggctagcatttaggtgacactatagaatacaagctacttgttctttttgcactcgagaattcatggccctgtggatgcgcctcctgcccctgctggcgctgctggccctctggggacctgacccagccgcagcctttgtgaaccaacacctgtgcggctcacacctggtggaagctctctacctagtgtgcggggaacgaggcttcttctacacacccaagaccatggtcttcacactcgaagatttcgttggggactggcgacagacagccggctacaacctggaccaagtccttgaacagggaggtgtgtccagtttgtttcagaatctcggggtgtccgtaactccgatccaaaggattgtcctgagcggtgaaaatgggctgaagatcgacatccatgtcatcatcccgtatgaaggtctgagcggcgaccaaatgggccagatcgaaaaaatttttaaggtggtgtaccctgtggatgatcatcactttaaggtgatcctgcactatggcacactggtaatcgacggggttacgccgaacatgatcgactatttcggacggccgtatgaaggcatcgccgtgttcgacggcaaaaagatcactgtaacagggaccctgtggaacggcaacaaaattatcgacgagcgcctgatcaaccccgacggctccctgctgttccgagtaaccatcaacggagtgaccggctggcggctgtgcgaacgcattctggcggctgctgctgcgcgccgggaggcagaggacctgcaggtggggcaggtggagctgggcgggggcccaggccctggtgcaggcagcctgcagcccttggccctggaggggtccctgcagaagcgtggcattgtggaacaatgctgtaccagcatctgctccctctaccagctggagaactactgcaactaggaattcacgcgtggtacctctagagtcgacccgggcggccgcttcgagcagacatgataagatacattgatgagtttggacaaaccacaactagaatgcagtgaaaaaaatgctttatttgtgaaatttgtgatgctattgctttatttgtaaccattataagctgcaataaacaagttaacaacaacaattgcattcattttatgtttcaggttcagggggagatgtgggaggttttttaaagcaagtaaaacctctacaaatgtggtaaaatcgataaggatccgggctggcgtaatagcgaagaggcccgcaccgatcgcccttcccaacagttgcgcagcctgaatggcgaatggacgcgccctgtagcggcgcattaagcgcggcgggtgtggtggttacgcgcagcgtgaccgctacacttgccagcgccctagcgcccgctcctttcgctttcttcccttcctttctcgccacgttcgccggctttccccgtcaagctctaaatcgggggctccctttagggttccgatttagtgctttacggcacctcgaccccaaaaaacttgattagggtgatggttcacgtagtgggccatcgccctgatagacggtttttcgccctttgacgttggagtccacgttctttaatagtggactcttgttccaaactggaacaacactcaaccctatctcggtctattcttttgatttataagggattttgccgatttcggcctattggttaaaaaatgagctgatttaacaaaaatttaacgcgaattttaacaaaatattaacgcttacaatttcctgatgcggtattttctccttacgcatctgtgcggtatttcacaccgcatatggtgcactctcagtacaatctgctctgatgccgcatagttaagccagccccgacacccgccaacacccgctgacgcgccctgacgggcttgtctgctcccggcatccgcttacagacaagctgtgaccgtctccgggagctgcatgtgtcagaggttttcaccgtcatcaccgaaacgcgcgagacgaaagggcctcgtgatacgcctatttttataggttaatgtcatgataataatggtttcttagacgtcaggtggcacttttcggggaaatgtgcgcggaacccctatttgtttatttttctaaatacattcaaatatgtatccgctcatgagacaataaccctgataaatgcttcaataatattgaaaaaggaagagtatgagtattcaacatttccgtgtcgcccttattcccttttttgcggcattttgccttcctgtttttgctcacccagaaacgctggtgaaagtaaaagatgctgaagatcagttgggtgcacgagtgggttacatcgaactggatctcaacagcggtaagatccttgagagttttcgccccgaagaacgttttccaatgatgagcacttttaaagttctgctatgtggcgcggtattatcccgtattgacgccgggcaagagcaactcggtcgccgcatacactattctcagaatgacttggttgagtactcaccagtcacagaaaagcatcttacggatggcatgacagtaagagaattatgcagtgctgccataaccatgagtgataacactgcggccaacttacttctgacaacgatcggaggaccgaaggagctaaccgcttttttgcacaacatgggggatcatgtaactcgccttgatcgttgggaaccggagctgaatgaagccataccaaacgacgagcgtgacaccacgatgcctgtagcaatggcaacaacgttgcgcaaactattaactggcgaactacttactctagcttcccggcaacaattaatagactggatggaggcggataaagttgcaggaccacttctgcgctcggcccttccggctggctggtttattgctgataaatctggagccggtgagcgtgggtctcgcggtatcattgcagcactggggccagatggtaagccctcccgtatcgtagttatctacacgacggggagtcaggcaactatggatgaacgaaatagacagatcgctgagataggtgcctcactgattaagcattggtaactgtcagaccaagtttactcatatatactttagattgatttaaaacttcatttttaatttaaaaggatctaggtgaagatcctttttgataatctcatgaccaaaatcccttaacgtgagttttcgttccactgagcgtcagaccccgtagaaaagatcaaaggatcttcttgagatcctttttttctgcgcgtaatctgctgcttgcaaacaaaaaaaccaccgctaccagcggtggtttgtttgccggatcaagagctaccaactctttttccgaaggtaactggcttcagcagagcgcagataccaaatactgttcttctagtgtagccgtagttaggccaccacttcaagaactctgtagcaccgcctacatacctcgctctgctaatcctgttaccagtggctgctgccagtggcgataagtcgtgtcttaccgggttggactcaagacgatagttaccggataaggcgcagcggtcgggctgaacggggggttcgtgcacacagcccagcttggagcgaacgacctacaccgaactgagatacctacagcgtgagctatgagaaagcgccacgcttcccgaagggagaaaggcggacaggtatccggtaagcggcagggtcggaacaggagagcgcacgagggagcttccagggggaaacgcctggtatctttatagtcctgtcgggtttcgccacctctgacttgagcgtcgatttttgtgatgctcgtcaggggggcggagcctatggaaaaacgccagcaacgcggcctttttacggttcctggccttttgctggccttttgctcacatggctcgacagatct

SEQ ID NO: 96 - DNA, 864 bp, synthetic construct; identical to SEQ ID NO: 77
  source 1..864: mol_type = other DNA; note = PreProIns B chain Nluc c peptide PG duplication

SEQ ID NO: 97 - DNA, 4934 bp, synthetic construct
  source 1..4934: mol_type = other DNA; note = pCMVTnT_sNluc_hPPI_c-peptide
tcaatattggccattagccatattattcattggttatatagcataaatcaatattggctattggccattgcatacgttgtatctatatcataatatgtacatttatattggctcatgtccaatatgaccgccatgttggcattgattattgactagttattaatagtaatcaattacggggtcattagttcatagcccatatatggagttccgcgttacataacttacggtaaatggcccgcctggctgaccgcccaacgacccccgcccattgacgtcaataatgacgtatgttcccatagtaacgccaatagggactttccattgacgtcaatgggtggagtatttacggtaaactgcccacttggcagtacatcaagtgtatcatatgccaagtccgccccctattgacgtcaatgacggtaaatggcccgcctggcattatgcccagtacatgaccttacgggactttcctacttggcagtacatctacgtattagtcatcgctattaccatggtgatgcggttttggcagtacaccaatgggcgtggatagcggtttgactcacggggatttccaagtctccaccccattgacgtcaatgggagtttgttttggcaccaaaatcaacgggactttccaaaatgtcgtaataaccccgccccgttgacgcaaatgggcggtaggcgtgtacggtgggaggtctatataagcagagctcgtttagtgaaccgtcagatcactagaagctttattgcggtagtttatcacagttaaattgctaacgcagtcagtgcttctgacacaacagtctcgaacttaagctgcagaagttggtcgtgaggcactgggcaggtaagtatcaaggttacaagacaggtttaaggagaccaatagaaactgggcttgtcgagacagagaagactcttgcgtttctgataggcacctattggtcttactgacatccactttgcctttctctccacaggtgtccactcccagttcaattacagctcttaaggctagagtacttaatacgactcactataggctagcatttaggtgacactatagaatacaagctacttgttctttttgcactcgaggaattcgccgccaccatgaactccttctccacaagcgccttcggtccagttgccttctccctgggcctgctcctggtgttgcctgctgccttccctgccccagtcttcacactcgaagatttcgttggggactggcgacagacagccggctacaacctggaccaagtccttgaacagggaggtgtgtccagtttgtttcagaatctcggggtgtccgtaactccgatccaaaggattgtcctgagcggtgaaaatgggctgaagatcgacatccatgtcatcatcccgtatgaaggtctgagcggcgaccaaatgggccagatcgaaaaaatttttaaggtggtgtaccctgtggatgatcatcactttaaggtgatcctgcactatggcacactggtaatcgacggggttacgccgaacatgatcgactatttcggacggccgtatgaaggcatcgccgtgttcgacggcaaaaagatcactgtaacagggaccctgtggaacggcaacaaaattatcgacgagcgcctgatcaaccccgacggctccctgctgttccgagtaaccatcaacggagtgaccggctggcggctgtgcgaacgcattctggcgggtggaggctttgtgaaccaacacctgtgcggctcacacctggtggaagctctctacctagtgtgcggggaacgaggcttcttctacacacccaagacccgccgggaggcagaggacctgcaggtggggcaggtggagctgggcgggggcccaggccctggtgcaggcagcctgcagcccttggccctggaggggtccctgcagaagcgtggcattgtggaacaatgctgtaccagcatctgctccctctaccagctggagaactactgcaactaggaattccggtacctctagagtcgacccgggcggccgcttcgagcagacatgataagatacattgatgagtttggacaaaccacaactagaatgcagtgaaaaaaatgctttatttgtgaaatttgtgatgctattgctttatttgtaaccattataagctgcaataaacaagttaacaacaacaattgcattcattttatgtttcaggttcagggggagatgtgggaggttttttaaagcaagtaaaacctctacaaatgtggtaaaatcgataaggatccgggctggcgtaatagcgaagaggcccgcaccgatcgcccttcccaacagttgcgcagcctgaatggcgaatggacgcgccctgtagcggcgcattaagcgcggcgggtgtggtggttacgcgcagcgtgaccgctacacttgccagcgccctagcgcccgctcctttcgctttcttcccttcctttctcgccacgttcgccggctttccccgtcaagctctaaatcgggggctccctttagggttccgatttagtgctttacggcacctcgaccccaaaaaacttgattagggtgatggttcacgtagtgggccatcgccctgatagacggtttttcgccctttgacgttggagtccacgttctttaatagtggactcttgttccaaactggaacaacactcaaccctatctcggtctattcttttgatttataagggattttgccgatttcggcctattggttaaaaaatgagctgatttaacaaaaatttaacgcgaattttaacaaaatattaacgcttacaatttcctgatgcggtattttctccttacgcatctgtgcggtatttcacaccgcatatggtgcactctcagtacaatctgctctgatgccgcatagttaagccagccccgacacccgccaacacccgctgacgcgccctgacgggcttgtctgctcccggcatccgcttacagacaagctgtgaccgtctccgggagctgcatgtgtcagaggttttcaccgtcatcaccgaaacgcgcgagacgaaagggcctcgtgatacgcctatttttataggttaatgtcatgataataatggtttcttagacgtcaggtggcacttttcggggaaatgtgcgcggaacccctatttgtttatttttctaaatacattcaaatatgtatccgctcatgagacaataaccctgataaatgcttcaataatattgaaaaaggaagagtatgagtattcaacatttccgtgtcgcccttattcccttttttgcggcattttgccttcctgtttttgctcacccagaaacgctggtgaaagtaaaagatgctgaagatcagttgggtgcacgagtgggttacatcgaactggatctcaacagcggtaagatccttgagagttttcgccccgaagaacgttttccaatgatgagcacttttaaagttctgctatgtggcgcggtattatcccgtattgacgccgggcaagagcaactcggtcgccgcatacactattctcagaatgacttggttgagtactcaccagtcacagaaaagcatcttacggatggcatgacagtaagagaattatgcagtgctgccataaccatgagtgataacactgcggccaacttacttctgacaacgatcggaggaccgaaggagctaaccgcttttttgcacaacatgggggatcatgtaactcgccttgatcgttgggaaccggagctgaatgaagccataccaaacgacgagcgtgacaccacgatgcctgtagcaatggcaacaacgttgcgcaaactattaactggcgaactacttactctagcttcccggcaacaattaatagactggatggaggcggataaagttgcaggaccacttctgcgctcggcccttccggctggctggtttattgctgataaatctggagccggtgagcgtgggtctcgcggtatcattgcagcactggggccagatggtaagccctcccgtatcgtagttatctacacgacggggagtcaggcaactatggatgaacgaaatagacagatcgctgagataggtgcctcactgattaagcattggtaactgtcagaccaagtttactcatatatactttagattgatttaaaacttcatttttaatttaaaaggatctaggtgaagatcctttttgataatctcatgaccaaaatcccttaacgtgagttttcgttccactgagcgtcagaccccgtagaaaagatcaaaggatcttcttgagatcctttttttctgcgcgtaatctgctgcttgcaaacaaaaaaaccaccgctaccagcggtggtttgtttgccggatcaagagctaccaactctttttccgaaggtaactggcttcagcagagcgcagataccaaatactgttcttctagtgtagccgtagttaggccaccacttcaagaactctgtagcaccgcctacatacctcgctctgctaatcctgttaccagtggctgctgccagtggcgataagtcgtgtcttaccgggttggactcaagacgatagttaccggataaggcgcagcggtcgggctgaacggggggttcgtgcacacagcccagcttggagcgaacgacctacaccgaactgagatacctacagcgtgagctatgagaaagcgccacgcttcccgaagggagaaaggcggacaggtatccggtaagcggcagggtcggaacaggagagcgcacgagggagcttccagggggaaacgcctggtatctttatagtcctgtcgggtttcgccacctctgacttgagcgtcgatttttgtgatgctcgtcaggggggcggagcctatggaaaaacgccagcaacgcggcctttttacggttcctggccttttgctggccttttgctcacatggctcgacagatct